European Patent Application EP 4 212 169 A1, published July 19, 2023. Title: HIGH-TRANSDUCING HSV VECTORS. Applicant: Periphagen, Inc. Application EP. The sequence listing filed with the application follows.

SEQUENCE LISTING (19 sequences)

SEQ ID NO: 1 - DNA, 151135 bp, unidentified
  misc_feature 61968..62069
  source 1..151135: mol_type = genomic DNA; note = human herpesvirus 1 strain McKrae
gcagcccgggccccccgcgcgcggggcggcgcgcaaaaaaggcgggcggcggtccgggcggcgtgcgcgcgcgcggcgggcgtggggggcggggccgcgggagcgggggaggagccccacccacagacggggaggagcgggggaggagcgggggaggagcgggggaggagccccacccacagacggggaggagcgggggaggagcggccagaccccaaaaacgggcccccccgaaacacaccccccgggggtcgcgcgcggccctttaaagcgcggcggcgggcagcccgggccccccgcggccgagactagcgagttagacaggcaagcactactcgcctctgcacgcacatgcttgcctgtcaaactctaccaccccggcacgctctctgtctccatggcccgccgccgccgccatcgcggcccccgccgcccccggccgcccgggcccacgggcgccgtcccaaccgcacagtcccaggtaacctccacgcccaactcggaacccgcggtcaggagcgcgcccgcggccgccccgccgccgccccccgccggtgggcccccgccttcttgttcgctgctgctgcgccagtggctccacgttcccgagtccgcgtccgacgacgacgatgacgacgactggccggacagccccccgcccgagccggcgccagaggcccggcccaccgccgccgccccccggccccggtccccaccgcccggcgtgggcccggggggcggggctgacccctcccaccccccctcgcgccccttccgccttccgccgcgcctcgccctccgcctgcgcgtcaccgcggagcacctggcgcgcctgcgcctgcgacgcgcgggcggggagggggcgccggagccccccgcgacccccgcgacccccgcgacccccgcgacccccgcgacccccgcgacccccgcgacccccgcgacccccgcgcgggtgcgcttctcgccccacgtccgggtgcgccacctggtggtctgggcctcggccgcccgcctggcgcgccgcggctcgtgggcccgcgagcgggccgaccgggctcggttccggcgccgggtggcggaggccgaggcggtcatcgggccgtgcctggggcccgaggcccgtgcccgggccctggcccgcggagccggcccggcgaactcggtctaacgttacacccgaggcgcctgggtcttccgcggagctcccgggagctccgcaccaagccgctctccggagagacgatggcaggagccgcgcatatatacgctgggagccggtccgcccccaaggcgggcccgcctcgggggcgggactggccaatcggcggccgccagcgcggcggggcccggccaaccagcgtccgccgagtcttcggggcccggcccattgggcgggagttaccgcccaatgggccgggccgcccacttcccggtatggtaattaaaaacttgcaagaggccttgttccgcttcccggtatggtaattagaaactcattaatgggcggccccggccgcccttcccgcttccggcaattcccgcggcccttaatgggcaaccccggtattccccgcctcccgcgccgcgcgtaaccactcccctggggttccgggttatgctaattgcttttttggcggaacacacggcccctcgcgcattggcccgcgggtcgctcaatgaacccgcattggtcccctggggttccgggtatggtaatgagtttcttcgggaaggcgggaagccccggggcaccgacgcaggccaagcccctgttgcgtcggcgggaggggcatgctaatggggttctttgggggacaccgggttggtcccccaaatcgggggccgggccgtgcatgctaatgatattctttgggggcgccgggttggtccccggggacggggccgccccgcggtgggcctgcctcccctgggacgcgcggccattgggggaatcgtcactgccgcccctttggggaggggaaaggcgtggggtataagttagccctggcccgacggtctggtcgcatttgcacctcggcactcggagcgagacgcagcagccaggcagactcgggccgccccctctccgcatcaccacagaagccccgcctacgttgcgacccccagggaccctccgtccgcgaccctccagccgcatacgacccccatggagccccgccccggagcgagtacccgccggcctgagggccgcccccagcgcgaggtgaggggccgggcgccatgtctggggcgccatattggggggcgccatgttgggggacccccgacccttaccctggaaccggcccccatgttgggggacccccactcatacacgggagccgggcgccatgttggggcgccatgttagggggcgtggaaccccgtgacactatatatacagggaccgggggcgccatgttagggggcgcggaaccccctgaccctatatatacagggaccggggtcgccctgttgggggtcgccatgtgaccccctgactttatatatacagacccccaacacatacacatggcccctttgactcagacgcagggcccggggtcgccgtgggaccccctgactcatacacagagacacgcccccacaacaaacacacagggaccggggtcgccgtgttgggggcgtggtccccactgactcatacgcaggccccccttactcacacgcatctaggggggtggggaggagccgcccgccatatttgggggacgccgtgggacccccgactccggtgcgtctggagggcgggagaagagggaagaagaggggtcgggatccaaaggacggacccagaccacctttggttgcagacccctttctcccccctcttccgaggccagcaggggggcaggactttgtgaggcggggggggagagggggaactcgtgggcgctgattgacgcgggaaatccccccccattcttacccgccccccttttttccccttagcccgccccggatgtctgggtgtttccctgcgaccgagacctgccggacagcagcgactctgaggcggagaccgaagtgggggggcggggggacgccgaccaccatgacgacgactccgcctccgaggcggacagcacggacacggaactgttcgagacggggctgctggggccgcagggcgtggatgggggggcggtctcgggggggagccccccccgcgaggaagaccccggcagttgcgggggcgccccccctcgagaggacggggggagcgacgagggcgacgtgtgcgccgtgtgcacggatgagatcgcgccccacctgcgctgcgacaccttcccgtgcatgcaccgcttctgcatcccgtgcatgaaaacctggatgcaattgcgcaacacctgcccgctgtgcaacgccaagctggtgtacctgatagtgggcgtgacgcccagcgggtcgttcagcaccatcccgatcgtgaacgacccccagacccgcatggaggccgaggaggccgtcagggcgggcacggccgtggactttatctggacgggcaatcagcggttcgccccgcggtacctgaccctgggggggcacacggtgagggccctgtcgcccacccacccggagcccaccacggacgaggatgacgacgacctggacgacggtgaggcggggggcggcaaggaccctgggggaggaggaggagggaggaatgggcgggcgggcgaggaaagggcgggccggggagggggcgtaacctgatcgcgccccccgttgtctcttgcagcagactacgtcccgcccgccccccgccggacgccccgcgcccccccacgcagaggcaccgccgcgccccccgtgacgggcggggcgtctaacgcagccccccagccggccgcggctcggacagcgcccccctcggcgcccatcgggccacacggcagcagtaacaccaacaccaccaccaacagcagcggcggcggcggctcccgccagtcgcgagccgcggcgccgcggggggcgtctggcccctccgggggggttggggttggggttggggttgttgaagcggaggcggggcggccgaggggccggacgggcccccttgtcaacagacccgccccccttgcaaacaacagagaccccatagtgatcagcgactcccccccggcctctccccacaggccccccgcggcgcccatgccaggctccgccccccgccccgggccccccgcgtcctcggccgcgtcgggacccgcgcgcccccgcgcggccgtggccccgtgcgtgcgagcgccgcctccggggcccggcccccgcgccccggcccccggggcggagccggccgcccgccccgcggacgcgcgccgtgtgccccagtcgcactcgtccctggctcaggccgcgaaccaagaacagagtctgtgccgggcgcgtgcgacggtggcgcgcggctcgggggggccgggcgtggagggtgggcacgggccctcccgcggccgcaccccctccggcgccgccccgctcccctccgccgtctctgtcgagcaggaggcggcggtgcgtccgaggaagaggcgcgggtcgggccaggaaaacccctccccccagtccacgcgtccccccctcgcgccggcaggggccaagagggcggcgacgcaccccccctccgactcagggccgggggggcgcggccagggtgggcccgggacccccctgacgtcctcggcggcctccgcctcttcctcctctgcctcttcctcctcggccccgacccccgcgggggccgcctcttccgccgccggggccgcgtcctcctccgcttccgcctcctcgggcggggccgtcggtgccctgggagggagacaagaggaaacctccctcggcccccgcgctgcttctgggccgcgggggccgaggaagtgtgcccggaagacgcgccacgcggagacttccggggccgtccccgcgggcggcctcacgcgctacctgcccatctcgggggtctctagcgtggtcgccctgtcgccttacgtgaacaagactatcacgggggactgcctgcccatcctggacatggagacggggaacatcggggcgtacgtggtcctggtggaccagacgggaaacatggcgacccggctgcgggccgcggtccccggctggagccgccgcaccctgctccccgagaccgcgggtaaccacgtgatgccccccgagtacccgacggcccccgcgtcggagtggaacagcctctggatgacccccgtggggaacatgctgttcgaccagggcaccctagtgggcgccctggacttccgcagcctgcggtctcggcacccgtggtccggggagcagggggcgtcgacccgggacgagggaaaacaataagggacgccccccgtgtttgtggggaggggggtcgggtgctgggtggtctctggccgcgcccactacaccagccaatccgtgtcggggaggggaaagtgaaagacacgggcaccacacaccagcgggtctttagtgttggccctaataaaaaactcaggggatttttgctgtctattgggaaataaaggtttacttttgtatcttttccctgtctgtgttggatggatcttgggggtgcgtgggagtgggggtgcgtgggagtgggggtgcgtgggagtgggggtgcgtgggagtgggggtgcgtgggagtgggggtgcgtgggagtgggggtgcgtgggagtgggggtgcgtgggagtgggggtgcgtgggagtgggggtgcgtgggagtgggggtgcgtgggagtgggggtgcgtgggagtgggggtgcgtgggagtgggggtgccatgttgggcaggctctggtgttaaccacagagccgcggcccgggctgcctgaccaccgatccccgaaagcatcctgccactggcatggagccagaaccacagtgggctgggtgtgggtgttaagtttccgcgagcgcctgcccgcccggactgacctggcctctggccgccacaaagggcggggggggggttaactacactatagggcaacaaaggacgggaggggtggcgggacggggcgcccaaaagggggtcggccacaccacagacgtgggtgttggggggtggggcggaggggtgggggggagacagaaacaggaacatagttagaaaacaagaatgcggtgcagccagagaatcacaggagacgaggggatgggcgtgttggttaccaacccacacccaggcatgctcggtggtatgaaggagggggggcggtgcttcttagagaccgccgggggacgtggggttggtgtgcaaaggcacgcgcacccgcgtcggccaggtgggccggtaccccatccccccctcccccgacccttccccccccgcgtgccagagatcacccccgtcccccggcacccgccactcctccatatcctcgctttaggaacaactttggggggggggtacacacgcgccgtgcatttccttccacaccccccctcccccgcatccccccccccaggcagtaagacccaagcatagagagccaggcacaaaaacacaggcggggtgggacacatgccttcttggagtacgtgggtcattggcgtggggggttacagcgacaccggccgaccccctggcggtcttccagccggcccttagataagggggcagttggtggtcggacgggtaagtaacagagtctgactaagggtgggagggggggaaaagaacgggctggtgtgctgtaacacgagcccacccgcgagtggcgtggccgaccttagcctctggggcgccccctgtcgtttgggtccccccccctctattggggagaagcaggtgtctaacctacctggaaacgcggcgtctttgttgaacgacaccggggcgccctcgacgagtgggataacgggggaggaagggagggaggagggtactgggggtgaagaaggggggggggaagaagcgagaacaggaaaggcgacggagcccggcagaacaccgaggaaaaaaaaaacacagcgcatgcgccgggccgttgtggggccccgggccggggccccttgggtccgccggggccccgggccgggccgccacgggggccggccgttggcggtaaccccgattgtttatctcaggccccgggccgggaacccggaaaagcctccggggggcctttttcgcgtcgcgtgccggcgagcgggcccggacggggcccggaccgccgcggtcgggggcccctcgtcccgggccgtacgcggccttcgccccgtgaggggccgaacgaacgaaacatcccggcgacggaacgaaaaacaccccagacgggtttaaaaaacagaaaccgtaaccccccccacccccgaaacggggaaaacaaaaaacagaccagcggccggccggcgcttagggggaggatgtcgccgacgccccttggccgccccggctgcaggggggcccggagagccgcggcacccggacgcgcccggaaagtctttcgcaccacccgcgatcggcacggccgcgcccccgcttttataaaggctcagatgacgcagcaaaaacaggccacagcaccacgtgggtaggtgatgtaattttattttcctcgtctgcggcctaatggatttccgggcgcggtgcccctgtctgcagagcacttaacggattgatatctcgcgggcacgcgcgcccttaatggaccggcgcggggcggggggccggatacccacacgggcgggggggtgtcgcgggccgtctgctggcccgcggccacataaacaatgactcggggcctttctgcctctgccgcttgtgtgtgcgcgcgccggctctgcggtgtcggcggcggctgcggcggctgcggcggccgccgtgttcggtctcggtagccggccggcgggtggactcgcggggggccggagggtggaaggcaggggggtgtaggatgggtatcaggacttccacttcccgtccttccatcccccgttcccctcggttgttcctcgcctcccccaacaccccgccgctttccgttggggttgttattgttgtcgggatcgtgcgggccgggggtcgccggggcaggggcgggggcgggggtgctcgtcgatcgaccgggctcagtgggggcgtggggtgggtgggaaaaggcgaggagactggggtggggggtgtcgggggtggctgtttttttgtggttgttttttgtgtctgttcccgtcccccgtcacccccctccctccgtccccccgtcgcgggtgtttgtgtttgtttattccgacatcggtttatttaaataaacacagccgttctgcgtgtctgttcttgcgtgtggctgggggcttatatgtggggtcccgggggcgggatggggtttagcggcggggggcggcgcgccggacggggcgctggagataacggcccccggggaacgggggaccggggctgggtctcccgcggtgggtgggtgggcggcggtggccgggccgggccgggccgggtgggcggggtttggaaaaacgaggaggaggagaaggaggaggagggggggggagacggggggaaagcaaggacacggccccgggggggggggagcgcgggccgggccgcttggcaacccccctgtttcttccggaaaccaggcttgtggccccacccgacatcacaagggacctcttgtcgggcctcccgacgtacgccgaggctatgtcggaccaccccccaacctaagaggggagaggggagaggggagaggggagaggggagaggggagaggggaggagagggggtatataaaccaacgaaaagcgcgggaacggggatacggggcttgtgtggcacgacgtcgtggttgtgttactgggcaaacacttggggactgtaggtttctgtggtgccgaccctaggcgctatggggattttgggttgggttgggcttattgccgttggggttttgtgtgtgcgggggggcttgccttcaaccgaatatgttattcggagtcgggtggctcgagaggtgggggatatattaaaggtgccttgtgtgccgctcccgtctgacgatcttgattggcgctacgagaccccctcggctataaactatgctttgatagacggtatatttttgcgttatcactgtcccggattggacacggtcttgtgggataggcacgcccagagggcgtattgggttaacccctttttgtttggggcgggttttttggaggacttgagtcatcccgcgtttcctgccgacacccaggaaacagaaacgcgcttggccctttataaagagatacgccaggcgctggacagtcgcaagcaggccgccagccacacacctgtgaaggctgggtgtgtgaactttgactattcgcgcacccgccgctgtgtagggcgccaggatttgggacttaccaacagaacgtctggacggaccccggttctgccgtcggacgatgaagcgggcctgcagccgaagcccctcaccacgccgtcgcccatcatcgccacgtcggaccccaccccgcgacgggacgccgccacaaaaagcagacgccgacgaccccattcccggcgcatctaatgatgcctcgacggaaaaccgtccgggtttggggggcgaaccggccgcctgtcgctcgtcagggccggcgggcgctcctcgccgccctagaggctgtcccgctggtgtgacgttttcctcgtccgcgccccccgaccctcccatggatttaacaaacgggggggtgtcgcctgcggcgacctcggcgcctctggactggaccacgtttcggcgtgtgtttctgatcgacgacgcgtggcggcccctgttggagcctgagctggcgaaccccttaaccgcccacctcctggccgaatataatcgtcggtgccagaccgaagaggtgctgccgccgcgggaggatgtgttttcgtggactcgttattgcacccccgacgaggtgcgcgtggttatcatcggccaggacccatatcaccaccccggccaggcgcacggacttgcgtttagcgtgcgcgcgaacgtgccgcctcccccgagtcttcggaatgtcttggcggccgtcaagaactgttatcccgaggcacggatgagcggccacggttgcctggaaaagtgggcgcgggacggcgtcctgttactaaacacgaccctgaccgtcaagcgcggggcggcggcgtcccactctagaatcggttgggaccgcttcgtgggcggagttatccgccggttggctgcgcgccgccccggcctggtgtttatgctctggggcgcacatgcccagaatgccatcaggccggaccctcgggtccattgcgtcctcaagttttcgcacccgtcgcccctctccaaggttccgttcggaacatgccagcatttcctcgtggcgaatcgatatctcgagacccggtcgatttcacccatcgactggtcggtttgaaaggcatcgacgtccggggttttcgtctgtgggggcttttgggtatttccgatgaataaagacggttaatggttaaacctctggtctcatacgggtcggtgatgtcgggcgtcgggggagagggagttccctctgcgcttgcgattctagcctcgtggggctggacgttcgacacgccaaaccacgagtcagggatatcgccagatacgactcccgcagattccattcggggggccgctgtggcctcacctgaccaacctttacacgggggcccggaacgggaggccacagcgccgtctttctccccaacgcgcgcggatgacggcccgccctgtaccgacgggccctacgtgacgtttgataccctgtttatggtgtcgtcgatcgacgaattagggcgtcgccagctcacggacaccatccgcaaggacctgcggttgtcgctggccaagtttagcattgcgtgcaccaagacctcctcgttttcgggaaacgccccgcgccaccacagacgcggggcgttccagcgcggcacgcgggcgccgcgcagcaacaaaagccttcagatgtttgtgttgtgcaaacgcgcccacgccgctcgagtgcgagagcagcttcgggtcgttattcagtcccgcaagccgcgcaagtattacacgcgatcttcggacgggcggctctgccccgccgtccccgtgttcgtccacgagttcgtctcgtccgagccaatgcgcctccaccgagataacgtcatgctggcctcgggggccgagtaaccgccccccccccgcgccaccctcactgcccgtcgcgcgtgtttgatgttaataaataacacataaatttggctggttgtttgttgtctttaatggaccgcccgcagggggggtggcatttcagtgtcgggtgacgagcgcgatccggccgggatcctaggaccccaaaagtttgtctgcgtattccagggcggggctcagttgaatctcccgcagcacctctaccagcaggtccgcggtgggctggagaaactcggccgtcccggggcaggcggtcgtcgggagtggaggcgcggcgcccaccccgtgtgccgcgcctggcgtctcctctgggggcgacccgtaaatggttgcagtgatgtaaatggtgtccgcggtccagaccacggtcaaaatgccggccgtggtgctccgggcgctttcgccgcgcgaggagctgacccaggagtcgaacggatacgcgtacatatgggcgtcccacccgcgttcgagcttctggtcgctgtcccggcctataaagcggtaggcacaaaattcggcgcgacagtcgataatcaccaacagcccaatgggggtgtgctggataacaacgcctccgcgcggcaggcggtcctggcgctcccggccccgtaccataatcgcgcgggtgccgtactcaaaaacatgcaccacctgcgcggcgtcgggcagtgcgctggtcagcgaggccctggcgtggcataggctatacgcgatggtcgtctgtggattggacatctcgcggtgggtagtgagtcccccgggccgggttcggtagaactgtaaggggacggcgggttaatagacaatgaccacgttcggatcgcgcagagccgatagtatgtgctcactaatgacgtcatcgcgctcgtggcgctcccggagcggatttaagttcatgcgaaggaattcggaggaggtggtgcgggacatggccacgtacgcgctgttgaggcgcaggttgccgggcgtaaagcagatggcgaccttgtccaggctaaggccctgggagcgcgtgatggtcatggcaagcttggagctgatgccgtagtcggcgtttatggccatggccagctccgtagagtcaatggactcgacaaactcgctgatgttggtgttgacgacggacatgaagccgtgttggtcccgcaagaccacgtaaggcaggggggcctcttccagtaactcggccacgttggccgtcgcgtgccgcctccgcagctcgtccgcaaaggcaaacacccgtgcgtacgtgtatcccatgagcgtataattgtccgtctgcagggcgacggacatcagccccccgcgcggcgagccggtcagcatctcgcagccccggaagataacgttgtccacgtacgtgctaaagggggcgccttcaaatgcctccccgaagagctcttggaggattcggaatctcccgaggaaggcccgcttcagcagcgcaaactgggtgtgaacggcggcggtggtctccggttccccgggggtgtagtggcagtaaaacacgtcgagctgttgttcgtccagccccgcgaaaataacgtcgaggtcgtcgtcgggaaaatcgtccgggcccccgtcccgcggccccagttgcttaaaatcaaacgcacgctcgccgggggcgcctgcgtcggctattaccgacgcctgcgtcggcgcccccgaagatttggggcgcagagacagaatctccgccgttagttctcccatgcgggcgtaggcgagggtcctctgggtcgcatccaggcccgggcgctgcagaaagttgtaaaaggagataagcccgctaaatatgagccgcgacaggaacctgtaggcaaactccaccgaagtctccccctgagtctttacaaagctgtcgtcacgcaacactgcctcgaaggcccggaacgtcccactaaacccaaaaaccagttttcgcaggcgcgcggtcaccgcgatctggctgttgaggacgtaagtgacgtcgttgcgggccacgaccagctgctgtttgctgtgcacctcgcagcgcatgtgccccgcgtcctggtcctggctctgcgagtagttggtgatgcggctggcgttggccgtgagccacttttcaatagtcaggccgggctggtgtgtcagccgtcggtattcgtcaaactccttgaccgacacgaacgtaagcacggggagggtgaacacgacgaactccccctcacgggtcaccttcaggtaggcgtggagcttggccatgtacgcgctcacctctttgtgggaggagaacagccgcgtccagccggggaggttggcggggttggtgatgtagctttccgggacgacgaagcgatccacgaactgcatgtgctcctcggtgatgggcaggccgtactccagcaccttcatgaggttaccgaactcgtgctcgacgcaccgtttgttgttaataaaaatggcccagctatacgagaggcgggcgtactcgcgcagcgtgcggttgcagatgaggtacgtgagcacgttctcgctctggcggacggaacaccgcagtttctggtgctcgaaggtcgactccagggacgccgtctgcgtcggcgagcccacacacaccaacacgggccgcaggcgggccgcatactggggggtgtggtacagggcgttaatcatccaccagcaatacaccacggccgtgaggaggtgacgcccaaggagcccggcctcgtctatgacgatcacgttgctgcgggtaaaggccggcagcgccccgtgggtggccggggccaaccgcgtcagggcgccctcggccaaccccagggtccgttccagggcggccagggcgcgaaactcgttccgcgactcctcgcccccggaggcggccagggcgcgcttcgtgaggtccaaaatcacctcccagtagtacgtcagatctcgtcgctgcaggtcctccagcgaggcggggttgctggtcagggtgtacgggtactgtcccagttgggcctggacgtgattcccgcgaaacccaaattcatgaaagatggtgttgatgggtcggctgagaaaggcgcccgagagtttggcgtacatgttttgggccgcaatgcgcgtggcgcccgtcaccacacagtccaagacctcgttgattgtctgcacgcacgtgctctttccggagccagcgttgccggtgataagatacaccgcgaacggaaactccctgaggggcaggcctgcgggggactctaaggccgccacgtcccggaaccactgcagacggggcacttgcgctccgtcgagctgttgttgcgagagctctcggatgcgcttaaggattggctgcaccccgtgcatagacgtaaaatttaaaaaggcctcggccctccctggaacggctggtcggtccccgggttgctgaaggtgcggcgggccgggtctctgtccgtctagctggcgctccccgccggccgccgccatgaccgcaccacgctcgcgggcccccactacgcgtgcgcggggggacacggaagcgctgtgctcccccgaggacggctgggtaaaggttcaccccacccccggtacgatgctgttccgtgagattctccacgggcagctggggtataccgagggccagggggtgtacaacgtcgtccggtccagcgaggcgaccacccggcagctgcaggcggcgatctttcacgcgctcctcaacgccaccacttaccgggacctcgaggcggactggctcggccacgtggcggcccgcggtctgcagccccaacggctggttcgccggtacaggaacgcccgggaggcggatatcgccggggtggccgagcgggtgttcgacacgtggcggaacacgcttaggacgacgctgctggactttgcccacgggttggtcgcctgctttgcgccgggcggcccgagcggcccgtcaagcttccccaaatatatcgactggctgacgtgcctggggctggtccccatattacgcaagcgacaagaagggggtgtgacgcagggtctgagggcgtttctcaagcagcacccgctgacccgccagctggccacggtcgcggaggccgcggagcgcgccggccccgggttttttgagctggcgctggccttcgactccacgcgcgtggcggactacgaccgcgtgtatatctactacaaccaccgccggggcgactggctcgtgcgagaccccatcagcgggcagcgcggagaatgtctggtgctgtggcctcccttgtggaccggggaccgtctggtcttcgattcgcccgtccagcggctgtttcccgagatcgtcgcgtgtcactccctccgggaacacgcgcacgtctgccggctgcgcaataccgcgtccgtcaaggtgctgctggggcgcaagagcgacagcgagcgcggggtggccggcgccgcgcgggtcgttaacaaggtgttgggggaggacgacgagaccaaggccgggtcggccgcctcacgcctcgtgcggcttatcatcaacatgaagggcatgcgccacgtaggcgacattaacgacaccgtgcgtgcctacctcgacgaggccggggggcacctgatagacgccccggccgtcgacggtaccctccctggattcggcaagggcggaaacagccgcgggtctgcgggccaggaccagggggggcgggcgccgcagcttcgccaggccttccgcacggccgtggttaacaacatcaacggcgtgttggagggctatataaataacctgtttggaaccatcgagcgcctgcgcgagaccaacgcgggcctggcgacccaattgcaggagcgcgaccgcgagctccggcgcgcaacagcgggggccctggagcgccagcagcgcgcggccgacctggcggccgagtccgtgaccggtggatgcggcagccgccctgcgggggcggacctgctccgggccgactatgacattatcgacgtcagcaagtccatggacgacgacatgtacgtcgccaacagctttcagcacccgtacatcccttcgtacgcccaggacctggagcgcctgtcgcgcctctgggagcacgagctggtgcgctgttttaaaattctgtgtcaccgcaacaaccagggccaagagacgtcgatctcgtactccagcggggcgatcgccgcattcgtcgccccctactttgaggcagtgcttcgggccccccgggtaggcgcgcccatcacgggctccgatgtcatcctgggggaggaggagttatgggatgcggtgtttaagaaaacctgcctgcaaacgtacctgacagacatcgcggccctgttcgtcgcggacgtccagcacgcagcgctgcccccgcccccctccccggtcggcgccgatttccggcccggcgcgtccccgcggggccggtccagatcgcggtcgcccggaagaactgcgcgaggcgcaccggaccagggcgggggcatcgggcaccgggatggccgccgcgacggccgacgatgaggggtcggccgtcaccatcctcaagcaggccatcgccggggaccgcagcctggtcgaggcggccgaggcgattagccagcagacgctgctccgcctggcctgcgaggtgcgccaggtcggcgaccgccagccgcggtttaccgccaccagcatcgcgcgcgtcgacgtcgcgcctgggtgccggttgcggttcgttctggacgggagtcccgaggacgcctatgtgacgtcggaggattactttaagcgctgctgcggccagtccagttatcgcggcttcgcggtggcggtcctgacggccaacgaggaccacgtgcacagcctggccgtgccccccctcgttctgctgcaccggttctccctgttcaaccccagggacctcctggactttgagcttgcctgtctgctgatgtacctggagaactgcccccgaagccacgccaccccgtcgacctttgccaaggttctggcgtggctcggggtcgcgggtcgccgcacgtccccattcgaacgcgttcgctgccttttcatccgcagttgccactgggtcctaaacacactcatgttcatggtgcacgtaaaaccgttcgacgacgagttcgtcctgccccactggtacatggcccggtacctgctggccaacaacccgccccccgttctctcggccctgttctgtgccaccccgacgagctcctcattccggctgccggggccgcccccccgctccgactgcgtggcctataaccccgccgggatcatggggagctgctgggcgtcggaggaggtgcgcgcgcctctggtctattggtggctttcggagaccccaaaacgacagacgtcgtcgctgttttatcagttttgttgaattttagtaaataaacccggttttgtttctatggcctcctgacggatgcgcgtgtccttactccgttttggtgggtgggtggctgtgtatggcgtcccatctgtgcggggagggggcaagtcggcacgtattcggacagactcaagcacacacgggggagcgctcttggctcagggcaatgtttttattggtcaaactcaggcaaacagaaacaacatcttgtcgtcaaagggatacacaaacttccccccctcgccccatactcccgccagcaccccggtaaacaccaactcaatctcgcgcaggatttcgcgcaggtgatgagcgcagtccacgggggggagcacaaggggccgcgggtatagatcgacggggacgccgaccgactccccgcctccgggacagacacgcacgacgcgccgccagtagtgctctgcgtccaacaaggcgccgccgcggaaggcagtggggggcaaggggtcgctggcctcaaagggggacacccgaacgctccagtactccgcgtccaaccgtttattaaacgcgtccacgataaggcggtcgcaggcgtcctccataaggccccgggccgtgagcgcgtcctcctccggcacgcctgccgttgtcaggcccaggacccgtcgcagcgtgtcgcgtacgaccccggccgccgtggtgtacgcgggcccgcggagaggaaatcccccaagatggtcagtgttgtcgcgggagttccagaaccacactcccgcttggctccaggcgacggcgtgggtgtagacgccctcgagcgccaggcacagtgggtgccgcagccggaggccgttggccataagcacggctcccacggccgtctcgatggcccgccgggcgtcctcgatcaccccggaagccgcatccgcgtcttgggggtccacgttaaagacaccccagaacgcacccccatcgcccccgcagaccgcgaacttaaccgagctggccgtctcctcaatctgcaggcagacggcggccatcaccccgcccaggagctgccgcagcgcagggcaggcgtcgcacgtgtccgggaccaggcgctccaagacggccccggcccagggctctgagggagcggccaccaccagcgcgtccagtcttgctaggcccgtccggccgtggggttccgccagcccgctccccccgaggtcggccagggccgccaggagctgggcgcgaagtccggggaagcaaaaccgcgccgtccagacgggcccgacggccgcgggcgggtctaacagttggatgattttagtggcgggatgccaccgcgccaccgcctcccgcaccgcgggcaggaggcatccggctgccgccgaggccacgccgggccaggctcgcggggggaggacgaccctggcccccaccgcgggccaggcccccaggagcgcggcgtaagcggccgcggccccgcgcaccaggtcccgtgccgactcggccgtggccggcacggtgaacgtgggccaacccggaaaccccaggacggcaaagtacgggacgggtcccccccggacctcaaactcgggccccagaaaggcaaagacgggggccagggccccgggggcggcgtggaccgtggtatgccactgccggaaaagggcgacgagcgccggcgcggagaacttctcgccggcgcttacaaagtagtcgtaatcgcggggcagcagcacccgtgccgtgactcgttgcgggtgcccgcgtggccgcaggcccacctcgcacacctcgaccaggtccccgaacgctccctccttcttgatcggcggaaacgcaagagtctggtattcgcgcgcaaatagcgcggttccggtggtgatgttaacggtcagcgaagcggcggacgcgcactggggggtgtcgcgaatggccgccaggcgcgcccacgccagccgcgcgtcgggatgctcggcaacgcgcgccgccagggccatagggtcgatgtcaatgttggcctccgcgaccaggagagcggcgcgaggggcggcgggcgggccccacgacgctctctcaactttcaccaccagtcccgtgcgtgggtccgagccgatacgcagcggggcgaacagggccaccggcccggtctggcgctccagggccgccaggacgcacgcgtacagcgcccgccacagagtcgggttctccaggggctccagcggggaggcggccggcgtcgtcgcggcgcgggcggccgccacgacggcctggacggagacgtccgcggagccgtagaaatcccgcagctccgtcgcggtgacggagacctccgcaaagcgcgcgcgaccctcccctgcggcgttgcgacatacaaaatacaccagggcgtggaagtactcgcgagcgcgggggggcagccataccgcgtaaagggtaatggcgctgacgctctcctccacccacacgatatctgcggtgtccatcgcacggcccctaaggatcacgggcggtctgtgggtcccatgctgccgtgcctggccgggcccggtgggtcgcggaaaccggtgacgggggggggcggtttttggggttggggtgggggtgggaaacggcccgggtccgggggccaacttggcccctcggtgcgttccggcaacagcgccgccggtccgcggacgaccacgtaccgaacgagtgcggtcccgagacttatagggtgctaaagttcaccgccccctgcatcatgggccaggcctcggtggggagctccgacagcgccgcctccaggatgatgtcagcgttggggttggcgctggatgagtgcgtgcgcaaacagcgcccccacgcgggcacgcgtagcttgaagcgcgcgcccgcaaactcccgcttgtgggccataagcagggcgtacagctgcctgtgggtccggcaggcgctgtggtcgatgtggtgggcgtccaacaaccccacgattgtctgtttggtgaggtttttaacgcgccccgccccgggaaacgtctgcgtgcttttggccatctgcacgccaaacagttcgccccagattatcttgaacagcgccaccgcgtggtccgtctcgctaacggacccgcgcgggggacagccgcttagggcgtcggcgacgcgcttgacggcttcctccgagagcagaagtccgtcggttacgttacagtggcccagttcgaacaccagctgcatgtagcggtcgtagtggggggtcagtaggtccagcacgtcatcggggccgaaggtcctcccagatcccccggccgccgagtcccaatgcaggcgcgcggccatggtgctgcacaggcacaacagctcccagacgggggttacgttcagggtggggggcagggccacgagctccagctctccggtgacgttgatcgtggggatgacgcccgtggcgtagtggtcatagatccgccgaaatatggcgctgctgcgggtggccatgggaacgcggagacaggcctccagcaacgccaggtaaataaaccgcgtgcgtcccatcaggctgttgaggttgcgcatgagcgcgacaatttccgccggcgcgacatcggaccggaggtatttttcgacgaaaagacccacctcctccgtctcggcggcctgggccggcagcgacgcctcgggatcccggcaccgcagctcccgtagatcgcgctgggccctgagggcgtcgaaatgtacgccccgcaaaaacagacagaagtcctttggggtcagggtatcgtcgtgtccccagaagcgcacgcgtatgcagtttagggtcagcagcatgtgaaggatgttaaggctgtccgagagacacgccagcgtgcatctctcaaagtagtgtttgtaacggaatttgttgtagatgcgcgacccccgccccagcgacgtgtcgcatgccgacgcgtcacagcgccccttgaaccggcgacacagcaggtttgtgacctgggagaactgcgcgggccactggccgcaggaactgaccacgtggttcaggagcatgggcgtaaagacgggctccgagcgcgccccggagccgtccatgtaaatcagtagctcccccttgcggagggtgcgcacccgtcccagggactggtacacggacaccatgtccggtccgtagttcatgggtttcacgtaggcgaacatgccatcaaagtgcaggggatcgaagctgaggcccacggttacgaccgtcgtgtatataaccacgcggtattggccccacgtggtcacgtccccgaggggggtgagcgagtgaagcaacagcacgcggtccgtaaactgacggcagaaccgggccacgatctccgcgaaggagaccgtcgatgaaaaaatgcagatgttatcgcccccgccaaggcgcgcttccagctccccaaagaacgtggccccccgggcgtccggagaggcgtccggagacgggccgcttggcggcccgggcgggcgcagggcagcctgcaggagctcggtccccagacgcgggagaaacaggcaccggcgcgccgaaaacccgggcatggcgtactcgccgaccaccacatgcacgtttttttcgccccggagaccgcacaggaagtccaccaactgcgcgttggcggttgcgtccatggcgatgatccgaggacaggtgcgcagcaggcgtagcattaacgcatccacgcggcccagttgctgcatcgttggcgaatagagctggcccagcgtcgacataacctcgtccagaacgaggacgtcgtagttgttcagaaggttggggcccacgcgatgaaggctttccacctggacgataagtcggtggaaggggcggtcgttcataatgtaattggtggatgagaagtaggtgacaaagtcgaccaggcctgactcagcgaaccgcgtcgccagggtctgggtaaaactccgacgacaggagacgacgagcacactcgtgtccggagagtggatcgcttcccgcagccagcggatcagcgcggtagtttttcccgaccccattggcgcgcggaccacagtcacgcacctggccgtcggggcgctcgcgttggggaaggtgacgggtccgtgctgctgccgctcgatcgttgttttcgggtgaacccggggcacccattcggccaaatcccccccgtacaacatccgcgctagcgatacgctcgacgtgtactgttcgcactcgtcgtccccaatgggacgcccggcccccagaggatcccccgactccgcgccccccacgaaaggcatgaccggggcgcggacggcgtggtgggtctggtgtgtgcaggtggcgacgtttgtggtctctgcggtctgcgtcacggggcttctcgtcctggcctctgtgttccgggcacggtttccctgcttttatgccacggcgagctcttatgccggggtgaactccacggccgaggtgcgcgggggtgtagccgtgcccctcaggttggacacgcagagccttgtgggcacttatgtaatcacggccgtgttgttgttggccgcggccgtgtatgccgtggtcggcgccgtgacctcccgctacgaccgcgccctggacgcgggccgccgtctggctgcggcccgcatggccatgccgcacgccacgctgatcgccggaaacgtctgctcttggttgctgcagatcaccgtcctgttgctggcccatcgcatcagccagctggcccacctggtttacgtcctgcactttgcgtgtctggtgtattttgcggcccatttttgcaccaggggggtcctgagcgggacgtatctgcgtcaggtgcacggcctgatggagccggccccgactcatcatcgcgtcgtcggcccggctcgagccgtgctgacaaacgccttgctgttgggcgtcttcctgtgcacggccgacgccgcggtatccctgaataccatcgccgcgttcaactttaatttttcggccccgggcatgctcatatgcctgaccgtgctgttcgcccttctcgtcgtatcgctgttgttggtggtcgagggggtgttgtgtcactacgtgcgcgtgttggtgggcccccacctgggggccgtggccgccacgggcatcgtcggcctggcctgcgagcactattacaccaacggctactacgttgtggagacgcagtggccgggggcccagacgggagtccgcgtcgccctcgccctggtcgccgcctttgccctcggcatggccgtgctccgctgcacccgcgcctatctgtatcacaggcggcaccacaccaaattttttatgcgcatgcgcgacacgcgacaccgcgcacattccgccctcaggcgcgtacgcagttccatgcgcggatcgcgagacggccgccacaggcccgcacccggcagcccgcccgggattcccgaatatgcggaagacccctacgcgatctcatacggcggccagctcgaccggtacggagattccgacggggagccgatttacgacgaggtggctgacgaccaaaccgacgtattgtacgccaagatacaacacccgcggcacctgcccgacgacgagcccatctatgacaccgttggggggtacgaccccgagcccgccgaggaccccgtgtacagcaccgtccgccgttggtagctgtttggttccgttttaataaaccgtttgtgtttaacccgaccgtggtgtatgtctggtgtgtggcgtccgatcccgttactatcaccgtttcccccccccccccctcaaccccggcgattgtgggttttttaaaaacgacacgcgtgcgaccgtatacagaacattgttttggtttttattcgctatcggacatggggggtggaaactgggtggcggggcaggcgcctccgggggtccgccggtgagtgtggcgcgagggggggtccgacgaacgcaggcgctgtctccccggggcccgcgtaaccacgcgcatatccgggggcacgtagaaattaccttcctcttcggactcgatatccacgacatcaaagtcgtgggcggtcagcgagacgacctccccgtcgtcggtgatgaggacgttgtttcggcagcagcagggccgggccccggagaacgagaggcccatagctcggcgagcgtgtcgtcgaacgccaggcggctgcttcgctggatggccttatagatctccggatcgatgcggacgggggtaatgatcagggcgatcggaacggcctggttcgggagaatggacgccttgctgggtcctgcggccccgagagccccggcgccgtcctccaggcggaacgttacgccctcctccgcgctggtgcggtgcctgccgataaacgtcaccagatgcgggtggggggggcagtcggggaagtggctgtcgagcacgtagccctgcaccaagatctgcttaaagttcgggtgacgggggttcgcgaagacgggctcgcggcggaccagatccccggagctccaggacacgggggagatggtgtggcgtccgaggtcgggggcgccaaacagaagcacctccgagacaacgccgctatttaactccaccaaggcccgatccgcggcggagcaccgccttttttcgcccgaggcgtgggcctctgaccaggcctggtcttgcgtgacgagagcctcctccgggccggggacgcgcccgggcgcgaagtatcgcacgctgggcttcgggatcgaccggataaatgcccggaacgcctccggggaccggtgtgtcatcaagtcctcgtacgcggaggccgtggggtcgctggggtccatggggtcgaaagcgtacttggcccggcatttgacctcgtaaaaggccaggggggtcttggggactggggccaggtagccgtgaatgtcccgaggacagacgagaatatccagggacgccccgaccatccccgtgtgaccgtccatgaggaccccacacgtatgcacgttctcttcggtgaggtcgctgggttcgtggaagataaagcgccgcgtgtcggcgccggcctcgccgccgtcgtccgcgcggcccacgcagtagcgaaacagcaggcttcgggccgtcggctcgttcacccgcccgaacatcaccgccgaagactgtacatccggccgcaggctggcgttgtgcttcagccactggggcgagaaacacggaccctgggggccccagcggagggtggatgcggtcgtgaggccccgccggagcagggcccatagctggcagtcggcctggttttgcgtggccgcctcgtaaaaccccatgaggggccggggcgccacggcgtccgcggcggccgggggcccgcggcgcgtcaggcgccataggtgccggccgagtccgcggtccaccatacccgcctcctcgaggaccacggccagggaacacagataatccaggcgggcccagaggggaccgatggccagaggggcgcggacgccgcgcagcaacccgcgcaggtggcgctcgaacgtctcggctagtatatgggagggcagcgcgttggggatcaccgacgccgaccacatagagtcaaggtccggggagtcgggatcggcgtccgggtcgcgggcgtgggtgcccccaggagatagcggaatgtctggggtcggaggccctgaggcgtcagaaagtgccggcgacgcggcccggggcttttcgtctgcggtgtcggtggcgtgctgatcacgtggggggttaacgggcgaatgggagctcgggtccacagctgacgtcgtctggggtggggggggcaggggacggaaggtggttgtcagcggaagactgttagggcgggggcgcttgggggggctgtcggggccacgaggggtgtcctcggccagggcccagggacgcttagtcacggtgcgtcccggcggacatgctgggcctaccgtggactccatttccgagacgacgtgggggagcggtggttgagcgcgccgccgggtgaacgctgattctcacgacagcgcgtgccgcgcgcacgggttggtgtgacacaggcgggacaccagcaccaggagaggcttaagctcgggaggcagcgccaccgacgacagtatcgccttgtgtgtgtgctggtaatttatacaccgatccgtaaacgcgcgccgaatcttgggattgcggaggtggcgccggatgccctctggtacgtcatacgccaggccgtgggtgttggtctcggccgagttgacaaacagggctgggtgcagcacgcagcgataggcgagcagggccagggcgaagtccggcgacagctggttgttgaaatactggtaaccgggaaaccgggtcacgggtacgcccaggctcggggcgacgtacacgctaaccaccaactccagcagcgtctggccaagggcgtacaggtcaaccgctaacccgacgtcgtgcttcaggcggtggttggtaaattcggcccgttcgttgttaaggtatttcaccaacagctccgggggctggttatacccgtgacccaccagggtgtgaaagttggctgtggttagggcggtgggcatgccaaacatccggggggacttgaggtccggctcctggaggcaaaactgcccccgggcgatcgtggagttggagttgagggtgacgaggctaaagtcggcgaggacggcccgccggagcgagacggcgtccgaccgcagcatgacgaggatgttggcgcacttgatatccaggtggctgatcccgcaggtggtgtttaaaaacacaacggcgcgggccagctccgtgaagcactggtggagggccgtcgagaccgaggggtttgttgtgcgcagggacgccagttggccgatatacttaccgaggtccatgtcgtacgcggggaacactatctgtcgttgttgcagcgagaacccgaggggcgcgatgaagccgcggatgttgtgggtgcggccggcgcgtagagcgcactccccgaccaacagggtcgcgatgagctcaacggcaaaccactccttttcctttatggtcttaacggcaagcttatgttcgcgaatcagttggacgtcgccgtatcccccagaccccccgaagcttcgggccccggggatctcgagggtcgtgtagtgtagggcggggttgatggcgaacacggggctgcatagcttgcggatgcgcgtgagggtaaggatgtgcgagggggacgaggggggtgcggttaacgccgcctgggatctgcgcaggggcgggcggttcagtttggccgccgtaccgggcgtctcgggggacgcgcggcgatgagacgagcggctcattcgccatcgggatagtcccgcgcgaagccgctcgcggaggccggatcggtggcgggacccgtgggaggagcgggagccggcggcgtcctggagagaggggccgctggggcgcccggaggccccgtgtgggttggagtgtatgtaggatgcgagccaatccttgaaggaccgttggcgtgcaccttgggggctgaggttagctgccacatgaccagcaggtcgctgtctgcgggactcatccatccttcggccaggtcgccgtctccccacagagaagcgttggtcgctgcttcctcgagttgctcctcctggtccgcaagacgatcgtccacggcgtccaggcgctcaccaagcgccggatcgaggtaccgtcggtgtgcggttagaaagtcacgacgcgccgcttgctcctccacgcgaattttaacacaggtcgcgcgctgtcgcatcatctctaagcgcgcgcgggactttagccgcgcctccaattccaagtgggccgcctttgcagccataaaggcgccaacaaaccgaggatcttgggtgctgacgccctcccggtgcagctgcagggtctggtccttgtaaatctcggctcggaggtgcgtctcggccaggcgtcggcgcagggccgcgtgggcggcatctcggtccattccgccaccctgcgggcgacccggggggtgctctgatagtctcgcgtgcccaaggcccgtgatcggggtacttcgccgccgcgacccgccacccggtgtgcgcgatgtttggtcagcagctggcgtccgacgtccagcagtacctggagcgcctcgagaaacagaggcaacttaaggtgggcgcggacgaggcgtcggcgggcctcacaatgggcggcgatgccctacgagtgccctttttagatttcgcgaccgcgacccccaagcgccaccagaccgtggtcccgggcgtcgggacgctccacgactgctgcgagcactcgccgctcttctcggccgtggcgcggcggctgctgtttaatagcctggtgccggcgcaactaaaggggcgtgatttcgggggcgaccacacggccaagctggaattcctggcccccgagttggtacgggcggtggcgcgactgcggtttaaggagtgcgcgccggcggacgtggtgcctcagcgtaacgcctactatagcgttctgaacacgtttcaggccctccaccgctccgaagcctttcgccagctggtgcactttgtgcgggactttgcccagctgcttaaaacctccttccgggcctccagcctcacggagaccacgggcccccccaaaaaacgggccaaggtggacgtggccacccacggccggacgtacggcacgctggagctgttccaaaaaatgatccttatgcacgccacctactttctggccgccgtgctcctcggggaccacgcggagcaggtcaacacgttcctgcgtctcgtgtttgagatccccctgtttagcgacgcggccgtgcgccacttccgccagcgcgccaccgtgtttctcgtcccccggcgccacggcaagacctggtttctagtgcccctcatcgcgctgtcactggcctcctttcgggggatcaagatcggctacacggcgcacatccgcaaggcgaccgagccggtgtttgaggagatcgacgcctgcctgcggggctggttcggttcggcccgagtggaccacgttaaaggggaaaccatctccttctcgtttccggacgggtcgcgcagtaccatcgtgtttgcctccagccacaacacaaacgtaagtcctcttttctttcgcatggctctcccaaggggccccgggtcgacccgacccacacccacccacccacccacatacacacacaaccagacgcgggaggaaagtctgccccgtgggcactgatttttattcgggatcgcttgaggaggcccgggcaacggcccgggcaacggtggggcaactcgtagcaaataggcgactgatgtacgaagagaagacacacaggcgccacccggcgctggtcggggggatgttgtccgcgccgcaccgtcccccgacgacctcttgcagacggtccgtgatgcaaggacggcggggggcctgcagcagggtgaccgtatccacgggatggccaaagagaagcggacacaggctagcatccccctggaccgccagggtacactgggccatcttggcccacagacacggggcgacgcagggacaggactccgttacgacggaggagagccacagtgcgttggcggaatcgatgtggggcggcggggcgcaggactcgcagccccccgggtggttggtgatcctggccaggagccatcccagatggcgggccctgcttcccggtggacagagcgaccccaggtcgctgtccatggcccagcagtagatctggccgctggggaggtgccaccaggcccccgggcccaaggcgcagcacgcgcccggctccgggggggtcttcgcggggaccagatacgcgccatccagctcgccgaccactggctcctccgcgagctgttcggtggttgggtcgggggtttcctccgggggggtggccgcccgtatgcgggcgaacgtgagggtgcacaggagcggggtcagggggtgcgtcacgctccggaggtggacgatcgcgcagtagcggcgctcgcggttaaagaaaaagagggcaaagaaggtgttcgggggcaaccgcagcgccttggggcgcgtcagatacagaaaaatctcgcagaagagggcgcgcccggggtctgggttaggaagggccacctgacacagaggctcggtgaggaccgttagacaccgaaagatcttgagccgctcgtccgcccgaacgacgcgccacacaaagacggagttgacaatgcgcgcgatagagtcgacgtccgtccccaggtcgtcgactctgtcgcgcgtgccgcgagctccggcccgggaatccggccggggcaaggtccccgggggaccaggcggcgccaggggccgccggggtcccagctgcgccatgccgggggcggggggagggcaaaccccagaggcgggggccaacggcgcggggaggagtgggtgggcgaggtggccgggggaaggcgcccgctagcgagaacggccgttcccggacgacaccttgcgacaaaacctaaggacagcggcccgcgcgacggggtccgagaggctaaggtaggccgcgatgttaatggtgaacgcaaagccgccgggaaagacaactatgccacagaggcggcgattaaaccccaggcagaggtaggcgtagctttccccgggcaggtattgctcgcagaccctgcgtggggctgtggaggggacggcctccatgaagcgacatttactctgctcgcgtttactgacgtcaccatccatcgccacggcgattggacgattgttaagccgcagcgtgtctccgcttgtgctgtagtagtcaaaaacgtaatggccgtcggagtcggcaaagcgggccgggaggtcgtcgccgagcgggacgacccgccgcccccgaccgccccgtccccccaggtgtgccaggacggccagggcatacgcggtgtgaaaaaaggagtcgggggcggtcccctcgacggcgcacatcaggttctcgaggagaatggggaagcgcctggtcacctcccccaaccacgcgcgttggtcggggccaaagtcatagcgcaggcgctgtgagattcgcgggccgccctgaagcgcggcccggatggcctggcccagggcccggaggcacgccagatgtatgcgcgcggtaaaggcgacctcggcggcgatgtcaaagggcggcaggacggggcgcgggtggcgcaggggcacctcgagcgcgggaaagcgtagcagcagctccgcctgcccagcgggagacagctggtgggggcgcacgacgcgttctgcggcgcaggcctcggtcagggccgtggccagcgccgaggacagcagcggagggcgggcgcgtcgcccgccccacgccacggagttctcgtaggagacgacgacgaagcgctgcttggttccgtagtggtggcgcaggaccacggagatagaacgacggctccacagccagtccggccggtcgccgccggccagggcttcccatccgcgatccaaccactcgaccagcgaccgcggctttgcggtaccaggggtcagggttagaacgtcgttcaggatgtcctcgcccccgggcccgtggggcacgggggccacaaagcggcccccgcctgggggctccagacccgccaacaccgcatctgcgtcagccgcccccatggcgcccccgctgacggcctggtgaaccagggcgccctggcggagccccgatgcaacgccacaggccgcacgcccggtccgagcgcggaccgggtggcggcgggtgacgtcctgcactgcccgctgaaccaacgcgaggatctcctcgttctcctgcgcgatggacacgtcctgggccgcggtcgtgtcgccgccgggggccgtcagctgctcctccggggagatgggggggtcggacgccccgacgatgggcgggtctgcgggcgcccccgcgtggggccgggccaagggctgcggacgcggggacgcgctttcccccagacccatggacaggtgggccgcagcctccttcgcggccggcggggcggcggcgccaagcagagcgacgtagcggcacaaatgccgacagacgcgcatgatgcgcgtgctgtcggccgcgtagcgcgtgttgggggggacgagctcgtcgtaactaaacagaatcacgcgggcacagctcgcccccgagccccacgcaaggcgcagcgccgccacggcgtacgggtcatagacgccctgcgcgttacacaccacgggcagggagacgaacaaccccccggcgctggacgcacgcggaaggaggccagggtgtgccggcacgacgggggccagaagctcccccaccgcatccgcgggcacgtaggcggcaaacgccgtgcaccacggggtacagtcgccggtggcatgagcccgagtctggatttcgacctggaagtttgcggccgtcccgagtccggggtggccgcgcatcagggcggccagagggattcccgcggccgccaggcactcgctggatatgatgacgtgaaccaaagacgagggccgacccgggccgtggccgagatcgtactggacctcgttggccaagtgcgcgttcatggttcgggggtgggtgtgggtgtgtaggcgatgcgggtcccccgagtccgcgggaagggcgtgggtttggcgcgcgtatgcgtattcgccaacggaggcgtgcgtgcttatgcgcggcgcgtttcttctgtctctagggaatccgaggccaggactttaacctgctctttgtcgacgaggccaactttattcgcccggatgcggtccagacgattatgggctttctcaaccaggccaactgcaagattatcttcgtgtcgtccaccaacaccgggaaggccagtacgagctttttgtacaacctccgcggggccgcagacgagcttctcaacgtggtgacctatatatgcgatgatcacatgccgagggtggtgacgcacacaaacgccacggcctgttcttgttatatcctcaacaagcccgttttcatcacgatggacggggcggttcgccggaccgccgatttgtttctggccgattccttcatgcaggagatcatcgggggccaggccagggagaccggcgacgaccggcccgttctgaccaagtctgcgggggagcggtttctgttgtaccgcccctcgaccaccaccaacagcggcctcatggcccccgatttgtacgtgtacgtggatcccgcgttcacggccaacacccgagcctccgggaccggcgtcgctgtcgtcgggcggtaccgcgacgattatatcatcttcgccctggagcacttttttctccgcgcgctcacgggctcggcccccgccgacatcgcccgctgcgtcgtccacagtctgacgcaggtcctggccctgcatcccggggcgtttcgcggcgtccgggtggcggtcgagggaaatagcagccaggactcggccgtcgccatcgccacgcacgtgcacacagagatgcaccgcctactggcctcggagggggccgacgcgggctcgggccccgagcttctcttctaccactgcgagcctcccgggagcgcggtgctgtacccctttttcctgctcaacaaacagaagacgcccgcctttgaacactttattaaaaagtttaactccgggggcgtcatggcctcccaggagatcgtttccgcgacggtgcgcctgcagaccgacccggtcgagtatctgctcgagcagctaaataacctcaccgaaaccgtctcccccaacactgacgtccgtacgtattccggaaaacggaacggcgcctcggatgaccttatggtcgccgtcattatggccatctacctcgcggcccaggccggacctccgcacacattcgctcctatcacacgcgtcttgtgagcgcccaataaacacacccaggtatgctacgcacgaccacggtgtcgtctgttaaggggggggggaagggggtgttggcgggaagcgtgggaacacgggggattctctcacgaccggcaccagtaccacccccctgtgaacacagaaaccccaacccaaatcccataaacatacgacacacaggcatattttggaatttcttaggtttttatttatttaggtatgctggggtttctccctggatgcccacccccacccccccgtgggtctagccgggccttagggatagcgtataacgggggccatgtctccggaccgcacaacggccgcgccgtcaaaggtgcacacccgaaccacgggagccagggccaaggtgtctcctagttggcccgcgtgggtcagccaggcgacgagcgcctcgtaaagcggcagccttcgctctccatcctgcatcagggccggggcttcggggtgaatgagctgggcggcctcccgcgtgacactctgcatctgcaggagagcgttcacgtacccgtcctgggcacttagcgcaaagagccgggggattagcgtaaggatgatggtggttccctccgtgatcgagtaaaccatgttaaggaccagcgatcgcagctcggcgtttacgggaccgagttgttggacgtccgccagcagcgagaggcgactcccgttgtagtacagcacgttgaggtctggcagccctccggggtttctggggctggggttcaggtcccggatgcccctggccacgagccgcgccacgatttcgcgcgccaggggcgatggaagcggaacgggaaaccgcaacgtgaggtccagcgaatccaggcgcacgtccgtcgcttggccctcgaacacgggcgggacgaggctgatggggtccccgttacagagatctacgggggaggtgttgcgaaggttaacggtgccggcgtgggtgaggcccacgtccagggggcaggcgacgattcgcgtgggaagcacccgggtgatgaccgcggggaagcgccttcggtacgccagcaacaaccccaacgtgtcgggactgacgcctccggagacgaaggattcgtgcgccacgtcggccagcgtcagttgccggcggatggtcggcaggaataccacccgcccttcgcagcgctgcagcgccgccgcatcggggcgcgagatgcccgagggtatcgcgatgtcagtttcaaagccgtccgccagcatggcgccgatccacgcggcagggagtgcagtggtgggtcgggtggcgggaggagcgcggtgggggtcagcggcgtagcagagacgggcgaccaacctcgcataggacggggggtgggtcttagggggttgggaggcgacagggaccccagagcatgcgcggggaggtctgtcgggcccagacgcaccgagagcgaatccgtccgcggagtcccggcttgggttttatggggcccggccctcggaatcgcggcttgtcggcggggacaaagggggcggggctaggggcttgcggaaacagaagacgcgtgggataaaagaatcgcactaccccaaggaagggcggggcggtttattacagagccagtcccttgagcggggatgcgtcatagacgagatactgcgcgaagtgggtctcccgcgcgtgggcttccccgttgcgggcgctgcggaggagggcggggtcgctggcgcaggtgagcgggtaggcctcctgaaacaggccacacgggtcctccacgagttcgcggcaccccggggggcgcttaaactgtacgtcgctggcggcggtggccgtggacaccgccgaacccgtctccacgatcaggcgctccaggcagcgatgtttggcggcgatgtcggccgacgtaaagaacttaaagcaggggctgagcaccggcgaggccccgttgaggtggtaggccccgttatagagcaggtccccgtacgaaaatcgctgcgacgcccacgggttggccgtggccgcgaaggcccgggacgggtcgctctggccgtggtcgtacatgagggcggtgacatccccctccttgtcccccgcgtaaacgcccccggcggcgcgtccccgggggttgcagggccggcggaagtagttgacgtcggtcgacacgggggtggcgataaactcacacacggcgtcctggccgtggtccatccctgcgcgccgcggcacctgggcgcacccgaacacggggacgggctgggccggccccaggcggtttcccgccacgaccgcgttccgcaggtacacggctgccgcgttgtccaggagagggggagccccgcggcccaggtaaaagttttggggaaggttgcccatgtcggtgacggggttgcggacggttgccgtggccacgacggcggtgtagcccacgcccaggtccacgttcccgcgcggctgggtgagcgtgaagtttacccccccgccagtttcgtgccgggccacctggagctggcccaggaagtacgcctccgacgcgcgctccgagaacagcacgttctcagtcacaaagcggtcctgtcggacgacggtgaacccaaacccgggatggaggcccgtcttgagctgatgatgcaaggccacgggactgatcttgaagtaccccgccatgagcgcgtaggtcagcgcgttctccccggccgcgctctcgcggacgtgctgcacgacgggctgtcggatcgacgaaaagtagttggcccccagagccggggggaccagggggacctgccgcgacaggtcgcgcagggccggggggaaattgggcgcgttcgccacgtggtcggccccggcgaacagcgcgtggacggggagggggtaaaaatagtcgccattttggatggtatggtccagatgctggggggccatcagcaggattccggcgtgcaacgccccgtcgaatatgcgcatgttggtggtggacgcggtgttggcgcccgcgtcgggcgccgccgagcagagcagcgccgttgtgcgttcggccatgttgtgggccagcacctgcagcgtgagcatggcgggcccgtccactaccacgcgcccgttgtgaaacatggcgttgaccgtgttggccaccagattggccgggtgcagggggtgcgcggggtccgtcacggggtcgctggggcactcctcgccgggggcgatctccgggaccaccatgttctgcagggtggcgtatacgcggtcgaagcgaacccccgcggtgcagcagcggccccgcgagaaggcgggcaccatcacgtagtagtaaatcttgtggtgcacggtccagtccgccccccggtgcggccggtcatccgcggcgtccgcggctcgggcctgggtgttgtgcagcagctggccgtcgttgcggttgaagtccgcggtcgccacgttacatgccgccgcgtacacggggtcgtggccccccgcgctaacccggcagtcgcgatggcggtccagggccgcgcgccgcatcagggcgtcacagtcccacacgaggggtggcagcagcgccgggtctcgcattaggtgattcagctcggcttgcgcctgcccgcccagctccgggccggtcagggtaaagtcatcaaccagctgggccagggcctcgacgtgcgccaccaggtcccggtacacggccatgcactcctcgggaaggtctcccccgaggtaggtcacgacgtacgagaccagcgagtagtcgttcacgaacgccgcgcaccgcgtgttgttccagtagctggtgatgcactggaccacgagccgggccagggcgcagaagacgtgctcgctgccgtgtatggcggcctgcagcaggtaaaacaccgccgggtagttgcggtcgtcgaacgccccgcgaacggcggcgatggtggcgggggccatggcgtggcgtcccacccccagctccaggccccgggcgtcccggaacgccgccggacatagcgccaggggcaagttgccgttcaccacgcgccaggtggcctggatctcccccgggccggccgggggaacgtccccccccggcagctccacgtcggccacccccacaaagaagtcgaacgcggggtgcagctcaagagccaggttggcgttgtcgggctgcataaactgctccggggtcatctggccttccgcgacccatcggacccgcccgtgggccaggcgctgcccccaggcgttcaaaaacagctgctgcatgtctgcggcggggccggccggggccgccacgtacgccccgtacggattggcggcttcgacggggtcgcggttaaggcccccgaccgccgcgtcaacgttcatcagcgaagggtggcacacggtcccgatcgcgtgttccagagacaggcgcagcacctggcggtccttcccccaaaaaaacagctggcggggcgggaaggcgcggggatccgggtggccgggggcggggactaggtccccggcgtgcgcggcaaaccgttccatgaccggattgaacaggcccaggggcaggacgaacgtcaggtccatggcgcccaccagggggtagggaacgttggtggcggcgtagatgcgcttctccagggcctccagaaagaccagcttctcgccgatggacaccagatccgcgcgcacgcgcgtcgtctggggggcgctctcgagctcgtccagcgtctgccggttcaggtcgagctgctcctcctgcatctccagcaggtggcggcccacgtcgtccagacttcgcacggccttgcccatcacgagcgccgtgaccaggttggccccgttcaggaccatctcgccgtacgtcaccggcacgtcggcttcggtgtcctccgctttcaggaaggactgcaggaggcgctgtttgatcggggcggtggtgacgagcaccccgtcgaccggccgcccgcgcgtgtcggcatgcgtcagacggggcacggccacggagggctgcgtggccgtggtgaggtccacgagccaggcctcgacggcctcccggcggtggcccgccttgcccaggaaaaagctcgtctcgcagaagcttcgctttagctcggcgaccagggtcgcccgggccaccctggtggccaggcggccgttgtccaggtatcgttgcatcggcaacaacaaagccaggggcggcgccttttccagcagcacgtgcagcatctggtcggccgtgccgcgctcaaacgccccgaggacggcctggacgttgcgagcgagctgttggatggcgcgcaactggcgatgcgcgccgatacccgtcccgtccagggcctcccccgtgagcagggcgatggcctcggtggccaggctgaaggcggcgttcagggcccggcggtcgataatcttggtcatgtaattgtgtgtgggttgctcgatggggtgcgggccgtcgcgggcaatcagcggctggtggacctcgaactgtacgcgcccctcgttcatgtaggccagctccggaaacttggtacacacgcacgccaccgacaacccgagctccagaaagcgcacgagcgacagggtgttgcaatacgaccccagcagggcgtcgaactcgacgtcgtacaggctgtttgcatcggagcgcacgcgggaaaaaaaatcgaacaggcgtcgatgcgacgccacctcgatcgtgctaaggagggacccggtcggcaccatggccgcggcataccggtatcccggagggtcgcggttgggagctgccatggggtcgcgtggagatcggctggatctagcgatatttgcccggggaggctaagatccaccccaacgcccggccacccgtgtacgtgcccgacggcccaaggtccaccgaaagacacgacgggcccggacccaaaaaggcgggggatgctgtgtgaggggccgggtgtcggtcgggggggaaaggcaccgggagaaggctgcggcctcgttccaggagaacccagtgtccccaacagacccggggacgtgggatcccaggccttatataccccccccgccccacccccgttagaacgcgacgggtgcattcaagatggccctggtccaaaagcgtgccaggaagaaattggcagaggcggcaaagctgtccgccgccgccacccacatcgaggccccggccgcgcaggctatccccagggcccgtgtgcgcaggggatcggtgggcggcagcatttggttggtggcgataaagtggaaaagcccgtccggactgaaggtctcgtgggcggcggcgaacaaggcacacagggccgtgcctcccaaaaacacggacatcccccaaaacactggcgccgacaacggcagacgatccctcttgatgttaacgtacaggaggagcgcccgcaccgcccacgtaacgtagtagccgacgatggcggccaggatacaggccggcgccaccacccttccggtcagcccgtaatacatgcccgctgccaccatctccaacggcttcaggaccaaaaacgaccaaaggaacagaatcacgcgctttgaaaagaccggctgggtatggggcggaagacgcgagtatgccgaactgacaaaaaaatcagaggtgccgtacgaggacaatgaaaactgttcctccagcggcagttctccctcctcccccccgaaggcggcctcgtcgaccagatctcgatccaccagaggaaggtcatcccgcatggtcatggggtgtgcggtggaggtggggagaccgaaaccgcaaagggtcgcttacgtcagcaggatcccgagatcaaagacacccgggttcttgcacaaacaccacccgggttgcatccgcggaggcgagtgttttgataaggccgttccgcgccttgatataacctttgatgttgaccacaaaacccggaatttacgcctacgccccaatgcccacgcaagatgaggtaggtaacccccccgtgggtgtgacgttgcgtttagttcattggaggccaaggggaaaaatggggtggggaggaaacggaaaacccagtaggccgtgtcgggaacacgcccggggttgtcctcaaaaggcagggtccatactacggaagccgtcgttgtattcgagacctgcctgtgcgacgcacgtcggggttgcctgtgtccggttcggcccccaccgcgtgcggcacgcacgaggacgagtccgcgtgctttattggcgttccaagcgttgccctccagtttctgttgtcggtgttcccccatacccacgcccacatccaccgtagggggcctctgggccgtgttacgtcgccgcccgcgatggagcttagctacgccaccaccatgcactaccgggacgttgtgttttacgtcacaacggaccgaaaccgggcctactttgtgtgcggggggtgtgtttattccgtggggcggccgtgtgcctcgcagcccggggagattgccaagtttggtctggtcgttcgagggacaggcccagacgaccgcgtggtcgccaactatgtacgaagcgagctccgacaacgcggcctgcaggacgtgcgtcccattggggaggacgaggtgtttctggacagcgtgtgtcttctaaacccgaacgtgagctccgagctggatgtgattaacacgaacgacgtggaagtgctggacgaatgtctggccgagtactgcacctcgctgcgaaccagcccgggtgtgctaatatccgggctgcgcgtgcgggcgcaggacagaatcatcgagttgtttgaacacccaacgatagtcaacgtttcctcgcactttgtgtataccccgtccccatacgtgttcgccctggcccaggcgcacctcccccggctcccgagctcgctggaggccctggtgagcggcctgtttgacggcatccccgccccacgccagccacttgacgcccacaacccgcgcacggatgtggttatcacgggccgccgcgccccacgacccatcgccgggtcgggggcggggtcggggggcgcgggcgccaagcgggccaccgtcagcgagttcgtgcaagtcaaacacattgaccgcgtgggccccgctggcgtttcgccggcgcctccgccaaacaacaccgactcgagttccctggtgcccggggcccaggattccgccccgcccggccccacgctaagggagctgtggtgggtgttttatgccgcagaccgggcgctggaggagccccgcgccgactctggcctcacccgcgaggaggtacgtgccgtacgtgggttccgggagcaggcgtggaaactgtttggctccgcgggggccccgcgggcgtttatcggggccgcgttgggcctgagccccctccaaaagctggccgtttactactatatcatccaccgagagaggcgcctgtcccccttccccgcgctagtccggctcgtaggccggtacacacagcgccacggcctgtacgtccctcggcccgacgacccagtcttggccgatgccatcaacgggctggttcgcgacgcgctggcggccggaaccacagccgagcagctcctcatgttcgaccttctccccccaaaggacgtgccggtgggaagcgacgtgcaggccgacagcaccgctctgctgcgctttatagaatcgcaacgtctcgccgtccccgggggggtgatctcccccgagcacgtcgcgtaccttggtgcgttcctgagcgtgctgtacgctggccgcgggcgcatgtccgcagccacgcacaccgcgcggctgacaggggtgacctccctggtgctagcggtgggtgacgtggaccgtctttccgcgtttgaccgcggagcggcgggcgcggccagccgcacgcgggccgccgggtacctggatgtgcttcttaccgttcgtctcgctcgctcccaacacggacagtctgtgtaaaagaccccaataaacgtatgtcgctactacacccttgtgtgtcaatggacgcctctccgggggggggaagggaaagcaaagaggggctgggggagcggcaccaccggggcctgaacaaacaaaccacagacacggttacagtttattcggtcgggcggagaaacggccgaagccacgcccactttattcgcgtctccaaaaaaacgggacacttgtccggagaacctttaggatgccagccagggcggcggtaatcataaccacgcccagcgcagaggcggccagaaacccgggcgcaattgcggccacgggctgcgtgtcaaaggctagcaaatgaatgacggttccgtttggaaatagcaacaaggccgtggacggcacgtcgctcgaaaacacgcttggggcgccctccgtcggcccggcggcgatttgctgctgtgtgttgtccgtatccaccagcaacacagacatgacctccccggccggggtgtagcgcataaacacggcccccacgagccccaggtcgcgctggttttgggtgcgcaccagccgcttggactcgatatcccgggtggagccttcgcatgtcgcggtgaggtaggttaggaacagtgggcgtcggacgtcgacgccggtgagcttgtagccgatcccccggggcagaggggagtgggtgacgacgtagctggcgctgtgggtgatgggtaccaggatccgtggctcgacgttggcagactgccccccgcaccgatgtgaggcctcagggacgaaggcgcggatcagggcgttgtagtgtgcccaacgcgtcagggtcgaggcgaggccgtgggtctgctgggccaggacttcgaccggggtctcggatcgggtggcttgagccagcgcgtccaggataaacacgctctcgtctagatcaaagcgcagggaggccgcgcatggcgaaaagtggtccggaagccaaaagagggttttctggtggtcggcccgggccagcgcggtccggaggtcggcgttggtcgctgcggcgacgtcggacgtacacagggccgaggctatcagaaggctccggcgggcgcgttcccgctgcaccgccgaggggacgccagccaagaacggctgccggaggacagccgaggcgtaaaatagcgcccggtggacgaccggggtggtcagcacgcggccccctagaaactcggcatacagggcgtcgatgagatgggctgcgctgggcgccactgcgtcgtacgccgaggggctatccagcacgaaggccagctgatagcccagcgcgtgtaatgccaagctctgttcgcgctccagaatctcggccaccaggtgctggagccgagcctctagctgcaggcgggccgtgggatccaagactgacacattaaaaaacacagaatccgcggcacagcccgcggccccgcgggcggccaacccggcaagcgcgcgcgagtgggccaaaaagcctagcaggtcggagaggcagaccgcgccgtttgcgtgggcggcgttcacgaaagcaaaacccgacgtcgcgagcagccccgttaggcgccagaagagaggggggcgcgggccctgctcggcgcccgcgtcccccgagaaaaactccgcgtatgcccgcgacaggaactgggcgtagttcgtgccctcctccgggtagccgcccacgcggcggagggcgtccagcgcggagccgttgtcggcccgcgtcagggaccctaggacaaagacccgataccgggggccgcccgggggcccgggaagagcccccggggggttttcgtccgcggggtccccgacccgatctagcgtctggcccgcggggaccaccatcacttccaccggagggctgtcgtgcatggatatcacgagccccatgaattcccgcccgtagcgcgcgcgcaccagcgcggcatcgcacccgagcaccagctcccccgtcgtccagatgcccacgggccacgtcgaggccgacggggagaaatacacgtacctacctggggatctcaacaggccccgggtggccaaccaggtcgtggacgcgttgtgcaggtgcgtgatgtccagctccgtcgtcgggtgccgccgggccccaaccggcggtcgggggggcggtgtatcacgcggcccgctcgggtggctcgccgtcgccacgttgtctccccgcgggaacgtcagggcctcggggtcagggacggccgaaaacgttacccaggcccgggaacgcagcaacacggaggcggctggattgtgcaagagacccttaaggggggcgaccgaggggggaggctgggcggtcggctcgaccgtggtgggggcgggcaggctcgcgttcgggggccggccgagcaggtaggtcttcgggatgtaaagcagctggccggggtcccgcggaaactcggccgtggtgaccaatacaaaacaaaagcgctcctcgtaccagcgaagaaggggcagagatgccgtagtcaggtttagttcgtccggcggcgccagaaatccgcgcggtggtttttgggggtcgggggtgtttggcagccacagacgcccggtgttcgtgtcgcgccagtacatgcggtccatgcccaggccatccaaaaaccatgggtctgtctgctcagtccagtcgtggacctgaccccacgcaacgcccaaaataataacccccacgaaccataaaccattccccatgggggaccccgtccctaacccacggggcccgtggctatggcagggcttgccgccccgacgttggctgcgagccctgggccttcacccgaacttggggggtggggtggggaaaaggaagaaacgcgggcgtattggccccaatggggtctcggtggggtatcgacagagtgccagccctgggaccgaaccccgcgtttatgaacaaacgacccaacacccgtgcgttttattctgtctttttattgccgtcatagcgcgggttacttccggtattgtctccttccgtgtttcagttagcctcccccatctcccgggcaaacgtgcgcgccaggtcgcagatcgtcggtatggagccgggggtggtgacgtgggtctggaccatcccggaggtaagttgcagcagggcgtcccggcagccggcgggcgattggtcgtaatccaggataaagacgtgcatgggacggaggcgtttggccaagacgtccaaggcccaggcaaacacgttatacaggtcgccgttgggggccagcaactcgggggcccgaaacagggtaaataacgtgtccccgatatggggttgtgggcccgcgttgctctggggctcggcaccctggggcggcacggccgtccccgaaagctgtccccaatcctcccgccacgacccgccgccctgcagataccgcaccgtattggcaagcagctcgtaaacgcggcgaatcgcggccaacatagccaggtcaagccgctcgccggggcgctggcgtttggccaggcggtcgatgtgtctgtcctccggaagggcccccaacacgatgtttgtgccgggcaaggtcggcgggatgagggccacgaacgccagcacggcctggggggtcatgctgcccataaggtatcgcgcggccgggtaacacaggagggcggcgatgggatggcggtcgaagatgagggtgagggccgggggcggggcatgtgagctcccagcctcccccccgatatgaggagccagaacggcgtcggtcacggcataaggcatgcccattgttatctgggcgcttgtcattaccaccgccgcgtccccggccgatatctcaccctggtcgaggcggtgttgtgtggtgtagatgttcgcgattgtctcggaagcccccaacacccgccagtaagtcatcggctcgggtacgtagacgatatcgtcgcgcgaacccagggccaccagcagttgcgtggtggtggttttccccatcccgtggggaccgtctatataaacccgcagtagcgtgggcattttctgctccaggcggacttccgtggctttttgctgccggcgagggcgcaacgccgtacgtcggttgttatggccgcgagaacgcgcagcctggtcgaacgcagacgcgtgttgatggcaggggtacgaagccatacgcgcttctacaaggcgctggccgaagaggtgcgggagtttcacgccaccaagatctgcggcacgctgttgacgctgttaagcgggtcgctgcagggtcgctcggtattcgaggccacacgcgtcaccttaatatgcgaagtggacctgggaccgcgccgccccgactgcatctgcgtgttcgaattcgccaatgacaagacgctgggcggggtttgtgtcatcatagaactaaagacatgcaaatatatttcttccggggacaccgccagcaaacgcgagcaacgggccacggggatgaagcagctgcgccactccctgaagctcctgcagtccctcgcgcctccgggtgacaagatagtgtacctgtgccccgtcctggtgtttgtcgcccaacggacgctccgcgtcagccgcgtgacccggctcgtcccgcagaaggtctccggtaatatcaccgcagtcgtgcggatgctccagagcctgtccacgtatacggtccccattgagcctaggacccagcgagcccgtcgccgccgcggcggcgccgcccgggggtctgcgagcagaccgaaaaggtcacactctggggcgcgcgacccgcccgagtcagcggcccgccagttaccacccgccgaccaaacccccgcctccacggagggcgggggggtgcttaagaggatcgcggcgctcttctgcgtgcccgtggccaccaagaccaaaccccgagccgcctccgaatgagagtgtttcgttccttccccctccccccgcgtcagacaaaccctaaccaccgcttaagcggcccccgcgaggtccgaagactcatttggatccggcgggagccacccgacaacagcccccgggttttcccacgccagacgccggtccgctgtgccatcgcgccccctcatcccaccccccatcttgtccccaaataaaacaaggtctggtagttaggacaacgaccgcagttctcgtgtgttattttcgctctccgcctctcgcagatggacccgtactgcccatttgacgctctggacgtctgggaacacaggcgcttcatagtcgccgattcccgaaacttcatcacccccgagttcccccgggacttttggatgtcgcccgtctttaacctcccccgggagacggcggcggagcaggtggtcgtcctacaggcccagcgcacagcggctgccgctgccctggagaacgccgccatgcaggcggccgagctccccgtcgatatcgagcgccggttacgcccgatcgaacggaacgtgcacgagatcgcaggcgccctggaggcgctggagacggcggcggccgccgccgaagaggcggatgccgcgcgcggggatgagccggcgggtgggggcgacgggggggcgcccccgggtctggccgtcgcggagatggaggtccagatcgtgcgcaacgacccgccgctacgatacgacaccaacctccccgtggatctgctacacatggtgtacgcgggccgcggggcgaccggctcgtcgggggtggtgttcgggacctggtaccgcactatccaggaccgcaccatcacggactttcccctgaccacccgcagtgccgactttcgggacggccggatgtccaagaccttcatgacggcgctggtcctgtccctgcagtcgtgcggccggctgtatgtgggccagcgccactattccgccttcgagtgcgccgtgttgtgtctctacctgctgtaccgaaacacgcacggggccgccgacgatagcgaccgcgctccggtcacgttcggggatctgctgggccggctgccccgctacctggcgtgcctggccgcggtgatcgggaccgagggcggccggccacagtaccgctaccgcgacgacaagctccccaagacgcagttcgcggccggcgggggccgctacgaacacggagcgctggcgtcgcacatcgtgatcgccacgctgatgcaccacggggtgctcccggcggccccgggggacgtcccccgggacgcgagtacccacgttaaccccgacggcgtggcgcaccacgacgacataaaccgcgccgccgccgcgttcctcagccggggccacaacctattcctgtgggaggaccagactctgctgcgggcaaccgcgaacaccataacggccctgggcgttatccagcggctcctcgcgaacggcaacgtgtacgcggaccgcctcaacaaccgcctgcagctgggcatgctgatccccggagccgtcccttcggaggccatcgcccgtggggcctccgggtccgactcgggggccatcaagagcggagacaacaatctggaggcgctatgtgccaattacgtgcttccgctgtaccgggccgacccggcggtcgagctgacccagctgtttcccggcctggccgccctgtgtcttgacgcccaggcggggcggccggtcgggtcgacgcggcgggtggtggatatgtcatcgggggcccgccaggcggcgctggtgcgcctcaccgccctggaactcatcaaccgcacccgcacaaaccccacccccgtgggggaggttatccacgcccacgacgccctggcgatccaatacgaacaggggcttggcctgctggcgcagcaggcacgcattggcttgggctccaacaccaagcgtttctccgcgttcaacgttagcagcgactacgacatgttgtactttttatgtctggggttcattccacagtacctgtcggcggtttagtgggtggtgggcgaggggggagggggcattagggagaaagaacaagagcctccgttgggttttctttgtgcctgtactcaaaaggtcataccccgtaaacggcgggctccagtcccggcccggtggttggcgtgaacgcaacggcgggagctgggttagcgtttagtttagcattcgctctcgcctttccgcccgccccccgaccgttgcgccttttttttcgtccaccaaagtctctgtgggtgcgcgcatggcagccgatgccccgggagaccggatggaggagcccctgcccgacagggccgtgcccatttacgtggctgggtttttggccctgtatgacagcggggactcgggcgagttggcattggatccggatacggtgcgggcggccctgcctccggataacccactcccgattaacgtggaccaccgcgctggctgcgaggtggggcgggtgctggccgtggtcgacgacccccgcgggccgttttttgtggggctgatcgcctgcgtgcagctggagcgcgtcctcgagacggccgccagcgctgcgattttcgagcgccgcgggccgccgctctcccgggaggagcgcctgttgtacctgatcaccaactacctgccctcggtctccctggccacaaaacgcctggggggcgaggcgcaccccgatcgcacgctgttcgcgcacgtcgcgctgtgcgcgatcgggcggcgcctcggcactatcgtcacctacgacaccggtctcgacgccgccatcgcgccctttcgccacctgtcgccggcgtctcgcgagggggcgcggcgactggccgccgaggccgagatcgcgctgtccgggcgcacctgggcgcccggcgtggaggcgctgacccacacgctgctttccaccgccgttaacaacatgatgctgcgggaccgctggagcctggtggccgagcggcggcggcaggccgggatcgccggacacacctacctccaggcgagcgaaaaattcaaaatgtggggggcggagcctgtttccgcgccggcgcgcgggtataagaacggggccccggagtccacggacataccgcccggctcgatcgctgccgcgccgcagggtgaccggtgcccaatcgtccgtcagcgcggggtcgccttgtccccggtactgccccccatgaaccccgttccgacatcgggcaccccggcccccgcgccgcccggcgacgggagctacctgtggatcccggcctcccattacaaccagctcgtcgccggccatgccgcgccccaaccccagccgcattccgcgtttggtttcccggctgcggcgggggccgtggcctatgggcctcacggcgcgggtctttcccagcattaccctccccacgtcgcccatcagtatcccggggtgctgttctcgggacccagcccactcgaggcgcagatagccgcgttggtgggggccatagccgcggaccgccaggcgggcggtcagccggccgcgggagaccctggggtccgggggtcgggaaagcgtcgccggtacgaggcggggccgtcggagtcctactgcgaccaggacgaaccggacgcggactacccgtactaccccggggaggctcgaggcgggccgcgcggggtcgactctcggcgcgcggcccgccagtctcccgggaccaacgagaccatcacggcgctgatgggggcggtgacgtctttgcagcaggaactggcgcacatgcgggctaggaccagcgccccctatgggatgtacacgccggtggcgcactatcgccctcaggtgggggagccggaaccaacaacgacccacccggccctttgtcccccggaggccgtgtatcgccccccaccacacagcgccccctacggtcctccccagggtccggcgtcccatgcccccactcccccgtatgccccagctgcctgcccgccaggcccgccaccgcccccatgtccttccacccagacgcgcgcccctctaccgacggagcccgcgttcccccccgccgccaccggatcccaaccggaggcatccaacgcggaggccggggcccttgtcaacgccagcagcgcagcacacgtggacgttgacacggcccgcgccgccgatttgttcgtctctcagatgatgggggcccgctgattcgccccggtctttggtaccatgggatgtcttactgtatatctttttaaataaaccaggtaataccaaagaagacccattggtgtatgttctttttttattgggaggcgcgggtaggcgggtagctttacaatgcaaaagccttcgacgtggaggaaggcgtgggggggaatcggcactgaccaagggggtccgttttgtcacgggaaaggaaagaggaaacaggccgcggacacccgggggagtttatgtgttcccttttctttcttcccacacacacaaaaggcgtaccaaacaaacaaaccaaaagatgcacatgcggtttaacacccgtggtttttatttacaacaaaccccccgtcacaggtcgtcctcgtcggcgtcaccgtctttgttgggaacttgggtgtagttggtgttgcggcgcttgcgcatgaccatgtcggtgaccttggcgctgagcagcgcgctcgtgcccttcttcttggccttgtgttccgtgcgctccatggcagacaccagggccatgtaccgtatcatctcccgggcctcggctagcttggcctcgtcaaagtcgccgccctcctcgccctccccggacgcgtccgggttggtggggttcttgagctccttggtggttagcgggtacagggccttcatggggttgctctgcagccgcatgacgtagcgaaaggcgaagaaggccgccgccaggccggccaggaccaacagacccacggccagcgccccaaaggggttggacatgaaggaggacacgcccgacacggccgataccacgccgcccacgatgcccatcaccaccttgccgaccgcgcgccccaggtcgcccatcccctcgaagaacgcgcccaggcccgcaaacatggcggcgttggcgtcggcgtggatgaccgtgtcgatgtcggcgaagcgcaggtcgtgcagctggttgcggcgctggacctccgtgtagtccagcaggccgctgtccttgatctcgtggcgggtgtacacctccagggggacaaactcgtgatcctccagcatggtgatgttgaggtcgatgaaggtgctgacggtggtgatgtcggcgcggctcagctggtgggagtacgcgtactcctcgaagtacacgtagcccccaccgaaggtgaagtagcgccggtgtcccacggtacacggctcgatcgcatcgcgcgtcagccgcagctcgttgttctcccccagctgcccctcgaccaacgggccctggtcttcgtaccgaaagctgaccagggggcggctgtagcaggccccgggccgcgagctgatgcgcatcgagttttggacgatcacgttgtccgcggcgaccggcacgcacgtggagacggccatcacgtcgccgagcatccgcgcgctcacccgccggcccacggtggccgaggcgatggcgttggggttcagcttgcgggcctcgttccacagggtcagctcgtgattctgcagctcgcaccacgcgatggcaacgcggcccaacatatcgttgacatggcgctgtatgtggttgtacgtaaactgcagcctggcgaactcgatggaggaggtggtcttgatgcgctccacggacgcgttggcgctggccccgggcggcgggggcgtggggtttgggggcttgcggctctgctctcggaggtgttcccgcacgtacagctccgcgagcgtgttgctgagaaggggctggtacgcgatcagaaagcccccattggccaggtagtactgcggctggcccaccttgatgtgcgtcgcgttgtacctgcgggcgaagatgcggtccatggcgtcgcgggcgtccttgccgatgcagtcccccaggtccacgcgcgagagcgggtactcggtcaggttggtggtgaaggtggtggatatggcgtcggaggagaatcggaaggagccgccgtactcggagcgcagcatctcgtccacctcctgccacttggtcatggtgcagaccgacgggcgctttggcacccagtcccaggccacggtgaacttgggggtcgtgagcaggttccgggtggtcggcgccgtggcccgggccttggtggtgaggtcgcgcgcgtagaagccgtcgacctgcttgaagcggtcggcggcgtagctggtgtgttcggtgtgcgacccctcccggtagccgtaaaacggggacatgtacacaaagtcgccagtcgccagcacaaactcgtcgtacgggtacaccgagcgcgcgtccacctcctcgacgatgcagtttaccgtcgtcccgtaccggtggaacgcctccacccgcgaggggttgtacttgaggtcggtggtgtgccagccccggctcgtgcgggtcgcggcgttggccggtttcagctccatgtcggtctcgtggtcgtcccggtgaaacgcggtggtctccaggttgttgcgcacgtacttggccgtggaccgacagacccccttggcgttgatcttgtcgatcacctcctcgaaggggacgggggcgcggtcctcaaagatccccataaactgggagtagcggtggccgaaccacacctgcgaaacggtgacgtctttgtagtacatggtggccttgaacttgtacggggcgatgttctccttgaagaccaccgcgatgccctccgtgtagttctgaccctcgggccgggtcgggcagcggcgcggctgctcgaactgcaccaccgtggcgcccgtggggggtgggcacacgtaaaagtttgcatcggtgttctccgccttgatgtcccgcaggtgctcgcgcagggtggcgtggcccgcggcgacggtcgcgttgtcgccggcggggcgcggcggctttgggggtttcggttttttgttcttcttcggtttcgggtcccccgttgggggggcgccaggggcgggcggcgccggagtggcagggcccccgttcgccgcctgggtcgcggccgcgaccccaggcgtgccgggggaactcggagccgccgacaccaccaggacccccagcgtcaaccccaagagcgcccatacgacgaaccaccggcgcccccgcgcgggggcgccctggcgcatggcgggactacgggggcccgtcgtgccccccgtcaggtagcctgggggcgaggtgctggaggaccgagtagaggatcgagaaaacgtctcggtcgtagaccacgaccgaccgggggccgatacagccgtcgggggcgctctcgacgatggccaccagcggacagtcggagtcgtacgtgagatatacgccgggcgggtaacggtaacgaccttcggaggtcgggcggctgcagtccgggcggcgcaactcgagctccccgcaccggtagaccgaggcaaagagtgtggtggcgataatcagctcgcgaatatatcgccaggcggcgcgctgagtgggcgttattccggaaatgccgtcaaaacagtaaaacctctgaaattcgctgacggcccaatcagcacccgagccccccgcccccatgatgaaccgggcgagctcctccttcaggtgcggcaggagccccacgttctcgacgctgtaatacagcgcggtgttggggggctgggcgaagctgtgggtggagtgatcaaagaggggcccgttgacgagctcgaagaagcgatgggtgatgctggggagcagggccgggtccacctggtgtcgcaggagagacgctcgcatgaaccggtgcgcgtcgaacacgcccggcgccgagcggttgtcgatgaccgtgcccgcgcccgccgtcagggcgcagaagcgcgcgcgcgccgcaaagccgttggcgaccgcggcgaacgtcgcgggcagcacctcgccgtggacgctgacccgcagcatcttctcgagctccccgcgctgctcgcggacgcagcgccccaggctggccaacgaccgcttcgtcaggcggtccgcgtacagccgccgtcgctcccgcacgtccgcggccgcttgcgtggcgatgtccccccacgtctcgggcccctgccccccgggcccgcggcgacggtcttcgtcctcgcccccgcccccgggagctcccaacccccgtgccccttcctctacggcgacacggtccccgtcgtcgtcggggcccgcgccgcccttgggcgcgtccgccgcgccccccgcccccatgcgcgccagcacgcgacgcagcgcctcctcgtcgcactgttcggggctgacgaggcgccgcaagagcggcgtcgtcaggtggtggtcgtagcacgcgcggatgagcgcctcgatctgatcgtcgggtgacgtggcctgaccgccgattattagggcgtccaccatatccagcgccgccaggtggctcccgaacgcgcgatcgaaatgctccgcccgccgcccgaacagcgccagttccacggccaccgcggcggtctcctgctgcaactcgcgccgcgccagcgcggtcaggttgctggcaaacgcgtccatggtggtctggccggcgcggtcgccggacgcgagccagaatcgcaattcgctgatggcgtacaggccgggcgtggtggcctgaaacacgtcgtgcgcctccagcagggcgtcggcctccttgcggaccgagtcattctcgggcgacgggtggggctgcccgtcgccccccgcggtccgggccagcgcatggtccaacacggagagcgcccgcgcgcggtcggcgtccgacagcccggcggcgtggggcaggtaccgccgcagctcgttggcgtccagccgcacctgcgcctgctgggtgacgtggttacagatacggtccgccaggcggcgggcgatcgtcgccccctggttcgccgtcacacacagttcctcgaaacagaccgcgcaggggtgggacgggtcgctaagctccggggggacgataaggcccgaccccaccgcccccaccataaactcccgaacgcgctccagcgcggcggtggcgccgcgcgagggggtgatgaggtggcagtagtttagctgctttagaaagttctcgacgtcgtgcaggaaacacagctccatatggacggtcccgccatacgtatccagcctgacccgttggtgatacggacagggtcgggccaggcccatggtctcggtgaaaaacgccgcgacgtctcccgcggtcgcgaacgtctccaggctgcccaggagccgctcgccctcgcgccacgcgtactctagcagcaactccagggtgaccgacagcggggtgagaaaggccccggcctgggcctccaggcccggcctcagacgacgccgcagcgcccgcacctgaagcgcgttcagcttcagttgggggagcttcccccgtccgatgtgggggtcgcaccgccggagcagctctatctgaaacacataggtctgcacctgcccgagcagggctaacaacttttgacgggccacggtgggctcggacaccggggcggccatctcgcggcgccgatctgtaccgcggccggagtatgcggtggaccgaggcggtccgtacgctacccggcgtctggctgagccccggggtccccctcttcggggcggcctcccgcgggcccgccgaccggcaagccgggagtcggcggcgcgtgcgtttctgctctattcccagacaccgcggagaggaatcacggcccgcccagagatatagacacggaacacaaacaagcacggatgtcgtagcaataatttattttacacacattccccgccccgccctaggttcccccacccccaacccctcacagcatatccaacgtcaggtctccctttttgtcggggggcccctccccaaacgggtcatccccgtggaacgcccgtttgcggccggcaaatgccggtcccggggcccccgggccgccgaacggcgtcgcgttgtcgtcctcgcagccaaaatccccaaagttaaacacctccccggcgttgccgagttggctgactagggcctcggcctcgtgcgccacctccagggccgcgtccgtcgaccactcgccgttgccgcgctccagggcacgcgcggtcagctccatcatctcctcgcttaggtactcgtcctccaggagcgccagccagtcctcgatctgcagctgctgggtgcggggccccaggcttttcacggtcaccacgaacacgctactggcgacggccgccccgccctcggagataatgccccggagctgctcgcacagcgagctttcgtgcgctccgccgccgaggctcgaggccgcgcacacaaacccggcccggggacaggccaggacgaacttgcgggtgcggtcaaaaataaggagcgggcacgcgtttttgccgcccatcaggctggcccagttcccggcctgaaacacacggtcgttgccggccatgccgtagtacttgctgatgctcaaccccaacacgaccatggggcgcgccgccatgacgggccgcagcaggttgcagctggcgaacatggacgtccacgcgcccggatgcgcgtccacggcgtccatcagcgcgcgggccccggcctccaggcccgccccgccctgcgcggaccacgcggccgcagcctgcacgctggggggacggcgggaccccgcgatgatggccgtaagggtgttgatgaagtacgtcgagtgatcgcagtaccgcagaatctggtttgccatgtagtacatcgccagctcgctcacgttgttgggggccaggttaataaagtttatcgcgccgtagtccagggaaaactttttaatgaacgcgatggtctcgatgtcctcgcgcgacaggagccgggcgggaagctggttgcgttggagggccgtccagaaccactgcgggttcggctggttggaccccgggggcttgccgttggggaagatggccgcgtggaactgcttcagcagaaagcccagcggtccgaggaggatgtccacgcgcttgtcgggcttctggtaggcgctctggaggctggcgacccgcgccttggcggcctcggacgcgttggcgctcgcgcccgcgaacaacacgcggctcttgacgcgcagctccttgggaaaccccagggtcacgcgggcaacgtcgccctcgaagctgctctcggcgggggccgtctggccggccgttaggctgggggcgcagatagccgccccctccgagagcgcgaccgtcagcgttttggccgacagaaacccgttgttaaacatgtccatcacgcgccgccgcagcaccggttggaattgattgcgaaagttgcgcccctcgaccgactgcccggcgaacaccccgtggcactggctcagggccaggtcctgatacacggcgaggttggatcgccgcccgagaagctgaagcagggggcatggcccgcacgcgtacgggtccagcgtcagggacatggcgtggttggcctcgcccagaccgtcgcgaaacttgaagttcctcccctccaccaggttgcgcatcagctgctccacctcgcggtccacgacctgcctgacgttgttcaccaccgtatgcagggcctcgcggttggtgatgatggtctccagccgccccatggccgtggggaccgcctggtccacgtactgcagggtctcgagttcggccatgacgcgctcggtcgccgcgcggtacgtctcctgcatgatggtccgggcggtctcggatccgtccgcgcgcttcagggccgagaaggcggcgtagtttcccagcacgtcgcagtcgctgtacatgctgttcatggtcccgaagacgccgatggctccgcgggcggcgctggcgaacttgggatggcgcgcccggaggcgcatgagcgtcgtgtgtacgcaggcgtggcgcgtgtcgaaggtgcacaggttgcagggcacgtcggtctggttggagtccgcgacgtatcgaaacacgtccatctcctggcgcccgacgatcacgccgccgtcgcagcgctccaggtaaaacagcatcttggccagcagcgccggggaaaacccacacagcatggccaggtgctcgccggcaaattcctgggttccgccgacgaggggcgcggtgggccgaccctcgaacccgggcaccacgtgtccctcgcggtccacctgtgggttggccgccacgtgggtcccgggcacgaggaagaagcggtaaaaggagggtttgctgtggtcctttgggtccgccggaccggcgtcgtccacctcggtgagatggagggccgagttggtgctaaataccatggcccccacgagtcccgcggcgcgcgccaggtacgccccgacggcgttggcgcgggccgcggccgtgtcctggccctcgcacagcggccatgcggagatgtcggtgggcggctcgtcgaagacggccatcgacacgatagactcgagggccagggcggcgtctccggccatgacggaggccaggcgctgttcgaacccgcccgccgggcccttgccgccgccgtcgcgcccaccccgcggggtcttaccctggctggcttcgaaggccgtgaacgtaatgtcggcggggagggcggcgccctcgtggttttcgtcaaacgccaggtgggcggccgcgcgggccacggcgtccacgtttcggcatcgcagtgccacggcggcgggtcccacgaccgcctcgaacaggaggcggttgagggggcggttaaaaaacggaagcgggtaggtaaaattctccccgatcgatcggtggttggcgttgaacggctcggcgatgacccggctaaaatccggcatgaacagctgcaacggatacacgggtatgcggtgcacctccgccccgcctatggttaccttgtccgagcctcccaggtgcagaaaggtgttgttgatgcacacggcctccttgaagccctcggtaacgaccagatacaggagggcgcggtccgggtccaggccgaggcgctcacacagcgcctcccccgtcgtctcgtgtttgaggtcgccgggccggggggtgtagtccgaaaagccaaaatggcggcgtgcccgctcgcagagtcgcgtcaggtttggggcctgggtgttggggtccaggtgccggccgccgtgaaagacgtacacggacgagctgtagtgcgatggcgtcagtttcagggacaccgcggtacccccgagccccgtcgtgcgagaacccacgaccacggctacgttggcctcaaagccgctctccacggtcaggcccacgaccaggggcgccacggcgacgtcggcatcgccgctgcgcgccgacagtaacgccagaagctcgatgccttcggatggacacgcgcgagcgtacacgtatcccaggggcccgggggggaccttgatggtggttgccgtcttgggctttgtctccatgtcctcctggcaatcggtccgcaaacggaggtaatcccggcacgacgacggacgcccgacgaggtatgtctcccgagcgtcaaaatccggggggggcggcgacggtcaaggggagggtgggagaccggggttggggaatgaatccctacccttcaccgacaacccccgggtaaccacggggtgccgatgaaccccggcggctggcaacgcggggtccctgcgagaggcacagatgcttacggtcaggtgctccgggccgggtgcgtctgatatgcggttggtatatgtacactttacctgggggcgtgccggaccgcaccagcccctcccacaccccgcgcgtcatcagccggtgggcgnnnnnnnnnnnnnnnnnnnnnnnnnnnnnnnnnnnnnnnnnnnnnnnnnnnnnnnnnnnnnnnnnnnnnnnnnnnnnnnnnnnnnnnnnnnnnnnnnnnnnntttttataatagcggccacgcccaccggctacgtcacgctcctgtcggccgccggcggtccataagcccggccggccgggccgacgcgaataaaccgggccgccggccggggcgccgcgcagcagctcgccgcccggatccgccagacaaacaaggcccttgcacatgccggcccgggcgagcctgggggtccggtaattttgccatcccacccaagcggcttttggggtttttcctcttcccccctccccacctcccccctctttaggggttcgggtgggaacaaccgcgatgttttccggtggcggcggcccgctgtcccccggaggaaagtcggcggccagggcggcgtccgggttttttgcgcccgccggccctcgcggagccggccggggacccccgccttgtttgaggcaaaacttttacaacccctacctcgccccagtcgggacgcaacagaagccgaccgggccaacccagcgccatacgtactatagcgaatgcgatgaatttcgattcatcgccccgcgggtgctggacgaggatgcccccccggagaagcgcgccggggtgcacgacggtcacctcaagcgcgcccccaaggtgtactgcgggggggacgagcgcgacgtcctccgcgtcgggtcgggcggcttctggccgcggcgctcgcgcctgtggggcggcgtggaccacgccccggcggggttcgaccccaccgtcaccgtctttcacgtgtatgacatcctggagaacgtggagcacgcgtacggcatgcgcgcggcccagttccacgcgcggtttatggacgccatcacaccgacggggaccgtcatcacgctcctgggcctgactccggaaggccaccgggtggccgttcacgtttacggcacgcggcagtacttttacatgaacaaggaggaggttgacaggcacctacaatgccgcgccccacgagatctctgcgagcgcatggccgcggccctgcgcgagtccccgggcgcgtcgttccgcggcatctccgcggaccacttcgaggcggaggtggtggagcgcaccgacgtgtactactacgagacgcgccccgctctgttttaccgcgtctacgtccgaagcgggcgcgtgctgtcgtacctgtgcgacaacttctgcccggccatcaagaagtacgagggtggggtcgacgccaccacccggttcatcctggacaaccccgggttcgtcaccttcggctggtaccgtctcaaaccgggccggaacaacacgctagcccagccgcgggccccgatggccttcgggacatccagcgatgtcgagtttaactgtacggcggacaacctggccatcgaggggggcatgagcgacctaccggcatacaagctcatgtgcttcgatatcgaatgcaaggcggggggggaggacgagctggcctttccggtggccgggcacccggaggacctggtcatccagatatcctgtctgctctacgacctgtccaccaccgccctggagcacgtcctcctgttttcgctcggttcctgcgacctccccgaatcccacctgaacgagctggcggccaggggcctgcccacgcccgtggttctggaattcgacagcgaattcgagatgctgttggccttcatgacccttgtgaaacagtacggccccgagttcgtgaccgggtacaacatcatcaacttcgactggcccttcttgctggccaagctgacggacatttacaaggtccccctggacgggtacggccgcatgaacggccggggcgtgtttcgcgtgtgggacataggccagagccacttccagaagcgcagcaagataaaggtgaacggcatggtgaacatcgacatgtacgggattataaccgacaagatcaagctctcgagctacaagctcaacgccgtggccgaagccgtcctgaaggacaagaagaaggacctgagctatcgcgacatccccgcctactacgccgccgggcccgcgcaacgcggggtgatcggcgagtactgcatacaggattccctgctggtgggccagctgttttttaagtttttgccccatctggagctctcggccgtcgcgcgcttggcgggtattaacatcacccgcaccatctacgacggccagcagatccgcgtctttacgtgcctgctgcgcctggccgaccagaagggctttattctgccggacacccaggggcgatttaggggcgccgggggggaggcgcccaagcgtccggccgcagcccgggaggacgaggagcggccagaggaggagggggaggacgagaacgaacgcgaggagggcgggggcgagcgggagccggagggcgcgcgggagaccgccggccggcacgtggggtaccagggggccagggtccttgaccccacttccgggtttcacgtgaaccccgtggtggtgttcgactttgccagcctgtaccccagcatcatccaggcccacaacctgtgcttcagcacgctctccctgagggccgacgcagtggcgcacctggaggcgggcaaggactacctggagatcgagatgggggggcgacggctgttcttcgtcaaggctcacgtgcgagagagcctcctcagcatcctcctgcgggactggctcgccatgcgaaagcagatccgctcgcggattccccagagcagccccgaggaggccgtgctcctggacaagcagcaggccgccatcaaggtcgtgtgtaactcggtgtacgggttcacgggagtgcagcacggactcctgccgtgcctgcatgttgccgcgacggtgacgaccatcggccgcgagatgctgctcgcgacccgcgagtacgtccacgcgcgctgggcggccttcgaacagctcctggccgatttcccggaggcggccgacatgcgcgcccccgggccctattccatgcgcatcatctacggggacacggactccatatttgtgctgtgccgcggcctcacggccgccgggctgacggccatgggcgacaagatggcgagccacatctcgcgcgcgctgtttctgccccccatcaaactcgagtgcgaaaagacgttcaccaagctgctgctgatcgccaagaaaaagtacatcggcgtcatctacgggggtaagatgctcatcaagggcgtggatctggtgcgcaaaaacaactgcgcgtttatcaaccgcacctccagggccctggtcgacctgctgttttacgacgataccgtatccggagcggccgccgcgttagccgagcgccccgcagaggagtggctggcgcgacccctgcccgagggactgcaggcgttcggggccgtcctcgtagacgcccatcggcgcatcaccgacccggagagggacatccaggactttgtcctcaccgccgaactgagcagacacccgcgcgcgtacaccaacaagcgcctggcccacctgacggtgtattacaagctcatggcccgccgcgcgcaggtcccgtccatcaaggaccggatcccgtacgtgatcgtggcccagacccgcgaggtagaggagacggtcgcgcggctggccgccctccgcgagctagacgccgccgccccaggggacgagcccgccccccccgcggccctgccctccccggccaagcgcccccgggagacgccgtcgcatgccgaccccccgggaggcgcgtccaagccccgcaagctgctggtgtccgagctggccgaggatcccgcatacgccattgcccacggcgtcgccctgaacacggactattacttctcccacctgttgggggcggcgtgcgtgacattcaaggccctgtttgggaataacgccaagatcaccgagagtctgttaaaaaggtttattcccgaagtgtggcaccccccggacgacgtggccgcgcggctccgggccgcagggttcggggcggtgggtgccggcgctacggcggaggaaactcgtcgaatgttgcatagagcctttgatactctagcatgagccccccgtcgaagctgatgtccctcattttacaataaatgtctgcggccgacacggtcggaatctccgcgtccgtgggtttctctgcgttgcgccggaccacgagcacaaacgtgctctgccacacgtgggcgacgaacctgtaccccgggcacgcggtgagcatccggtctatgagccggtagtgcaggtgggcggacgtgccgggaaagatgacgtacagcatgtggcccccgtaagtggggtccgggtaaaacaacagccgcgggtcgcacgccccgcctccgcgcaggatcgtgtggacgaaaaaaagctcgggttggccaagaatcccggccaagaggtcctggaggggggcgttgtggcggtcggccaacacgaccaaggaggccaggaaggcgcgatgctcgaatatcgtgttgatctgctgcacgaaggccaggattagggcctcgcggctggtggcggcgaaccgcccgtctcccgcgttgcacgcgggacagcaacccccgatgcctaggtagtagcccatcccggagagggtcaggcagttgtcggccacggtctggtccagacagaagggcagcgacacgggagtggtcttcaccaggggcaccgagagcgagcgcacgatggcgatctcctcggagggcgtctgggcgagggcggcgaaaaggccccgatagcgctggcgctcgtgtaaacacagctcctgtttgcgggcgtgaggcggcaggctcttccgggaggcccgacgcaccacgcccagagtcccgccggccgcagaggagcgcgaccgccggcgctccttgccgtgatagggcccgggccgggagccgcggcgatgggggtcggtatcatacataggtacacagggtgtgctccagggacaggagcgagatcgagtggcgtctaagcagcgcgcccgcctcacggacaaatgtggcgagcgcggtgggctttggtacaaatacctgatacgtcttgaaggtgtagatgagggcacgcaacgctatgcagacacgcccctcgaactcgttcccgcaggccagcttggccttgtggagcagcagctcgtcgggatgggtggcggggggatggccgaacagaacccaggggtcaacctccatctccgtgatggcgcacatggggtcacagaacatgtgcttaaagatggcctcgggccccgcggcccgcagcaggctcacaaaccggcccccgtccccgggctgcgtctcggggtccgcctcgagctggtcgacgacgggtacgatacagtcgaagaggctcgtgttgttttccgagtagcggaccacggaggcccggagtctgcgcagggccagccagtaagcccgcaccagtaacaggttacacagcaggcattctccgccggtgcgcccgcgcccccggccgtgtttcagcacggtggccatcagagggcccaggtcgaggtcgggctgggcatcgggttcggtaaactgcgcaaagcgcggagccacgtcgcgcgtgcgtgccccgcgatgcgcttcccaggactggcggaccgtggcgcgacgggcctccgcggcagcgcgcagctggggccccgactcccagacggcgggggtgccggcgaggagcagcaggaccagatccgcgtacgcccacgtatccggcgactcctccggctcgcggtccccggcgaccgtctcgaattccccgttgcgagcggcggcgcgcgtacagcagctgtccccgcccccgcgccgaccctccgtgcagtccaggagacgggcgcaatccttccagttcatcagtgcggtggtaagcgacggctgcgtgccggataccgccgccgaccccgccccctcctcgcccccggaggccaaggttccgatgagggcccgggtggcagactgcgccaggaacgagtagttggagtactgcaccttggcggctcccggggagggcgagggcttgggttgcttctgggcatgccgcccgggcaccccgccgtcggtacggaagcagcagtggagaaaaaagtgccggtggatgtcgtttatggtgagggcaaagcgtgcgaaggagccgaccagggtcgccttcttggtgcgcagaaagtggcggtccatgacgtacacaaactcgaacgcggccacgaagatgctagcggcgcagtggggcgcccccaggcatttggcacagagaaacgcgtaatcggccacccactgaggcgagaggcggtaggtttgcttgtacagctcgatggtgcggcagaccagacagggccggtccagcgcgaaggtgtcgatggccgccgcggaaaagggcccggtgtccaaaagcccctccccacagggatccgggggcgggttgcggggtcctccgcgcccgcccgaaccccctccgtcgcccgcccccccgcgggcccttgagggggcggtgaccacgtcggcggcgacgtcctcgtcgagcgtaccgacgggcggcacacctatcacgtgactggccgtcaggagctcggcgcagagagcctcgttaagagccaggaggctgggatcgaaggccacatacgcgcgctcgaacgcccccgccttccagctgctgccgggggactcttcgcacaccgcgacgctcgccaggaccccggggggcgaagttgccatggctgggcgggaggggcgcacgcgccagcgaactttacgggacacaatccccgactgcgcgctgcggtcccagaccctggagagtctagacgcgcgctacgtctcgcgagacggcgcgcatgacgcggccgtctggttcgaggatatgacccccgccgagctggaggttgtcttcccgactacggacgccaagctaaactacctgtcgcggacgcagcggctggcctccctcctgacgtacgccgggcctataaaagcgcccgacgacgccgccgccccgcagaccccggacaccgcgtgtgtgcacggcgagctgctcgcccgcaagcgggaaagattcgcggcggtcattaaccggttcctggacctgcaccagattctgcggggctgacgcgcgcgctgttgggcgggacggttcgcgaaccctttggtgggtttacgcgggcacgcacgctcccatcgcgggcgccatggcgggactgggcaagccctacaccggccacccaggtgacgccttcgagggtctcgttcagcgaattcggcttatcgtcccatctacgttgcggggcggggacggggaggcgggcccctactctccctccagcctcccctccaggtgcgcctttcagtttcatggccatgacgggtccgacgagtcgtttcccatcgagtatgtactgcggcttatgaacgactgggccgaggtcccgtgcaacccttacctgcgcatacagaacaccggcgtgtcggtgctgtttcaggggttttttcatcgcccacacaacgcccccgggggcgcgattacgccagagcggaccaatgtgatcctggggtccaccgagacgacggggttgtccctcggcgacctggacaccatcaaggggcggctcggcctggatgcccggccgatgatggccagcatgtggatcagctgctttgtgcgcatgccccgcgtgcagctcgcgtttcggttcatgggccccgaagatgccggacggacgagacggatcctgtgccgcgccgccgagcaggctattacccgtcgccgccgaacccggcggtcccgggaggcgtacggggccgaggccgggctgggggtggccggaacgggtttccgggccaggggggacggttttggcccgctccccttgttaacccaagggccctcccgcccgtggcaccaggccctgcggggtcttaagcacctacggattggcccccccgcgctcgttttggcggcgggactcgtcctgggggccgctatttggtgggtggttggtgctggcgcgcgcctataaaaaaggacgcaccgccgccctaatcgccagtgcgttccggacgccttcgccccacacagccctcccgaccgacacccccatatcgctccccgacctccggtcccgatggccgtcccgcaatttcaccgccccagcaccgttaccaccgatagcgtccgggcgcttggcatgcgcgggctcgtcttggccaccaataactctcagtttatcatggataacaaccacccacacccccagggcacccaaggggccgtgcgggagtttctccgcggtcaggcggcggcactgacggaccttggtctggcccacgcaaacaacacgtttaccccgcagcctatgttcgcgggcgacgcaccggccgcctggttgcggcccgcgtttggcctgcggcgcacctattcaccttttgtcgttcgagaaccttcgacgcccgggaccccgtgaggcccagggagttccttctggggtgttttaatcaataaaagaccacaccaacgcacgagccttgcgtttaatgtcgtgtttattcaagggagtgggatagggttcgacggttcgaaacttaacacaccaaataatcgagcgcgtctagcccagtaacatgcgcacgtgatgtaggctggtcagcacggcgtcgctgtgatgaagcagcgcccggcgggtccgctgtaactgctgttgtaggcggtaacaggcgcggatcagcaccgccagggcgctacgaccggtgcgttgcacgtagcgtcgcgacagaactgcgtttgccgatacgggcggggggccgaattgtaagcgcgtcacctcttgggagtcatcggcgtataacgcactgaatggttcgttggttatgggggagtgtggttccccagggagtgggtcgagcgcctcggcctcggaatccgagaggaacaacgaggtggcgtcggagtcttcgtcgtcagagacatacagggtctgaagcagcgacacgggcgtgggggtagcgtcgatgtgtagcgcgagggaggatgcccacgaagacaccccagacaaggagctgcccgtgcgtggatttgtggaagacgcggaagccgggacggatgggcggttttgcggtgcccggaaccgaaccgccggatactccccgggtgctacatgcccgttttggggctggggttggggctggggcgcggacaggcggctgacggtcaaatgcccccgggggcgcgcagatgtggcgggcgtggccaccggctgccgtgtagtggggcggcgggaaaccgggcctccgggcgtaacaccgccctccagcgtcaagtatgtggggggcgggcctgacgtcgggggcggggtgacgggttggaccgcgggaggcgggggagagggacctgcgggagaggatgaggtcggctcggccgggttgcggcctaaaacaggggccgtggggtcggcggggtcccagggtgaagggagggattcccgcgattcggacagcgacgcgacagcggggcgcgtaaggcgccgctgcggcccgcctacgggaaccctggggggggttggcgcgggacccgaggttagcggggggcggcggttttcgcccccgggcaaaaccgtgccggttgcgaccgggggcggaacgggatcgatagggagagcgggagaagcctggccggcggactggggaccgagcgggaggggcacaccagacaccaaagcgtggggcgctggctctgggggtttgggaggggccggggggcgcgcgaaatcggtaaccggggcgaccgtgtcggggagggcaggcggccgccaaccctgggtggtcgcggaagcctgggtggcgcgcgccagggagcgtgcccggcggtgtcggcgcgcgcgcgacccggacgaagaagcggcagaagcgcgggaggaggcgggggggcggggggcggtggcatcggggggcgccggggaactttggggggacggcaagcgccggacgtcgtcgcgggggcccacgggcgccggccgcgtgctttcggccgggacgcccggtcgtgcttcgcgagccgtgactgccggcccagggggccgcggtgcacactgggatgtggggacggactgatcggcggtgggcgaaagggggtccggggcaaggaggggcgcggggccgccggagtcgtcagacgcgagctcctccaggccgtgaatccatgcccacatgcgaggggggacgggctcgccgggggtggcgtcggtgaatagcgtgggggccaggcttccgggccccaacgagccctccgtcccaacaaggtccgccgggccgggggtcgggttcgggaccgaggggctctggtcgtcgggggcgcgctggtacaccggatgccccgggaatagctcccccgacaggagggaggcgtcgaacggccgcccgaggatagctcgtgcgaggaaggggtcctcgtcggtggcgctggcggcgaggacgtcctcgccgcccgccacaaacgggagctcctcggtggcctcgctgccaacaaaccgcacgtcgggggggccggggggtccgggttttcccacaacaccgcgaccggggtcatggagatgtccacgagcaccagacacggcgggccccgggcgaggggccgctcggcgatgagcgcggacaggcgcgggagctgtgccgccagacacgcgttttcgatcgggttcaggtcggcgtgcaggaggcggacggcccacgtctcgatgtcggacgacacggcatcgcgcaaggcggcgtccggcccgcgagcgcgtgagtcaaacagcgtgaggcacagctccagctccgactcgcgggaaaaggccgtggtgttgcggagcgccacgacgacgggcgcgcccaggagcactgccgccagcaccaggtccatggccgtaacgcgcgccgcgggggtgcggtgggtggcggcggccggcacggcgacgtgctggcccgtgggccggtagagggcgttggggggagcggggggtgacgcctcgcgcccccccgaggggctcagcgtctgcccagattccagacgcgcggtcagaagggcgtcgaaactgtcatactctgtgtagtcgtccggaaacatgcaggtccaaagagcggccagcgcggtgcttgggagacacatgcgcccgaggacgctcaccgccgccagcgcctgggcgggactcagctttcccagcgcggcgccgcgctcggttcccagctcggggaccgagcgccagggcgccagggggtcggtttcggacaacttgccgcggcgccagtctgccagccgcgtgccgaacatgaggccccgggtcggagggcctccggccgaaaacgctggcagcacgcggatgcgggcgtctggatgcggggtcaggcgctgcacgaatagcatggaatctgctgcgttctgaaacgcacgggggagggtgagatgcatgtactcgtgttggcggaccagatccaggcgccaaaaggtgtaaatgtgttccggggagctggccaccagcgccaccagcacgtcgttctcgttaaaggaaacgcggtgcctagtggagctctggggtccgagcggcggccccggggccgccgcgtcacccccccattccagctgggcccagcgacacccaaactcgcgcgtgagagtggtcgcgacgagggcgacgtagagctcggccgccgcatccatcgaggccccccatctcgcctggcggtggcgcacaaagcgtccgaagagctgaaagttggcggcctgggcgtcgctgagggccagctgaagccggttgatgacggtgaggacgtacatggccgtgacggtcgaggccgactccagggtgtccgtcggaagcggggggcgaatgcatgccgcctcgggacacatcagcagcgcgccgagcttgtcggtcacggccgggaagcagagcgcgtactgcagtggcgttccatccgggaccaaaaagctgggggcgaacggccgatccagcgtactggtggcctcgcgcagcaccaggggccccgggcctccgctcactcgcaggtacgcctcgccccggcggcgcagcatctgcgggtcggcctcttggccgggtggggcggacgcccgggcgcgggcgtctagggcgcgaagatccacgagcaggggcgcgggcgcggcggccgcgcccgcgcccgtctggcctgtggccttggcgtacgcgctatataagcccatgcggcgttggatgagctcccgcgcgccccggaactcctccatcgcccatggggccaggtccccggccaccgcgtcgaattccgccaacaggccccccagggtatcaaagttcatctcccaggccacccttggcaccacctcgtcccgcagccgggcgctcaggtcggcgtgttgggccacgcgccccccgagctcctccacggccccggcccgctcggcgctcttggcgcccaggacgccctggtacttggcgggaaggcgctcgtagtcccgctgggctcgcagccccgacacagtgttggtggtgtcctgcagggcgcgaagctgctcgcatgccgcgcgaaatccctcgggcgatttccaggcccccccgcgaacgcggccgaagcgaccccatacctcgtcccactccgcctcggcctcctcgagagacctccgcagggcctcgacgcggcgacgggtgtcgaagagcgcctgcaggcgcgcgccctgtcgcgtcaggaggcccgggccgtcgctgctggccgcgcttagcgggtgcgtctcaaaggtacgctgggcatgttccaaccaggcgaccgcctgcacgtcgagctcgcgcgccttctccgtctggtccaacagaatttcgacctgatccgcgatctcctccgccgagcgcgcctggtccagcgtcttggccacggtcgccgggacggcgaccaccttcagcagggtcttcagattggccagaccctcggcctcgagctgggcccggcgctcgcgcgcggccagcacatcccgcagccccgccgtgacccgctcggtggcttcggcgcgctgctgtttggcgcgcaccacggcgtccttggtatcggccaggtcctgtcgggtcacgaatgcgacgtagtcggagtacgccgtgtccttcacggggctctggtccacgcgctccagcgccgccacgcacgccaccagcgcgtcctcgctcgggcagggcagggtgacccctgcccggacaagctcggcggccgccgccgggtcgttgcgcaccgcggatatctcctccgcggcggcggccaggtccagcgccacgcttccgatcgcgcgccgcgcgtcggcccggagggcgtccaggcgatcgcggatatccacgtactcggcgtagcccttttgaaaaaacggcacgtactggcgcagggccggcacgccccccaagtcttccgacaggtgtagtacggcctcgtggtagtcgataaacccgtcgttcgcctgggcccgctccagcagcccccccgcgagccgcagaagccgcgccaggggctcggtgtccacccgaaacatgtcggcgtacgtgtcggccgcggccccaaaggccgcgctccagtcgatgcggtgaatggctgcgagcggggggagcatggggtggcgctggttctcgggggtgtatgggttaaacgcaagggccgtctccagggcaagggtcaccgccttggcgttggttcccagcgcctgctcggcccgctttcggaagtcccgggggttgtagccgtgcgtgcccgccagcgcctgcaggcgacggagctcgaccacgtcaaactcggcactgctttccacgcggtccagcacggcctccacgtcggcggcccagcgctcgtggctactgcgggcgcgctgggccgccatcttctctctgaggtcggcggtggcggcctcaagttcgtcggcgcggcgtcgcgtggcgccgatgacctttcccagctcctgcagggcgcgcccgctgggggagtggtccccggccgtcccttcggcgtgcaacaggcccccgaacctgccctcgtggcccgcgaggctttcccgcgcgccggtggtcgcgcgcgtcgcggcttggatcagggaggcatgctctcccttcggttggttggcggcccggcgcacctggacgacaaggtcggcggcagccgaccctaaggtcgtgagctgggcgatggccccccgcgcgtccagggccaaccgagtcgccttgacgtatcccgcggcgctgtcggccatggccgctaggaaggccaggggggaggccgggtcgctggcggccgcgcccagggccgtcaccgcgtcgaccaggacgcggtgcgcccgcacggccgcatccaccgtcgacgcggggtctgccgtcgcgacggcggcgctgccggcgttgatggcgttcgagacggcgtgggctatgatcggggcgtgatcggcgaagaactgcaagagaaacggagtctcgggggcgtcggcgaacaggttcttcagcaccaccacgaagctgggatgcaagccggacagagccgtcgccgtgtccggagtcgggtgctccagggcatctcggtactgccccagcagcccccacatgtccgcccgcagcgccgccgtaacctcagggggcgccccccgaacggcctcggggaggtccgaccagcccgccggcagggaggcccgcagggtcgccaggacggccggacaggcctttagccccacaaagtcagggagggggcgcaggaccccctggagtttgtgcaagaacttctcccgggcgtcgcgggccaccttcgcccgctcccgcgctccctcgagcattgcctccagggagcgcgcgcgctcccgcaaacggacacgcgcatcgggggcgagctctgccgtcagcttggcggcatccatggcccgcgcctgccgcagcgcttcctcggccatgcgcgtggcctctggcgacagcccgccgtcgtcggggtagggcgacgcgccgggcgcaggaacaaaggccgcgtcgctgtccagctgctggcccagggccgcatctagggcgtcgaagcgccgcagctcggccagacccgagctgcggcgcgcctgctggtcgttaatgtcgcggatgctgcgcgccagctcgtccagcggcttgcgttctatcagcccttggttggcggcgtccgtcaggacggagagccaggccgccaggtcctcgggggcgtccagcgtctggccccgctgtatcagatcccgcaacaggatggccgtggggctggtcgcgatcgggggcggggcgggaatggcggcgcgctgcgcgatgtcccgcgtgtgctggtcgaagacaggcagggactcgagcagctggaccacgggcacgacggcggccgaagccacgtgaaaccggcggtcgttgttgtcgctggcctgtagagccttggcgctgtatacggccccccggtaaaagtactccttaaccgccccctcgatcgcccgacgggcctgggtccgcacctcctccagccgaacctgaacggcctcggggcccagggggggtgggcgcggagccccctgcggggccgccccggccggggcgggcattacgccgaggggcccggcgtgctgtgagaccgcgtcgaccccgcgagcgagggcgtcgagggcctcgcgcatctggcgatcctccgcctccaccctaatctcttcgccacgggcaaatttggccagagcctggactctatacagaagcggttctgggtgcgtcggggtggcgggggcaaaaagggtgtccgggtgggcctgcgagcgctccagaagccactcgccgaggcgtgtatacagattggccggcggggccgcgcgaagctgcagctccaggtccgcgagttccccgtaaaaggcgtccgtctcccgaatgacatccctagccacaaggatcagcttcgccagcgccaggcgaccgatcagagagttttcgtccagcacgtgctggacgaggggcagatgggcggccacgtcggccaggctcaggcgcgtggaggccagaaagtcccccacggccgttttccggggcagcatgctcagggtaaactccaacagggcggcggccgggccggccaccccggcctgggtgtgcgtccgggccccgttctcgatgagaaaggcgaggacgcgttcaaagaaaaaaataacacagagctccagcagccccggagaagccggatacggcgaccgtaaggcgctgatggtgagccgcgaacacgcggcgacctcgcgggccagggcggcggagcacgcggtgaacttaaccgccgtggcggccacgtttgggtgggcctcgaacagctgggcaaggtctgcgcccgggggctcgggtgagcggcgagtcttcagcgcctcgagggcctgcgaggacgccggaaccgtgggcccgtcgtcctcgcccgcctcggcgaccggcggcccggccgggtcggggggtgccgaggcgaggacaggctccggaacggaggcggggaccgcggccccgacgggggttttgcctttgggggtggatttcttcttggttttggcagggggggccgagcgtttcgttttctcccccgaagtcaggtcttcgacgctggaaggcggagtccaggtgggtcggcggcgcttgggatggccggccgagtagcgtgcccggtgccgaccaaccgggacgacgcccatctccaggacccgcatgtcgtcgtcatcttcttcggccgcctctgcggcggggggcttgggggcggagggaggcggtggtgggatcgcggagggtgggtcggcggaggggggatccgtgggtggggtacccttcagggccaccgcccatacatcgtcgggcgcccgattcgggcgcttggcctctggttttgccgacggaccggccgtcccccgggatgtctcggaggccctgtcgtcgcgacgggcccgggtcggtggcggcgactgggcggctgtgggcgggtgtggccccgtgccccctaccccctcccgggggcccacgccgacgcagggctcccccaggcccgcgatctcgccccgcagggggtgcgtgatggccacgcgccgttcgctgaacgcttcgtcctgcaggtaagtctcgctggccccgtaaagatgcagagccgcggccgtcaagtccgcaggagccgcgggttccgggcccgacggcacgaaaaacaccatggctcccgcccaccgtacgtccgggcgatcgcgggtgtaatacgtcaggtatggatacatgtcccccgcccgcactttggcgatgaacgcgggggtgccctccggaaggccgtgcgggtcaaaaaggtatgcggtgtcgccgtccctgaacagccccatccctagggggccaatggttaggagcgtgtacgacagggggcgcagggcccacgggccggcgaagaacgtgtgtgcggggcattgtgtctccagcaggcccgccgcgggctccccgaagaagcccacctcgccgtatacgcgcgagaagacacagcgcagtccgccgcgcgcccctgggtactcgaggaagttggggagctcgacgatcgaacacatgcgcggcggcccagggcccgcggtcgcgcgcgtccactcgcccccctcgaccaaacaaccctcgatggcctccgcggacagaacgtcgcgagggcccacatcaaatatgaggctgagaaaggacagcgacgagcgcatgcacgataccgacccccccggctccaggtcgggcgcgaactggttccgagcaccggtgaccacgatgtcgcgatcccccccgcgttccatcgtggagtgcggtggggtgcccgcgatcatatgtgccctactggccagagacccggcctgtttatggaccggacccccggggttagtgttgtttccgccacccatgcccccgtaccatggccccggttcccctgattaggctacgagtcgcggtgatcgcttcccaaaaaccgagctgcgtttgtctgtcttgatcttcccccccccccccgcccgcccgcccgcccgcccgcccgcacaccataacaccgagaacaacacacgggggtgggcgtaacataataaagctttattggtaactagttaacggcaagtccgtgggtggcgcgacggtgtcctccgggctcatctcgtcgtcctcgacgggggtgttggaatgaggcgccccctcgcggtccgcctggcgtgggccgtgcccataggcctccggcttctgtgcgtccatgggcataggcgcggggagactgtttccggcgtcgcggacctccaggtccctgggagactccggtccggctaacggacgaaacgcggaagcgcgaaacacgccgtcggtgacccgcaggagctcgttcatcagtaaccaatccatactcagcgtaacggccagcccctggcgagacagatccacggagtccggaaccgcggtcgtctggcccagggggccgaggctgtagtccccccaggcccctaggtcgcgacggctcgtaagcacgacgcggtcggccgcggggctttgcgggggggcgtcctcgggcgcatgcgccattacctctcggatggccgcggcgcgctggtcggccgagctgaccaagggcgccacgaccacggcgcgctccgtctgcaggcccttccacgtgtcgtggagttcctggacaaactcggccacgggctcgggtcccgcggccgcgcgcgcggcttgatagcaggccgagagacgccgccagcgcgctagaaactgacccatgaagcaaaacccggggacctggtctcccgacagcagcttcgacgcccgggtgtgaatgccggacacaacggacagaaacccgtgaatttcgcgccggaccacggccagcacgttgtcctcgtgcgacacctgggccgccagctcgtcgcacacctccaggtgcgccgtggtttcggtgatgacggaacgcaggctcgcgagggacgcgaccagcgcgcgcttggcgtcgtgatacatgctgcagtactgactcaccgcgtcccccatggcctcggggggccagggccccaggcggtcgggagtgtccccgaccaccgcatacaggcggcgcccgtcgctctcgaaccgacactcgaaaaaggcggagagcgtgcgcatgtgcagccgcagcagcacgatggcgtcctccagttggcgaatcagggggtctgcgcgctcggcgaggtcctgcagcaccccccgggcggccagggcgtacatgctaatcaacaggaggctggtgcccacctcggggggcggggggggctgcagctggaccaggggccgcagctgctcgacggcacccctggagatcacgtacagctcccggagcagctgctctatgttgtcggccatctgcatagtggggccgaggccgccccgggcggccggttcgaggagggtaatcagcgcgcccagtttggtgcgatggccctcgaccgtggggagatagcccagcccaaagtcccgggcccaggccaacacacgcagggcgaactcgaccgggcgtggaaggtaggccgcgctacacgtggcccccaacgcgtccccgaccaccagggccagaacgtaggggacgaagcccgggtcggcgaggacgttggggtgaatgccctcgagggcggggaagcggatctgggtcgccgcggccaggtggacagagggggcgtggctgggctgcccgacggggagaagcgcggacagcggcgtggccggggtggtgggggtgatgtcccagtgggtctgaccatacacgtcgatccagatgagcgccgtctcgcggagaaggctgggttgaccggaactaaagcggcgctcggccgtctcaaactcccccacgagcgcccgccgcaggctcgccagatgttccgtcggcacggccggacccatgatacgcgccagtgtctggctcagaacgccccccgacaggccgaccgcctcgcagagccgcccgtgcgtgtgctcgctggcgccctggacccgcctgaaagtttttacgtagttggcatagtacccgtattcccgcgccagaccaaacacgttcgaccccgcgagggcaatgcacccaaagagctgctggacttcgccgagtccgtggccggcgggcgtccgcgcggggacgcccgccgccagaaacccctccagggccgaaaggtagtgcgtgcagtgcgagggcgtgaacccagcgtcgatcagggtgttgatcaccacggagggcgaattggtattctggatcaacgtccacgtctgctgcagcagagccagcagccgctgctgggcgccggcggagggctgctccccgagctgcagcaggctggagacggcaggctggaagactgccagtgccgacgaactcaggaacggcacgtcgggatcaaacacggccacgtccgtccgcacgcgcgccattagcgtccccgggggcgcacaggccgagcgcgggctgacgcggctgagggccgtcgacacgcgcacctcctcgcggctgcgaaccatcttgttggcctccagtggcggaatcattatggccgggtcgatctcccgcacggtgtgctgaaactgcgccaacaggggcggcgggaccacagccccccgctcgggggtcgtcaggtactcgtccaccagggccaacgtaaagagggcccgtgtgaggggagtgagggtcgcgtcgtctatgcgctggaggtgcgccgagaacagcgtcacccgattactcaccagggccaagaaccggaggccctcttgcacgaacggggcggggaagagcaggctgtacgccggggtggtaaggttcgcgctgggctgccccaacgggaccggcgccatcttgagtgacgtctccccaagggcctcgatggaggtccgcgggctcatggccaagcagctcttggtgacggtttgccagcggtctatccactccacggcgcactggcggacgcggaccggccccagggccgccgcggtgcgcaggccggcggaatccagcgcatgggacgtgtcggagccggtgaccgcgaggatggtgtccttgatgacctccatctcccggaaggcctggtcgggggcctcggggagagccaccaccaagcggtgtacgagcaacccggggaggttctcggccaagagcgccgtctccggaagcccgtgggcccggtggagcgcgcacaggtgttccagcagcggccgccagcatgcccgcgcgtctaccggggcaatggccgttcccgacaacagaaacgccgccatggcggcgcgcagcttggccgtggccagaaacgccgggtcgtccgccccgtttgccgtctcggccgtgggggttggcggttggcgaaggccggctaggctcgccaataggcgctgcataggtccgtccgagggcggaccggcgggtgaggtcgtgacgacgggggcctcggacgggagaccgcggtctgccatgacgcccggctcgcgtgggtgggggacagcgtagaccaacgacgagatcgggcgggaatgactgtcgtgcgctgtagggagcggcgaattatcgatcccccgcggccctccaggaaccccgcaggcgttgcgagtaccccgcgtcttcgcggggtgttatacggccacttaagtcccggcatcccgttcgcggacccaggcccgggggattgtccggatgtgcgggcagcccggacggcgtgggttgcggactttctgcggggcggcccaaatggccctttaaacgtgtgtatacggacgcgccgggccagtcggccaacacaacccaccggaggcggtagccgcgtttggctgtggggtgggtggttccgccttgcgtgagtgtcctttcgacccccctcccccgggttttgttaggtcgcgatctgcagtcgcaatgaagaccaatccgctacccgcaaccccttccgtgtggggcgggagtaccgtggaactcccccccaccacacgcgataccgcgggacagggcctgcttcggcgcgtcctgcgccccccgatctctcgccgcgacggcccagtgctccccagggggtcgggaccccggagggcggccagcacgctgtggttgcttggcctggacggcacagacgcgccccctggggcgctgacccccaacgacgataccgaacaggccctggacaagatcctgcggggcaccatgcgcgggggggcggccctgatctgctccccgcgccatcatctaacccgccaagtgatcctgacggatctgtgccaacccaacgcggatcgtgccgggacgctgcttctggcgctgcggcaccccgccgacctgcctcacctggcccaccagcgcgccccgccaggccggcagaccgagcggctgggcgaggcctggggccagctgatggaggcgaccgccctggggtcggggcgagccgagagcgggtgcacgcgcgcgggcctcgtgtcgtttaacttcctggtggcggcgtgtgccgcctcgtacgacgcgcgcgacgccgccgatgcggtacgggcccacgtcacggccaactaccgcgggacgcgggtgggggcgcgcctggatcgtttttccgagtgtctgcgcgccatggttcacacgcacgtcttcccccacgaggtcatgcggtttttcggggggctggtgtcgtgggtcacccaggacgagctagcgagcgtcaccgccgtgtgcgccgggccacaggaggcggcgcacaccggccacccgggccggccccgctcggccgtgatcctcccggcgtgtgcgttcgtggacctggacgccgagctggggctggggggcccgggtgcggcgtttctgtacctggtattcacttaccgccagcgccgggaccaggagctgtgttgtgtgtacgtgatcaagagccagctccccccgcgcgggttggagccggccctggagcggctgtttgggcgcctccggatcaccaacacgattcacggcaccgaggacatgacgcccccggccccaaaccgaaaccccgacttccccctcgcgggcctggccgccaatccccaaaccccgcgttgctcggctggccaggtcacgaacccccagttcgccgacaggctgtaccgctggcagccggacctgcgggggcgccccaccgcacgcacctgtacgtacgccgcctttgcagagctcggcatgatgcccgaggatagtccccgctgcctgcaccgcaccgagcgctttggggcggtcagcgtccccgttgtcatcctggaaggcgtggtgtggcgccccggcgagtggcgggcatgcgcgtgagcgtagcaaacgccccgcccacacaacgctccgcccccaaccccttccccgctgtcactcgtggttcgttgacccggacgtccgccaaataaagccactgaaacccgaaacgcgagtgttgtaacgtcctttgggcgggaggaagccacaaaatgcaaatgggatacatggaaggaacacacccccgtgactcaggacatcggcgtgtccttttgggtttcactgaaactggcccgcgccccacccctgcgcgatgtggataaaaagccagcgcgggtggtttagggtaccacaggtgggtgctttggaaacttgtcggtcgccgtgctcctgtgagcttgcgtccctccccggtttcctttgcgctcccgccttccggacctgctcttgcctatcttctttggctctcggtgcgattcgtcaggcagcggccttgtcgaatctcgaccccaccactcgccggacccgccgacgtcccctctcgagcccaccgaaacccgccgcgtctgttgaaatggccagccgcccagccgcatcctctcccgtcgaagcgcgggccccggttgggggacaggaggccggcggccccagcgcagccacccagggggaggccgccggggcccctctcgcccacggccaccacgtgtactgccagcgagtcaatggcgtgatggtgctttccgacaagacgcccgggtccgcgtcctaccgcatcagcgatagcaactttgtccaatgtggttccaactgcaccatgatcatcgacggagacgtggtgcgcgggcgcccccaggacccgggggccgcggcatcccccgctcccttcgttgcggtgacaaacatcggagccggcagcgacggcgggaccgccgtcgtggcattcgggggaaccccacgtcgctcggcggggacgtctaccggtacccagacggccgacgtccccaccgaggcccttgggggcccccctcctcctccccgcttcaccctgggtggcggctgttgttcctgtcgcgacacacggcgccgctctgcggtattcgggggggagggggatccagtcggccccgcggagttcgtctcggacgaccggtcgtccgattccgactcggatgactcggaggacacggactcggagacgctgtcacacgcctcctcggacgtgtccggcggggccacgtacgacgacgcccttgactccgattcgtcatcggatgactccctgcagatagatggccccgtgtgtcgcccgtggagcaatgacaccgcgcccctggatgtttgccccgggacccccggcccgggcgccgacgccggtggtccctcagcggtagacccacacgcgccgacgccagaggccggcgctggtcttgcggccgatcccgccgtggcccgggacgacgcggaggggctttcggacccccggccacgtctgggaacgggcacggcctaccccgtccccctggaactcacgcccgagaacgcggaggccgtggcgcgctttctgggagatgccgtgaaccgcgaacccgcgctcatgctggagtacttttgccggtgcgcccgcgaggaaaccaagcgtgtcccccccaggacattcggcagcccccctcgcctcacggaggacgactttgggcttctcaactacgcgctcgtggagatgcagcgcctgtgtctggacgttcctccggtcccgccgaacgcatacatgccctattatctcagggagtatgtgacgcggctggtcaacgggttcaagccgctggtgagccggtccgctcgcctttaccgcatcctgggggttctggtgcacctgcggatccggacccgggaggcctcctttgaggagtggctgcgatccaaggaagtggccctggattttggcctgacggaaaggcttcgcgagcacgaagcccagctggtgatcctggcccaggctctggaccattacgactgtctgatccacagcacaccacacacgctggtcgagcgggggctgcaatcggccctgaagtatgaggagttttacctaaagcgttttggcgggcactacatggagtccgtcttccagatgtacacccgcatcgccggctttttggcctgccgggccacgcgcggcatgcgccacatcgccctggggcgagaggggtcgtggtgggaaatgttcaagttctttttccaccgcctctacgaccaccagatcgtaccgtcgacccccgccatgctgaacctggggacccgcaactactacacctccagctgctacctggtaaacccccaggccaccacaaacaaggcgaccctgcgggccatcaccagcaacgtcagtgccatcctcgcccgcaacgggggcatcgggctatgcgtgcaggcgtttaacgactccggccccgggaccgccagcgtcatgcccgccctcaaggtccttgactcgctggtggcggcgcacaacaaagagagcgcgcgtccgaccggcgcgtgcgtgtacctggagccgtggcacaccgacgtgcgggccgtgctccggatgaagggggtcctcgccggcgaagaggcccagcgctgcgacaatatcttcagcgccctctggatgccagacctgtttttcaagcgcctgattcgccacctggacggcgagaagaacgtcacatggaccctgttcgaccgggacaccagcatgtcgctcgccgactttcacggggaggagttcgagaagctctaccagcacctcgaggtcatggggttcggcgagcagatacccatccaggagctggcctatggcattgtgcgcagcgcggccacgaccgggagccccttcgtcatgttcaaagacgcggtgaaccgccactacatctacgacacccagggggcggccatcgccggctccaacctctgcaccgagatcgtccatccggcctccaagcgatccagtggggtctgcaacctgggaagcgtgaatctggcccgatgcgtctccaggcagacgtttgactttgggcggctccgcgacgccgtgcaggcgtgcgtgctgatggtgaacatcatgatcgacagcacgctacaacccacgccccagtgcacccgcggcaacgacaacctgcggtccatgggaatcggcatgcagggcctgcacacggcctgcctgaagctggggctggatctggagtctgccgaatttcaggacctgaacaaacacatcgccgaggtgatgctgctgtcggcgatgaagaccagcaacgcgctgtgcgttcgcggggcccgtcccttcaaccactttaagcgcagcatgtatcgcgccggccgctttcactgggagcgctttccggacgcccggccgcggtacgagggcgagtgggagatgctacgccagagcatgatgaaacacggcctgcgcaacagccagtttgtcgcgctgatgcccaccgccgcctcggcgcagatctcggacgtcagcgagggctttgcccccctgttcaccaacctgttcagcaaggtgacccgggacggcgagacgctgcgccccaacacgctcctgctaaaggaactggaacgcacgtttagcgggaagcgcctcctggaggtgatggacagtctcgacgccaagcagtggtccgtggcgcaggcgctcccgtgcctggagcccacccaccccctccggcgattcaagaccgcgtttgactacgaccagaagttgttgatcgacctgtgtgcggaccgcgccccctacgtcgaccatagccaatccatgaccctgtatgtcacggagaaggcggacgggaccctcccagcctccaccctggtccgccttctggtccacgcatataagcgcggactaaaaacagggatgtactactgcaaggttcgcaaggcgaccaacagcggggtctttggcggcgacgacaacattgtctgcacgagctgcgcgctgtgaccgacaaaccccctccgcgccaggcccgccgccactgtcgtcgccgtcccacgctctcccctgctgccatggattccgcggccccagccctctcccccgctctgacggcccttacgggccagagcgcgacggcggacctggcgatccagattccaaagtgccccgaccccgagaggtacttctacacctcccagtgtcccgacattaaccacctgcgctccctcagcatccttaaccgctggctggaaaccgagcttgttttcgtgggggacgaggaggacgtctccaagctttccgagggcgagctcagcttttaccgcttcctcttcgctttcctgtcggccgccgacgacctggttacggaaaacctgggcggcctctccggcctgtttgagcagaaggacattctccactactacgtggagcaggaatgcatcgaagtcgtacactcgcgcgtgtacaacatcatccagctggtgcttttccacaacaacgaccaggcgcgccgcgagtacgtggccggcaccatcaaccacccggccatccgcgccaaggtggactggttggaagcgcgggtgcgggaatgcgcctccgttccggaaaagttcattctcatgatcctcatcgagggcatcttttttgccgcctcgtttgccgccatcgcctaccttcgcaccaacaaccttctgcgggtcacctgccagtcaaacgacctcatcagccgggacgaggccgtgcacacgacggcctcgtgttacatctacaacaactacctcggcgggcacgccaagcccccgcccgaccgcgtgtacgggctgttccgccaggcggtcgagatcgagatcggatttatccgatcccaggcgccgacggacagccatatcctgagcccggcggcgctggcggccatcgaaaactacgtgcgattcagcgcggatcgcctgttgggccttatccacatgaagccactgttttccgccccaccccccgacgccagctttccgctgagcctcatgtccaccgacaaacacaccaattttttcgagtgtcgcagcacctcctacgccggggcggtcgtcaacgatctgtgagtgtcgcggcgcgcttctacccgtgtttgcccataataaacctctgaaccaaactttgggtctcattgtgattcttgtcagggacgcgggggtgggagaggataaaaggcggcgcaaaaagcagtaaccaggtccgtccagattctgcgggcatagaataccataattttattggtgggtcgtttgttcggggacaagcgcgctcgtctgacgtttgggctactcgtcccagaatttggccaggacgtccttgtagaacgcgggtgggggggcctgggtccgcaactgctccagaaacctgtcggcgatatcaggggccgtgatatgccgggtcacgatagatcgcgccaggttttcgtcgcggatgtcctggtagataggcaggcgtttcagaagagtccacggcccccgctccttggggccgataagcgatatgacgtacttaatgtagcggtgttccaccagctcggtgatggtcatgggatcggggagccagtccagggactctggggcgtcgtggatgacgtggcgtcgccggttggccacataactgcggtgctcttccagcagctgcgcgttcgggacctggacgagctcgggcggggtgagtatctccgaggaggacgacctggggccggggtggcccccggtaacgtcccggggatccagggggaggtcctcgtcgtcttcgtatccgccggcgatctgttgggttagaatttcggtccacgagacgcgcgtctcggtgccgccggcggccggcggcagagggggcctggtttccgtggagcgcgagctggtgtgttcccggcggatggcccgccgggtctgagagcgactcgggggggtccagtgacattcgcgcagcacatcctccacggaggcgtaggtgttattgggatggaggtcggtgtggcagcggacaaagagggccaggaactgggggtagctcatcttaaagtacttcagtatatcgcgacagttgatcgtgggaatgtagcaggcgctaatatccaacacaatatcacagcccatcaacaggaggtcagtgtccgtggtgtacacgtacgcgaccgtgttggtgtgatagaggttggcgcaggcatcgtccgcctccaactgacccgagttaatgtaggcgtaccccagggcccggagaacgcgaatacagaacagatgcgccagacgcagggccggcttcgagggcgcggcggacggcagcgcggctccggacccggccgtcccccgggtccccgaggccagagaggtgccgcgtcggcgcatgttggaaaaggcagagctgggtctggagtcggtgatgggggaaggcggtggagaggcgtccacgtcactggcctcctcgtccgtccggcactgggccgtcgtgcgggccaggatggccttggctccaaacacaaccggctccatacaattgaccccgcgatcggtaacgaagatggggaaaagggacttttgggtaaacacctttaataagcgacagaggcagtgtagcgtaatggcctcgcggtcgtaactggggtatcggcgctgatatttgaccaccaacgtgtacatgacgttccacaggtccacggcaatgggggtgaagtacccggccggggccccaaggccccggcgcttgaccagatggtgtgtgtgggcaaacttcatcatcccgaacaaacccatgtcaggtcgattgtaactgcggatcggcctaactaaggcgtggttggtgcgacggtccgggacacccgagcctgtctctctgtgtatggtgacccagacaacaacaccgacacaagaggacaataatccgttaggggacgctctttataatttcgatggcccaactccacgcggattggtgcagcaccctgcatgcgccggtgcgggccaaccttccccccgctcattgcctcttccaaaagggtgtggcctaacgagctgggggcgtatttaatcaggctagcgcggcgggcctgccgtagtttctggctcggtgagcgacggtccggttgcttgggtcccctggctgccatcaaaaccccaccctcgcagcggcatacgccccctccgcgtcccgcacccgagaccccggcccggctgccctcaccaccgaagcccacctcgtcactgtggggtgttcccagcccgcgttgggatgacggattcccctggcggtgtggcccccgcctcccacgtggaggacgcgtcggacgcgtccctcgggcagccggaggagggggcgccctgccaggtggtcctgcagggcgccgaacttaatggaatcctacaggcgtttgccccgctgcgcacgagccttctggactcgcttctggttatgggcgaccggggcatccttatccataacacgatctttggggagcaggtgttcctgcccctggaacactcgcaattcagtcggtatcgctggcgcggacccacggcggcgttcctgtctctcgtggaccagaagcgctccctcctgagcgtgtttcgcgccaaccagtacccggacctacgtcgggtggagttggcgatcacgggccaggccccgtttcgcacgctggttcagcgcatatggacgacgacgtccgacggcgaggccgttgagctagccagcgagacgctgatgaagcgcgaactgacgagctttgtggtgctggttccccagggaacccccgacgttcagttgcgcctgacgaggccgcagctcaccaaggtccttaacgcgaccggggccgatagtgccacgcccaccacgttcgagctcggggttaacggcaaaatttccgtgttcaccacgagtacctgcgtcacatttgctgcccgcgaggagggcgtgtcgtccagcaccagcacccaggtccagatcctgtccaacgcgctcaccaaggcgggccaggcggccgccaacgccaagacggtgtacggggaaaatacccatcgcaccttctctgtggtcgtcgacgattgcagcatgcgggcggtgctccggcgactgcaggtcggcgggggcaccctcaagttcttcctcacgacccccgtccccagtctgtgcgtcaccgccaccggtcccaacgctgtatcggcggtatttctcctgaaaccccagaagatttgcctggactggctgggtcatagccaggggtctccttcagccgggagctcggcctcccgggcctctgggagcgagccaacagacagcaaggactccgcgtcggacgcggtcagccacggcgatccggaagacctcgatggcgctgcccgggcgggagaggcgggggcctcgcacgcctgtccgatgccgtcgtcgaccacgcgggtcactcccacgaccaagcgggggcgctcggggggcgaggatgcgcgcgcggacacggccctaaagaaacctaagacggggtcgcccaccgcacccccgcccgcagatccagtccccctggacacggaggacgactccgatgcggcggacgggacggcggcccgtcccgccgctccagacgcccggagcggaagccgttacgcgtgttactttcgcgacctcccgaccggagaagcaagccccggcgccttctccgccttccggggggggccccaaaccccgtatggttttggattcccctgacggggcggggccttggcggccgcccaactctcgcaccatcccgggttaatgtaaataaacttggtattgcccaacactctcccgcgtgtcgcgtgtggttcatgtgtgtgcctggcgtcccccaccctcgggttcgtgtatttcctttccctgtccttataaaagccgtatgtggggcgctgacggaaccaccccgcgtgccatcacggccaaggcgcgggatgctccgcaacgacagccaccgggccgcgtccccggaggacggccagggacgggtcgacgacggacggccacacctcgcgtgcgtgggggccctggcgcgggggttcatgcatatctggcttcaggccgccacgctgggttttgcgggatcggtcgttatgtcgcgcgggccgtacgcgaatgccgcgtctggggcgttcgccgtcgggtgcgccgtgctgggctttatgcgcgcaccccctcccctcgcgcggcccaccgcgcggatatacgcctggctcaaactggcggccggtggagcggcccttgttctgtggagtctcggggagcccggcacgcagccgggggccccggccccgggcccggccacccagtgcctggcgctgggcgccgcctatgcggcgctcctggtgctcgccgatgacgtctatccgctctttctcctcgccccggggcccctgttcgtcggcaccctggggatggtcgtcggcgggctgacgatcggaggcagcgcgcgctactggtggatcggtgggcccgccgcggccgccttggccgcggcggtgttggcgggcccgggggcgaccaccgccagggactgcttctccagggcgtgccccgaccaccgccgcgtctgcgtcatcgtcgcaggcgagtctgtttcccgccgccccccggaggacccagagcgacccggggaccccgggccaccgtcccccccgacaccccaacgatcccaggggccgccggccgatgaggtcgcaccggccggggtagcgcggcccgaaaacgtctgggtgcccgtggtcacctttctgggggcgggcgcgctcgccgtcaagacggtgcgagaacatgcccggggaacgccgggcccgggcctgccgctgtggccccaggtgtttctcggaggccatgtggcggtggccctgacggagctgtgtcaggcgcttgcgccctgggaccttacggacccgctgctgtttgttcacgccggactgcaggtcatcaacctcgggttggtgtttcggttttccgaggttgtcgtgtatgcggcgctagggggtgccgtgtggatttcgttggcgcaggtgctggggctccggcgtcgcctgcgcaggaaggaccccggggacggggcccggttggcggcgacgcttcggggcctcttcttctccgtgtacgcgctggggtttggggtgggggcgctgctgtgccctccggggtcaacgggcgggcggtcgggcgattgatatatttttcaataaaaggcattagtcccgaagaccgccggtgtgtgatgatttcgccataacacccaaaccccggatggggcccgggtataaattccggaaggggacacgggctaccctcactaccgagggcgcttggtcgggaggccgcatcgaacgcacacccccatccggtggtccgtgtggaggtcgttttcagtgcccggtctcgctttgccgggaacgctagccgatccctcgcgagggggaggcgtagggcatggccccggggcgggtgggccttgccgtggtcctgtggagcctgttgtggctcggggcgggggtgtccgggggctcggaaactgcctccaccgggcccacgatcaccgcgggagcggtgacgaacgcgagcgaggcccccacatcggggtcccccgggtcagccgccagcccggaagtcacccccacatcgaccccaaaccccaacaatgtcacacaaaacaaaaccacccccaccgagccggccagccccccaacaacccccaagcccacctccacgcccaaaagcccccccacgtccacccccgaccccaaacccaagaacaacaccacccccgccaagtcgggccgccccactaaaccccccgggcccgtgtggtgcgaccgccgcgacccattggcccggtacggctcgcgggtgcagatccgatgccggtttcggaattccacccgcatggagttccgcctccagatatggcgttactccatgggtccgtcccccccaatcgctccggctcccgacctagaggaggtcctgacgaacatcaccgccccacccgggggactcctggtgtacgacagcgcccccaacctgacggacccccacgtgctctgggcggagggggccggcccgggtgccgaccctccgttgtattctgtcaccgggccgctgccgacccagcggctgattatcggcgaggtgacgcccgcgacccagggaatgtattacttggcctggggccggatggacagcccgcacgagtacgggacgtgggtgcgcgtccgcatgttccgccccccgtctctgaccctccagccccacgcggtgatggagggtcagccgttcaaggcgacgtgcacggccgacgcctactacccgcgtaaccccgtggagttggtctggttcgaggacgaccgccaggtgtttaacccgggccagatcgacacgcagacgcacgagcaccccgacgggttcaccaccgtctctaccgtgacctccgaggctgtcggcggccaggtccccccgcggaccttcacctgccagatgacgtggcaccgcgactccgtgacattctcgcgacgcaatgccaccgggctggccctggtgctgccgcggccaaccatcaccatggaatttggggtccggcatgtggtctgcacggccggctgcgtccccgagggcgtgacgtttgcctggttcctgggggacgacccctcaccggcggctaagtcggccgttacggcccaggagtcatgcgaccaccccgggctggctacggtccggtccaccctgcccatttcgtacgactacagcgagtacatctgtcggttgaccggatatccggccgggattcccgttctagaacaccacggcagtcaccagcccccacccagggaccccaccgagcggcaggtgatcgaggcgatcgagtgggtggggattggaatcggggttctcgcggcgggggtcctggtcgtaacggcgatcgtgtacgtcgtccgcacatcacagtcgcggcagcgtcatcggcggtaacgcgagacccccccgttacctttttaatatctatatagtttggtcccccctctatcccgcccaccgctgggcgctataaagccgccaccctctcttccctcaggtcatccttggtcgatcccgaacgacacacggcgtggagcaaaacgcctccccctgagccgctttcctaccaacacaccggcatgcctctgcgggcatcggaacacgcctaccggcccctgggccccgggacaccccccatgcgggctcggctccccgccgcggcctgggttggcgtcgggaccatcatcgggggagttgtgatcattgccgcgttggtcctcgtgccctcgcgggcctcgtgggcactttccccatgcgacagcggatggcacgagttcaacctcgggtgcatatcctgggatccgacccccatggagcacgagcaggcggtcggcggctgtagcgccccggcgaccctgatcccccgcgcggctgccaaacagctggccgccgtcgcacgcgtccagtcggcaagatcctcgggctactggtgggtgagcggagacggcattcgggcctgcctgcggctcgtcgacggcgtcggcggtattgaccagttttgcgaggagcccgcccttcgcatatgctactatccccgcagtcccgggggctttgttcagtttgtaacttcgacccgcaacgcgctggggctgccgtgaggcgcgtgtactgcggtctgtctcgtctcctcttctccccttccctccccctccgcatcccaggatcacaccggccaacgagggttggggggtccggcacggacccaaaataataaacacacaatcacgtgcgataaaaagaacacgcggtcccctgtggtgtttttggttatttttattaaatctcgtcgacaaacagggggaaaggggcgtggtctagcgacggcagcacgggcggaggcgttcaccggctccggcgtccttcgcgtttaagcttggtcaggagggcgctcagggcggcgacgttggtcgggccgtcgttggtcagggcgttggctcgatggcgggcgaggacgggcgaggggctcaacggcgggggcgggggcccggtgcggcccgggggggaaaatagggcggatcccccccagtcgtacaggggattttccgcctcaatgtacggggaggccggcgctgcattcgccgtgttcacgcagacgttttcgtagacccgcatccatggtatttcctcgtagacacgccccccgtcctcgcgcaccgtctcgtatattgactcgtcgtcctcgtagggggcgtgccgttcgcgggccgaggcggcgtgggtggctttgcggcgggcgtcgtcgtcgtcgtcgtcggccgtcagatacgtggcttccatctggtcgggttctccctccggggcgggtccccacacccgtggccgatcgaggctccccagagacgcgcgccggacgaggagggggcacgtcgccgccggcggtcgcctgtcgggtcccgcgacgttacgggccgggaggcgcgggggcacctcccccatgtgcgtgtaatacgtggccggctgtgcggccgcagcggggggctcggcgaccgggtcgttcgcatccggaagcgggggccccgcgccgtccgcgcggcgcctccggaacctccgggtggacgcgggggtcgagtgtaggcgaggtcgggggaggggcgggggctcgttgtcgcgccgcgcccgctgaatcttttcccgacaggtcccaccccccgcgcgatgcccccccgggccgctggccatgtcgtccgggggaggccccgcggaccacgtcgtccggcgagacgccacgagccgcaggatggactcgtagtggagcgacggcgccccgctgcggagcagatccgcggccagggcggccccgaaccaagccttgatgctcaactccatccgggcccagctgggggcggtcatcgtggggaacaggggggcggtggtccgacagaaacgctcctggctgtccaccgcggcccgcagatactcgttgttcaggctgtcggtggcccagacgccgtacccggtgagggtcgcgttgatgatatactgggcgtggtgatggacgatcgacagaacctccaccgtggatacgacggtatccacggtcccgtacgtaccgccgctccgcttgccggtctgccacaggttggctaggcgcgtcaggtggcccaggacgtcgctgaccgccgccctgagcgccatgcactgcatggagccggttgtgccgctgggaccccggtccagatggcgcgcgaacgtttccgcgggcgcctccgggctgccgccgagcgggaggaaccggcgattggagggactcagccggtgacatacgtgcttgtctgtcgtccacagcatccaggacgcccaccggtacagcacggagacgtaggccaggagctcgttgagccgcagtgcggtgtcggtgctggggcggcttgggtccgccgggcgcataaagaacatgtactgctgaatccgatggagggcgtcgcgcaggccggccacggtggcggcgtacttggccgccacggccccgctcttgaacggggtgcgcgccagcagctttggcgccagggtgggccgcagcagcacgtgaaggctggggtcgcagtcgcccacggggtcctcggggacgtccaggccgctgggcaccaccgtctgcaggtacttccagtactgcgtgaggatggcgcggctcaactggccgccgggcagctccacctcgcccagcgcctgggtggcggccgaagcgtagtgccggatgtactcgtagtgcgggtcgctggcgagcccgtccacgatcaaactctcgggaaccgtgttgtgttgccgcgcggccaaccggacgctgcgatcggtgcaggtcagaaacgccggctgcgcgtcgtcggagcgctgccgcaaggcgcccacggccgcgctaaggagcccctccggggtggggagcagacacccgccgaagatgcgccgctcgggaacgcccgcgttgtcgccgcggatcaggttggcaggcgtcaggcaccgcgccagccgcagggagctcgcgccgcgcgtccggcgctgcatggtgacgcccgttcggtcgggacccgccggtcggagttatgccgcgtccagggccatcggggcgctttttatcgggaggagcttatgggcgtggcgggcctcccagcccggtcgcgcgcctccccgacacgtgcgcccgcagggcggcggccccctcgtctcccatcagcagtttcctaaactgggacatgatgtccaccacgcggacccgcgggcccaacacggacccgccgcttacgggggcgggggggaagggctccaggtccttgagaagaaaggcggggtctgccgtcccggacacgggggcccggggcgctgaggaggcggggcgcagatccacgtgctccgcggccgcgcggacgtccgcccagaacttggcgggggtggtgcgcgcgtacaggggctgggtcgctcggaggacgcacgcgtagcgcaggggggtgtacgtgcccacctcgggggccgtgaatcccccgtcaaacgcggccagtgtcacgcacgccaccacggtgtcggcaaagcccagcagccgctgcaggacgagcccggcggccagaatggcgcgcgtggccgccgcgtcgtcccggcgccggtgcgcgtccccgcacgcccgggcgtactttaaggtcacggtcgccagggccgtgtgcagcgcgtacaccgcagcgcccagcacggcgttgagcccgctgttggcgagcagccggcgcgctgcggtgtcgcccagcgcctcgtgctcggcccccacgaccgcggggcttcccaggggcagggcgcgaaacagctcctcccgcgccacgtccgcaaaggcggggtggtgcacgtgcgggtgcaggcgcgcccccacgaccaccgagagccactggaccgtctgctccgccatcaccgccagcacatccagcacgcgccccaggaaggcggcctcccgcgtcaaaacgcaccggacggcgtcgggattgaagcgggcgagcagggccccggtggccaggtacgtcatgcggccggcatagcgggcggccacgcgacagtcgcggtccagcagcgcgcgcaccccgggccagtacagcagggaccccagcgagctgcggaacaccgcggcgtcggggccggattggggggacactaacccccccgcgctcagtaacggcacggccgcggccccgacgggacgcaacgccgtgaggctcgcgaactgccgcctcagctcggccgccctgtcgtccaggtcagacccgcgcgcctccgcgtgaaggcgcgtcccgcacacccacccgttgatggccagccgcacgacggcatccgccaaaaagctcatcgcctgggcggggctggtttttgttcgacgatccgtcaggtcaagaatcccatcgcccgtgatataccaggccaacgcctcgccctgctgcagggtttggcggaaaaacaccgcggggttgtcgggggaggcgaagtgcatgacccccacgcgcgataacccgaacgcgctatccggacacgggtaaaacccggccggatgccccagggctagggcggagcgcacggactcgtcccacacggcaacctgaggggccagtcgatccaacgggaatgccgcccggagctccgggcccggcacgcgtccctccagaacctccaccttgggcggggaacgggccccgccgccgtcctccggcccgacggcttccgggtagtcgtcctcctcgtactgcagctcctctaggaacagcggcgacggcgccacccgcgaaccgccgacccgccccaaaatagcccgcgcgtcgacgggacccaggtatcccccctgccgggcctgcggaggaccgcggggaacctcatcatcatcgtccaggcgaccgcgcaccgactggctacgggccgcatcgggcccggggcgctgccgggacgctcggcgatgggatgtgggcggggcttccgacgcgcgccgtcgtcgggctcgcgggccttcccgtcgacggcgcacgggcggctcgtcgcccgccatctcctccagagcctctagctcgctgtcgtcatccccgcggaacaccgcacgcaggtaccccatgaaccccaccccatcgcccgctggctcgtccgccacgggcgaggcgcgggggcgggtggatgcgcgcctcctgcgccccgcgggttcgcgagccgacatggtggcgatagacgcgggttatcggatgtccgctaccccccaaaaaagaaaaagaccccacagcgcggatggaggccggggtaggtgccgccggaccccctcgcgatgggaatggacgggagcgacggggccggcgcaaaaaaacgcagtatctcccgcgaaggctacccgccgccccagcccccggccaaatgcggaaacggtcccgcgctctcgcctttatacgcgggccgccctgcgacacaatcacccgtccgtggtttcgaatctacacgacaggcccgcagacgcggctaacacacacgccggcaacccagaccccagtgggttggttgcgcggtcccgtctcctggctagttctttcccccaccaccaaataatcagacgacaaccgcaggttttgtaatgtatgtgctcgtgtttattgtggatacgaaccggtgacgggaggggaaaacccagacgggggatgcgggtccggtcgcgccccctacccaccgtactcgtcaattccaagggcatcggtaaacatctgctcaaactcgaagtcggccatatccagagcgccgtagggggcggagtcgtggggggtaaatcccggccccggggaatccccgtcccccaacatgtccagatcgaaatcgtctagcgcgtcggcatgcgccatcgccacgtcctcgccgtctaagtggagctcgtcccccaggctgacatcggtcgggggggccgtcgacagtctgcgcgtgtgtcccgcggggagaaaggacaggcgcggagccgccagccccgcctcttcgggggcgtcgtcgtccgggagatcgagcaggccctcgatggtagacccgtaattgtttttcgtacgcgcgcggctgtacgcgtgttcccgcatgaccgcctcggagggcgaggtcgtgaagctggaatacgagtccaacttcgcccgaatcaacaccataaagtacccagaggcgcgggcctgggtgccatgcagggtgggaggggtcgtcaacggcgcccctggctcctccgtagccgcgctgcgcaccagcgggaggttaaggtgctcgcgaatgtggtttagctcccgcagccggcgggcctcgattggcactccccggacggtgagcgctccgttgacgaacatgaagggctggaacagacccgccaactgacgccagctctccaggtcgcaacagaggcagtcaaacaggtcgggccgcatcatctgctcggcgtacgcggcccataggatctcgcgggtcaaaaatagatacaaatgcaaaaacagaacacgcgccagacgagcggtctctcggtagtacctgtccgcgatcgtggcgcgcagcatttctcccaggtcgcgatcgcgtccgcgcatgtgcgcctggcggtgcagctgccggacgctggcgcgcaggtaccggtacagggccgagcagaagttggccaacacggttcgatagctctcctcccgcgcccgtagctcggcgtggaagaaacgagagagcgcttcgtagtagagcccgaggccgtcgcgggtggccggaagcgtcgggaaggccacgtcgccgtgggcgcgaatgtcgatttgggcgcgttcggggacgtacgcgtccccccattccaccacatcgctgggcagcgttgataggaatttacactcccggtacaggtcggcgttggtcggtagcgccgaaaacagatcctcgttccaggtatcgagcatggtacatagcgcggggcccgcgctaaagcccaagtcgtcgaggagacggttaaagagggcggcgggggggacgggcatgggtggggagggcatgagctgggcctggctcaggcgccccgttgcgtacagcgggggggccgccggggtgtttttgggacccccggctgggcgggggggcggtggcgaagcgccgtccgcgttcatgtcggcaaacagctcgtcgaccaagaggtccattgggtggggttgatacgggaaagacgatatcgggcttttgatgcgatcgtccccgcccgcccagagagtgtgggacgcccgacggcgcgggaagagaaaaacccccaaacgcgttagaggaccggacggaccttatggggggaagtgggcagcgggaaccccgtccgttcccgaggaatgacagcccgtggtcgccaccacgcatttaagcaacccgcacgggccgccccgtacctcgtgacttccccccacattggctcctgtcacgtgaaggcgaaccgagggcggctgtccaacccaccccccgccacccagtcccggtccccgtcggattgggaaacaaaggcacgcaacgccaacaccgaatgaacccctgttggtgctttattgtctgggtacggaagttttcactcgacgggccgtctggggcgagaagcggagcgggctggggctcgaggtcgctcggtggggcgcgacgccgcagaacgccctcgagtcgccgtggccgcgtcgacgtcctgcaccacgtctggattcaccaactcgttggcgcgctgaagcaggtttttgccctcgcagaccgtcacgcggatggtggtgatgccaaggagttcgttgaggtcttcgtctgtgcgcggacgcgacatgtcccagagctggaccgccgccatccgggcatgcatggccgccaggcgcccgaccgcggcgcagaagacgcgcttgttaaagccggccacccggggggtccatggcgcgtcggggtttgggggggcggtgctaaagtgcagctttctggccagcccctgcgcgggtgtcttggatcgggttggcgccgtcgacgcgggggcgtctgggagtgcggcggattctggctgggccgatttcctgccgcgggtggtctccgccgccggggccgcgggggccttagtcgccacccgctgggttcggggggcccggggggcggtggtgggtgtgcgtccggcccctccggacccagcgggtggcggaggtgcccgcgcaggccccgggccggacaaaaccgccccggaaacgggacgccgcgtccgggggacctccgggtgttcgtcgtcttcggatgacgagcccccgtagagggcataatccgactcgtcgtactggacgaaacggacctcgcccctctggcgcgagcgtgtctgtagggcgccacggcgggaggtgtcaggcggactatcgggactcgccatacctgaagacggggtgtagtacagatcctcgtactcatcgcgcggaacctcccgcggacccgacttcacggagcggcgagaggtcatggttccacgaacacgctagggtcggatgcgcggacaattaggcctgggttcggacggcgggggtggtgcaggtgtggagaggtcgagcgataggggcggcccgggagagaagagagggtccgcaaaacccactggggatgcgtgagtggccctctgtgggcggtgggggagagtcttataggaagtgcatataaccacaacccatgggtctaaccaatccccaggggccaagaaacagacacgccccaaacggtctcggtttccgcgaggaaggggaagtcctgggacaccctccacccccacccctcaccccacacagggcgggttcaggcgtgcccggcagccagtagcctctggcagatctgacagacgtgtgcgataatacacacgcccatcgaggccatgcctacataaaagggcaccagggcccccggggcagacatttggccagtgttttgggtctcgcaccgcgcgcccccgatcccatcgcgcccgccctcctcgccgggcggctccccgtgcgggcccgcgtctcccgccgctaaggcgacgagcaagacaaacaacaggcccgcccgacagacccttctgggggggcccatcgtccctaacaggaagatgagtcagtggggatccggggcgatccttgtccagccggacagcttgggtcgggggtacgatggcgactggcacacggccgtcgctactcgcgggggcggagtcgtgcaactgaacctggtcaacaggcgcgcggtggcttttatgccgaaggttagcggggactccggatgggccgtcgggcgcgtctctctggacctgcgaatggctatgccggctgacttttgcgcgattattcacgcccccgcgctagccagccccgggcaccacgtaatactgggtcttatcgactcggggtaccgcggaaccgttatggccgtggtcgtagcgcctaaaaggacgcgggaatttgcccccgggaccctgtgggtcgacgtgacgttcctggacatcctggcgacccccccggccctcaccgagccgatttccctgcggcagttcccgcaactggcgcccccccctccaaccggggccgggatacgcgaagatccttggttggagggggcgctcggggccccaagcgtgactacggccctaccggcgcgacgccgagggcggtccctcgtctatgccggcgagctgacgccggttcagacggaacacggggacggcgtacgagaagccatcgccttccttccaaaacgcgaggaggatgccggtttcgacattgtcgtccgtcgcccggtcaccgtcccggcaaacggcaccacggtcgtgcagccatccctccgcatgctccacgcggacgccgggcccgcggcctgctatgtgttggggcggtcgtcgctcaacgcccgcggcctcctggtcgttcctacgcgctggctccccgggcacgtatgtgcgtttgttgtttacaaccttacgggggttcctgtgaccctcgaggccggcgccaaggtcgcccagctcctggttgcgggggcggacgctcttccttggatccccccggacaactttcacgggaccaaagcgcttcgaaactaccccaggggtgttccggactcaaccgccgaacccaggaacccgccgctcctggtgtttacgaacgagtttgacgcggaggcccccccgagcgagcgcgggaccgggggttttggctctaccggtatttagcccacagctttgggttcgttccgggcaataaaaaacgtttgtatcgcatctttcctgtgtgtagttgtttatgttggatgcctgtgggtctatcacacccgcccctccatcccacaaacacaaaacacacgggttggatgaaaacacgcatttattgacccaaaacacacggagctgctcgagatgggccagggcgaggtgcggttggggaggctgtaggtctgggaacggacacgcggggacacgattccggtttggggtccgggagggcgtcgccgtttcgggcggcaggcgccagcgtaacctccgggggcggcgtgtgggggtgccccaaggagggcgcctcggtcaccccaatcccccccgaccgggttcccccggcaaccccgaaggcggagaggccaagggcccgttcggcgatggccacatcctccatgaccacgtcactctcggccatgctccgaatagcctgggagacgagcacatccgcggacttgtcagccgcccccacggacatgtacatctgcaggatggtggccatacacgtgtccgccaggcgccgcatcttgtcctgatgggccgccacggccccgtcgatcgtgggggcctcgagcccggggtggtggcgcgccagtcgttctaggttcaccatgcaggcgtggtacgtgcgggccaaggcgcgggccttcacgaggcgtcgggtgtcgtccagggaccccagggcgtcatcgagcgtgatgggggcgggaagtagcgcgttaacgaccgccagggcctcctgcagccgcggctccgcctccgagggcggaacggccgcgcggatcatctcatattgttcctcggggcgcgctccccagccacatatagccccgagaagagaagccatcgcgggcgggtactggcccttgggcgcgcggacgcaatggggcaggaagacgggaaccgcggggagaggcgggcggccgggactcccgtggaggtgaccgcgctttatgcgaccgacgggtgcgttattacctcttcgatcgccctcctcacaaactctctactgggggccgagccggtttatatattcagctacgacgcatacacgcacgatggccgtgctgacgggcccacggagcaagacaggttcgaagagagtcgggcgctctaccaagcgtcgggcgggctaaatggcgactccttccgagtaaccttttgtttattggggacggaagtgggtgggacccaccaggcccgcgggcgaacccgacccatgttcgtctgtcgcttcgagcgagcggacgacgtcgccgcgctacaggacgccctggcgcacgggaccccgctacaaccggaccacatcgccgccaccctggacgcggaggccacgttcgcgctgcatgcgaacatgatcctggctctcaccgtggccatcaacaacgccagcccccgcaccggacgcgacgccgccgcggcgcagtatgatcagggcgcgtccctacgctcgctcgtggggcgcacgtccctgggacaacgcggccttaccacgctatacgtccaccacgaggcgcgcgtgcttgccgcgtaccgcagggcgtattatggaagcgcgcagagtcccttctggtttcttagcaaattcgggccggacgaaaaaagcctggtgctcaccactcggtactacctgcttcaggcccagcgtctggggggcgcgggggccacgtacgacctgcaggccatcaaggacatctgcgccacctacgcgattccccacgccccccgccccgacaccgtcagcgctgcgtccctgacctcgtttgccgccatcacgcggttctgttgcacgagccagtacgcccgcggggccgcggcggccgggtttccgctttacgtggagcgccgtattgcggccgacgtccgcgagaccagtgcgctggagaagttcataacccacgatcgcagttgcctgcgcgtgtccgaccgtgaattcattacgtacatctacctggcccattttgagtgtttcagccccccgcgcctagccacgcatcttcgggccgtgacgacccacgaccccaaccccgcggccagcacggagcagccctcgcccctgggcagggaggccgtggaacaatttttttgtcacgtgcgcgcccaactgaatatcggggagtacgtcaaacacaacgtgaccccccgggagaccgtcctggatggcgatacggccaaggcctacctgcgcgctcgcacgtacgcgcccggggccctgacgcccgcccccgcgtattgcggggccgtggactccgccaccaaaatgatggggcgtttggcggacgccgaaaagctcctggtcccccgcgggtggcccgcgtttgcgcccgccagtcccggggaggacacggcgggcggcacgccgcccccacagacctgcggaattgtcaagcgcctcctgagactggccgccacggaacagcagggcaccacacccccggcgatcgcggcgcttatccgtaatgcggcggtgcagactcccctgcccgtctaccggatatccatggtccccacgggacaggcatttgccgcgctggcctgggacgactgggcccgcataacgcgggacgctcgcctggccgaagcggtcgtgtccgccgaagcggcggcgcaccccgaccacggcgcgctgggcaggcggctcacggatcgcatccgcgcccagggccccgtgatgccccctggcggcctggatgccggggggcagatgtacgtgaatcgcaacgagatattcaacggcgcgctggcaatcacaaacatcatcctggatctcgacatcgccctgaaggagcccgtcccctttcgccggctccacgaggccctgggccactttaggcgcggggctctggctgcggttcagctcctgtttcccgcggcccgcgtggaccccgacgcatatccctgttattttttcaaaagcgcatgtcggcccggcccggcgtccgtgggttccggcagcggactcggcaacgacgacgacggggactggtttccctgctacgacgacgccggtgatgaggagtgggcggaggacccgggcgccatggacacatcccacgatcccccggacgacgaggttgcctactttgacctgtgccacgaagtcggccccacggcggaacctcgcgaaacggattcgcccgtgtgttcctgcaccgacaagatcggactgcgggtgtgcatgcccgtccccgccccgtacgtcgtccacggttctctaacgatgcggggggtggcacgggtcatccagcaggcggtgctgttggaccgagattttgtggaggccatcgggagctacgtaaaaaacttcctgttgatcgatacgggagtgtacgcccacggccacagcctgcgcttgccgtattttgccaaaatcgcccccgacgggcctgcgtgcggaaggctgctgccagtgtttgtgatcccccccgcctgcaaagacgttccggcgtttgtcgccgcgcacgccgacccgcggcgcttccattttcacgccccgcccacctatctcgcttccccccgggagatccgtgtcctgcacagcctgggtggggactatgtgagcttctttgaaaggaaggcgtcccgcaacgcgctggaacactttgggcgacgcgagaccctgacggaggtcctgggtcggtacaacgtacagccggatgcgggagggaccgtcgaggggttcgcatcggaactgctggggcggatagtcgcgtgcatcgaaacccactttcccgaacacgccggcgaatatcaggccgtatccgtccggcgggccgtcagtaaggacgactgggtcctcctacagctagtccccgttcgcggtaccctgcagcaaagcctgtcgtgtctgcgctttaagcacggccgggcgagtcgcgccacggcgcggacattcgtcgcgctgagcgtcggggccaacaaccgcctgtgcgtgtccttgtgtcagcagtgctttgccgccaaatgcgacagcaaccgcctgcacacgctgtttaccattgacgccggtacgccatgctcgccgtccgttccctgcagcacctctcaaccgtcgtcttgataacggcgtacggcctcgtgctcgtgtggtacaccgtcttcggtgccagtccgctgcaccgatgtatttacgcggtacgccccaccggcaccaacaacgacaccgccctcgtgtggatgaaaatgaaccagaccctattgtttctgggggccccgacgcacccccccaacgggggctggcgcaaccacgcccatatctgctacgccaatcttatcgcgggtagggtcgtgcccttccaggtcccacccgacgccatgaatcgtcggatcatgaacgtccacgaggcagttaactgtctggagaccctatggtacacacgggtgcgtctggtggtcgtagggtggttcctgtatctggcgttcgtcgccctccaccaacgccgatgtatgtttggtgtcgtgagtcccgcccacaagatggtggccccggccacctacctcttgaactacgcaggccgcatcgtatcgagcgtgttcctgcagtacccctacacgaaaattacccgcctgctctgcgagctgtcggtccagcggcaaaacctggttcagttgtttgagacggacccggtcaccttcttgtaccaccgccccgccatcggggtcatcgtaggctgcgagttgatgctacgctttgtggccgtgggtctcatcgtcggcaccgctttcatatcccggggggcatgtgcgatcacataccccctgtttctgaccatcaccacctggtgttttgtctccaccatcggcctgacagagctgtattgtattctgcggcggggcccggcccccaagaacgcagacaaggccgccgccccggggcgatccaaggggctgtctggcgtctgcgggcgctgttgttccatcatcctctcgggcatcgcagtgcgattgtgttatatcgccgtggtggccggggtggtgctcgtggcgcttcactacgagcaggagatccagaggcgcctgtttgatgtatgacgtcacatccaggccggcggaaaccggaacggcatatgcaaattggaaactgtcctgtcttggggcccacccacccgacgcgtcatatgcaaatgaaaatcggtcccccgaggccacgtgtagcctggatcccaacgaccccgcccatgggtcccaattggccgtcccgttaccaagaccaacccagccagcgtatccacccccgcccgggtccccgcggaagcggaacggtgtatgtgatatgctaattaaatacatgccacgtacttatggtgtctgattggtccttgtctgtgccggaggtggggcggggcccccgcccggggggcggaacgaggaggggtttgggagagccggccccggcaccacgggtataaggacatccaccacccggccggtggtggtgtgcagccgtgttccaaccacggtcacgcttctgtgcctctccccgattcgggcccggtcgctcgctaccggtgcaccaccaccagaggccatatccgacaccccagccccgacggcagccgacagcccggtcatggcgactgacattgatatgctaattgacctcggcctggacctctccgacagcgatctggacgaggacccccccgagccggcggagagccgccgcgacgacctggcatcggacagcagcggggagtgttcctcgtcggacgaggacatggaagacccccacggagaggacggaccggagccgatactcgacgccgctcgcccggcggtccgcccgtctcgtccagaagaccccggcgtacccagcacccagacgcctcgtccgacggagcggcagggccccaacgatcctcaaccagcgccccacagtgtgtggtcgcgcctcggggcccggcgaccgtcttgctcccccgagcagcacgggggcaaggtggcccgcctccaacccccaccgaccaaagcccagcctgcccgcggcggacgccgtgggcgtcgcaggggtcggggtcgcggtggtcccggggccgccgatggtttgtcggacccccgccggcgtgcccccagaaccaatcgcaacccggggggaccccgccccggggcggggtggacggacggccccggcgccccccatggcgaggcgtggcgcggaagtgagcagcccgacccacccggaggcccgcggacacggggcgtgcgccaagcaccccccccgctaatgacgctggcgattgcccccccgcccgcggacccccgcgccccggccccggagcgaaaggcgcccgccgccgacaccatcgacgccaccacgcggttggtcctgcgctccatctccgagcgcgcggcggtcgaccgcatcagcgagagctttggccgcagcgcacaggtcatgcacgacccctttggggggcagccgtttcccgccgcgaatagcccctgggccccggtgttggcgggccaaggagggccctttgacgccgagaccagacgggtctcctgggaaaccttggtcgcccacggcccgagcctctatcgcacttttgccggcaatcctcgggccgcatcgaccgccaaggccatgcgcgactgcgtgctgcgccaagaaaatttcatcgaggcgctggcctccgccgacgagacgctggcgtggtgcaagatgtgcatccaccacaacctgccgctgcgcccccaggaccccattatcgggacggccgcggctgtgctggataacctcgccacgcgcctgcggccctttctccagtgctacctgaaggcgcgaggcctgtgcggcctggacgaactgtgttcgcggcggcgtctggcggacattaaggacattgcatccttcgtgtttgtcattctggccaggctcgccaaccgcgtcgagcgtggcgtcgcggagatcgactacgcgacccttggtgtcggggtcggagagaagatgcatttctacctccccggggcctgcatggcgggcctgatcgaaatcctagacacgcaccgccaggagtgttcgagtcgtgtctgcgagttgacggccagtcacatcgtcgcccccccgtacgtgcacggcaaatatttttattgcaactccctgttttaggtacaataaaaacaaaacatttcaaacaaatcgccccacgtgttgtccttctttgctcatggccggcggggcgtgggtcacggcagatggcgggggtgggcccggcgtacggcctgggtgggcggagggaactaacccaacgtataaatccgtccccgctccaaggccggtgtcatagtgcccttaggagcttcccgcccgggcgcatccccccttttgcactatgacagcgacccccctcaccaacctgttcttacgggccccggacataacccacgttgcccccccttactgcctcaacgccacctggcaggccgaaacggccatgcacaccagcaaaactgactccgcttgcgtggccgtgtggagttacctggtccgcgcctcctgtgagaccagcggcacaatccactgctttttctttgtggtatacaaggacacccaccatacccctccgctgattaccgagctccgcaactttgcggacctggttaaccacccgccggtcctacgcgaactggaggataagcgcggggtgcggctgcggtgtgcgcggccgtttagcgtcgggacgattaaggacgtctctgggtccggcgcgtcctcggcgggagagtacacgataaacgggatcgtgtaccactgccactgtcggtatccgttctcaaaaacatgctggatgggggcctccgcggccctacagcacctgcgctccatcagctccagcggcatggccgcccgcgcggcagagcatcgacgcgtcaagattaaaattaaggcgtgatttccaaccccccatgaatgtgtgtaaccccccccaaaaaaataaagagccgtaacccaaccaaaccaggcgtggtgtgagtttgtggacccaaagccctcagagacaacgcgacaggccagtatggaccgtgagacttttatttattaactcacaggggcgcttaccgccacaggaataccagaataatgaccaccacaatcgcgaccaccccaaatacagcatggcgccccaccacgccacaacagccctgtcgccggtatggggcatgatcagacgagccgcgagccgcgcgttgggccctgtacagctcgcgcgaattgaccctaggaggccgccacgcgcccgagttttgcgttcgtcgctggtcgtcgggcaccaaagccccggacggctgttcggtcgaacgaacggccacgacagtggcataggttggggggtggtccgacatagcctcggcgtacgtcgggaggcccgacaagaggtcccttgtgatgtcgggtggggccacaagcctggtttccggaagaaacaggggggttgccaataacccgccagggccaaaactccggccctggcgcacgtcgttcggcgcggcgccgggcgcgccgagcggctcgctgggcggcttggcgtgagcggccccgctccgacgcctcgccctctccggaggaggttggtggaattggcacggacgacaggggcccagcagagtacggtggaggtgggtccgtgggggtgtccagatcaataacgacaaacggcccctcgttcctaccagacaagctatcgtaggggggcgggggatcaacaaacgcgttccccgcgctccatagacccgcgtcgggttgcgccgcctccgaagccatggatgcgccccaaagccacgactcccgcgcgctaggtccttggggtaagggaaaaggccctactccccatccaagccagccaagttaacgggctacgccttcggggatgggactggcaccccggcggattttgttgggctggcatgcgtcgcccaaccgagggccgcgtccacgggacgcgccttttataaccccgggggtcattcccaacgatcacatgcaatctaactggctcccctctcctcccctctcccctctcccctctcccctctcccctctcccctctcccctcttaggttggggggtggtccgacatagcctcggcgtacgtcgggaggcccgacaagaggtcccttgtgatgtcgggtggggccacaagcctggtttccggaagaaacaggggggttgccaagcggcccggcccgcgctcccccccccccggggccgtgtccttgctttccccccgtctccccccccctcctcctccttctcctcctcctcgtttttccaaaccccgcccacccggcccggcccggcccggccaccgccgcccacccacccaccgcgggagacccagccccggtcccccgttccccgggggccgttatctccagcgccccgtccggcgcgccgccccccgccgctaaaccccatcccgcccccgggaccccacatataagcccccagccacacgcaagaacagacacgcagaacggctgtgtttatttaaataaaccgatgtcggaataaacaaacacaaacacccgcgacggggggacggagggaggggggtgacgggggacgggaacagacacaaaaaacaaccacaaaaaaacagccacccccgacaccccccaccccagtctcctcgccttttcccacccaccccacgcccccactgagcccggtcgatcgacgagcacccccgcccccgcccctgccccggcgacccccggcccgcacgatcccgacaacaataacaaccccaacggaaagcggcggggtgttgggggaggcgaggaacaaccgaggggaacgggggatggaaggacgggaagtggaagtcctgatacccatcctacacccccctgccttccaccctccggccccccgcgagtccacccgccggccggctaccgagaccgaacacggcggccgccgcagccgccgcagccgccgccgacaccgcagagccggcgcgcgcacacacaagcggcagaggcagaaaggccccgagtcattgtttatgtggccgcgggccagcagacggcccgcgacacccccccgcccgtgtgggtatccggccccccgccccgcgccggtccattaagggcgcgcgtgcccgcgagatatcaatccgttaagtgctctgcagacaggggcaccgcgcccggaaatccattaggccgcagacgaggaaaataaaattacatcacctacccacgtggtgctgtggcctgtttttgctgcgtcatctgagcctttataaaagcgggggcgcggccgtgccgatcgcgggtggtgcgaaagactttccgggcgcgtccgggtgccgcggctctccgggcccccctgcagccggggcggccaaggggcgtcggcgacatcctccccctaagcgccggccggccgctggtctgttttttgttttccccgtttcgggggtggggggggttacggtttctgttttttaaacccgtctggggtgtttttcgttccgtcgccgggatgtttcgttcgttcggcccctcacggggcgaaggccgcgtacggcccgggacgaggggcccccgaccgcggcggtccgggccccgtccgggcccgctcgccggcacgcgacgcgaaaaaggccccccggaggcttttccgggttcccggcccggggcctgagataaacaatcggggttaccgccaacggccggcccccgtggcggcccggcccggggccccggcggacccaaggggccccggcccggggccccacaacggcccggcgcatgcgctgtgttttttttttcctcggtgttctgccgggctccgtcgcctttcctgttctcgcttcttccccccccccttcttcacccccagtaccctcctccctcccttcctcccccgttatcccactcgtcgagggcgccccggtgtcgttcaacaaagacgccgcgtttccaggtaggttagacacctgcttctccccaatagagggggggggacccaaacgacagggggcgccccagaggctaaggtcggccacgccactcgcgggtgggctcgtgttacagcacaccagcccgttcttttccccccctcccacccttagtcagactctgttacttacccgtccgaccaccaactgcccccttatctaagggccggctggaagaccgccagggggtcggccggtgtcgctgtaaccccccacgccaatgacccacgtactccaagaaggcatgtgtcccaccccgcctgtgtttttgtgcctggctctctatgcttgggtcttactgcctggggggggggatgcgggggagggggggtgtggaaggaaatgcacggcgcgtgtgtaccccccccccaaagttgttcctaaagcgaggatatggaggagtggcgggtgccgggggacgggggtgatctctggcacgcggggggggaagggtcgggggagggggggatggggtaccggcccacctggccgacgcgggtgcgcgtgcctttgcacaccaaccccacgtcccccggcggtctctaagaagcaccgccccccctccttcataccaccgagcatgcctgggtgtgggttggtaaccaacacgcccatcccctcgtctcctgtgattctctggctgcaccgcattcttgttttctaactatgttcctgtttctgtctcccccccacccctccgccccaccccccaacacccacgtctgtggtgtggccgacccccttttgggcgccccgtcccgccacccctcccgtcctttgttgccctatagtgtagttaaccccccccccgccctttgtggcggccagaggccaggtcagtccgggcgggcaggcgctcgcggaaacttaacacccacacccagcccactgtggttctggctccatgccagtggcaggatgctttcggggatcggtggtcaggcagcccgggccgcggctctgtggttaacaccagagcctgcccaacatggcacccccactcccacgcacccccactcccacgcacccccactcccacgcacccccactcccacgcacccccactcccacgcacccccactcccacgcacccccactcccacgcacccccactcccacgcacccccactcccacgcacccccactcccacgcacccccactcccacgcacccccactcccacgcacccccactcccacgcacccccaagatccatccaacacagacagggaaaagatacaaaagtaaacctttatttcccaatagacagcaaaaatcccctgagttttttattagggccaacactaaagacccgctggtgtgtggtgcccgtgtctttcactttcccctccccgacacggattggctggtgtagtgggcgcggccagagaccacccagcacccgacccccctccccacaaacacggggggcgtcccttattgttttccctcgtcccgggtcgacgccccctgctccccggaccacgggtgccgagaccgcaggctgcggaagtccagggcgcccactagggtgccctggtcgaacagcatgttccccacgggggtcatccagaggctgttccactccgacgcgggggccgtcgggtactcggggggcatcacgtggttacccgcggtctcggggagcagggtgcggcggctccagccggggaccgcggcccgcagccgggtcgccatgtttcccgtctggtccaccaggaccacgtacgccccgatgttccccgtctccatgtccaggatgggcaggcagtcccccgtgatagtcttgttcacgtaaggcgacagggcgaccacgctagagacccccgagatgggcaggtagcgcgtgaggccgcccgcggggacggccccggaagtctccgcgtggcgcgtcttccgggcacacttcctcggcccccgcggcccagaagcagcgcgggggccgagggaggtttcctcttgtctccctcccagggcaccgacggccccgcccgaggaggcggaagcggaggaggacgcggccccggcggcggaagaggcggcccccgcgggggtcggggccgaggaggaagaggcagaggaggaagaggcggaggccgccgaggacgtcaggggggtcccgggcccaccctggccgcgcccccccggccctgagtcggagggggggtgcgtcgccgccctcttggcccctgccggcgcgagggggggacgcgtggactggggggaggggttttcctggcccgacccgcgcctcttcctcggacgcaccgccgcctcctgctcgacagagacggcggaggggagcggggcggcgccggagggggtgcggccgcgggagggcccgtgcccaccctccacgcccggcccccccgagccgcgcgccaccgtcgcacgcgcccggcacagactctgttcttggttcgcggcctgagccagggacgagtgcgactggggcacacggcgcgcgtccgcggggcgggcggccggctccgccccgggggccggggcgcgggggccgggccccggaggcggcgctcgcacgcacggggccacggccgcgcgggggcgcgcgggtcccgacgcggccgaggacgcggggggcccggggcggggggcggagcctggcatgggcgccgcggggggcctgtggggagaggccgggggggagtcgctgatcactatggggtctctgttgtttgcaaggggggcgggtctgttgacaagggggcccgtccggcccctcggccgccccgcctccgcttcaacaaccccaaccccaaccccaacccccccggaggggccagacgccccccgcggcgccgcggctcgcgactggcgggagccgccgccgccgctgctgttggtggtggtgttggtgttactgctgccgtgtggcccgatgggcgccgaggggggcgctgtccgagccgcggccggctggggggctgcgttagacgccccgcccgtcacggggggcgcggcggtgcctctgcgtgggggggcgcggggcgtccggcggggggcgggcgggacgtagtctgctgcaagagacaacggggggcgcgatcaggttacgccccctccccggcccgccctttcctcgcccgcccgcccattcctccctcctcctcctcccccagggtccttgccgccccccgcctcaccgtcgtccaggtcgtcgtcatcctcgtccgtggtgggctccgggtgggtgggcgacagggccctcaccgtgtgcccccccagggtcaggtaccgcggggcgaaccgctgattgcccgtccagataaagtccacggccgtgcccgccctgacggcctcctcggcctccatgcgggtctgggggtcgttcacgatcgggatggtgctgaacgacccgctgggcgtcacgcccactatcaggtacaccagcttggcgttgcacagcgggcaggtgttgcgcaattgcatccaggttttcatgcacgggatgcagaagcggtgcatgcacgggaaggtgtcgcagcgcaggtggggcgcgatctcatccgtgcacacggcgcacacgtcgccctcgtcgctccccccgtcctctcgagggggggcgcccccgcaactgccggggtcttcctcgcggggggggctcccccccgagaccgcccccccatccacgccctgcggccccagcagccccgtctcgaacagttccgtgtccgtgctgtccgcctcggaggcggagtcgtcgtcatggtggtcggcgtccccccgcccccccacttcggtctccgcctcagagtcgctgctgtccggcaggtctcggtcgcagggaaacacccagacatccggggcgggctaaggggaaaaaaggggggcgggtaagaatggggggggatttcccgcgtcaatcagcgcccacgagttccccctctccccccccgcctcacaaagtcctgcccccctgctggcctcggaagaggggggagaaaggggtctgcaaccaaaggtggtctgggtccgtcctttggatcccgacccctcttcttccctcttctcccgccctccagacgcaccggagtcgggggtcccacggcgtcccccaaatatggcgggcggctcctccccacccccctagatgcgtgtgagtaaggggggcctgcgtatgagtcagtggggaccacgcccccaacacggcgaccccggtccctgtgtgtttgttgtgggggcgtgtctctgtgtatgagtcagggggtcccacggcgaccccgggccctgcgtctgagtcaaaggggccatgtgtatgtgttgggggtctgtatatataaagtcagggggtcacatggcgacccccaacagggcgaccccggtccctgtatatatagggtcagggggttccgcgccccctaacatggcgcccccggtccctgtatatatagtgtcacggggttccacgccccctaacatggcgccccaacatggcgcccggctcccgtgtatgagtgggggtcccccaacatgggggccggttccagggtaagggtcgggggtcccccaacatggcgccccccaatatggcgccccagacatggcgcccggcccctcacctcgcgctgggggcggccctcaggccggcgggtactcgctccggggcggggctccatgggggtcgtatgcggctggagggtcgcggacggagggtccctgggggtcgcaacgtaggcggggcttctgtggtgatgcggagagggggcggcccgagtctgcctggctgctgcgtctcgctccgagtgccgaggtgcaaatgcgaccagaccgtcgggccagggctaacttataccccacgcctttcccctccccaaaggggcggcagtgacgattcccccaatggccgcgcgtcccaggggaggcaggcccaccgcggggcggccccgtccccggggaccaacccggcgcccccaaagaatatcattagcatgcacggcccggcccccgatttgggggaccaacccggtgtcccccaaagaaccccattagcatgcccctcccgccgacgcaacaggggcttggcctgcgtcggtgccccggggcttcccgccttcccgaagaaactcattaccatacccggaaccccaggggaccaatgcgggttcattgagcgacccgcgggccaatgcgcgaggggccgtgtgttccgccaaaaaagcaattagcataacccggaaccccaggggagtggttacgcgcggcgcgggaggcggggaataccggggttgcccattaagggccgcgggaattgccggaagcgggaagggcggccggggccgcccattaatgagtttctaattaccataccgggaagcggaacaaggcctcttgcaagtttttaattaccataccgggaagtgggcggcccggcccattgggcggtaactcccgcccaatgggccgggccccgaagactcggcggacgctggttggccgggccccgccgcgctggcggccgccgattggccagtcccgcccccgaggcgggcccgccttgggggcggaccggctcccagcgtatatatgcgcggctcctgccatcgtctctccggagagcggcttggtgcggagctcccgggagctccgcggaagacccaggcgcctcgggtgtaacgttagaccgagttcgccgggccggctccgcgggccagggcccgggcacgggcctcgggccccaggcacggcccgatgaccgcctcggcctccgccacccggcgccggaaccgagcccggtcggcccgctcgcgggcccacgagccgcggcgcgccaggcgggcggccgaggcccagaccaccaggtggcgcacccggacgtggggcgagaagcgcacccgcgcgggggtcgcgggggtcgcgggggtcgcgggggtcgcgggggtcgcgggggtcgcgggggtcgcgggggtcgcggggggctccggcgccccctccccgcccgcgcgtcgcaggcgcaggcgcgccaggtgctccgcggtgacgcgcaggcggagggcgaggcgcggcggaaggcggaaggggcgcgagggggggtgggaggggtcagccccgccccccgggcccacgccgggcggtggggaccggggccggggggcggcggcggtgggccgggcctctggcgccggctcgggcggggggctgtccggccagtcgtcgtcatcgtcgtcgtcggacgcggactcgggaacgtggagccactggcgcagcagcagcgaacaagaaggcgggggcccaccggcggggggcggcggcggggcggccgcgggcgcgctcctgaccgcgggttccgagttgggcgtggaggttacctgggactgtgcggttgggacggcgcccgtgggcccgggcggccgggggcggcgggggccgcgatggcggcggcggcgggccatggagacagagagcgtgccggggtggtagagtttgacaggcaagcatgtgcgtgcagaggcgagtagtgcttgcctgtctaactcgctagtctcggccgcggggggcccgggctgcccgccgccgcgctttaaagggccgcgcgcgacccccggggggtgtgtttcgggggggcccgtttttggggtctggccgctcctcccccgctcctccccgtctgtgggtggggctcctcccccgctcctcccccgctcctcccccgctcctccccgtctgtgggtggggctcctcccccgctcccgcggccccgccccccacgcccgccgcgcgcgcgcacgccgcccggaccgccgcccgccttttttgcgcgccgccccgcgcgcggggggcccgggctgccacaggtgtaacaacaccaacagaacaccaacagcacggcgcaccggcgactccggttcctcatccacacgtcacgtcatccaacacacctgcccaacaacacaactcacagcgacaactcaccgcgcaacaactcctgttcctcatccacacgtcaccgcgcaccccccgctcctccagacgtcccccagcgcaacacgccgctcctgtcacacaccacagccccagccctccccagccccagccctccccagccccagccctccccagccccagccctccccagccccagccctccccagccccagccctccccagccccagccctccccagccccagccctccccagccccagccctccccagccccagccctccccagccccagccctccccagccccagccctccccagccgcgtcccgcgctccctcgggggggttcgggcatctctacctcagtgccgccaatctcaggtcagagatccaaaccctccgggggcgcccgcgcaccaccaccgcccctcgccccctcccgcccctcgccccctcccgcccctcgccccctcccgcccctcgccccctcccgcccctcgccccctcccgcccctcgccccctcccgcccctcgccccctcccgcccctcgccccctcccgcccctcgaataaacaacgctactgcaaaacttaatcaggtcgttgccgtttattgcgtcttcgggtttcacaagcgccccgccccgtcccggcccgttacagcaccccgtccccctcgaacgcgccgccgtcgtcttcgtcccaggcgccttcccagtccacaacgtcccgtcgcgggggcgtggccaagcccgcctccgcccccagcacctccacggcccccgccgccgccagcacggtgccgctgcggcccgtggccgaggcccagcgaatcccgggcggcgccggcggcagggcccccgggccgtcgtcgtcgccgcgcagcaccagcgggggggcgtcgtcgtcgggctccagcagggcgcgggcgcaaaagtccctccgcggcccgcgccaccgggccgggccggcgcgcaccgcctcgcgccccagcgccacgtacacgggccgcagcggcgcgcccaggccccagcgcgcgcaggcgcggtgcgagtgggcctcctcctcgcagaagtccggcgcgccgggcgccatggcgtcggtggtccccgaggccgccgcccggccgtccagcgccggcagcacggcccggcggtactcgcgcggggacatgggcaccggcgtgtccgggccgaagcgcgtgcgcacgcggtagcgcacgttgccgccgcggcacaggcgcagcggcggcgcgtcggggtacaggcgcgcgtgcgcggcctccacgcgcgcgaagacccccgggccgaacacgcggcccgaggccagcaccgtgcggcgcaggtcgcgcgccgccggccagcgcacggcgcactgcacggcgggcagcaggtcgcacgccaggtaggcgtgctgccgcgacaccgcgggcccgtcggcgggccagtcgcaggcgcgcacggtgttgaccacgatgagccgccggtcgccggcgctggcgagcagccccagaaactccacggccccggcgaaggccaggtcccgcgtggacagcagcagcacgccctgcgcgcccagcgccgacacgtcgggggcgccggtccagttgcccgcccaggcggccgtgtccggcccgcacagccggttggccagggccgccagcaggcaggacagcccgccgcgctcggcggaccactccggcggcccccccgaggccccgccgccggccaggtcctcgcccggcagcggcgagtacagcaccaccacgcgcacgtcctcggggtcggggatctggcgcatccaggccgccatgcggcgcagcgggcccgaggcgcgcagggggccaaagaggcggcccccggcggccccgtgggggtgggggttctcgtcgtcgtcgccgccgccgcacgcggcctgggcggcgggggcgggcccggcgcaccgcgcggcgatcgaggccagggcccgcgggtcaaacatgagggccggtcgccaggggacggggaacagcgggtggtccgtgagctcggccacggcgcgcggggagcagtaggcctccagggcggcggccgcgggcgccgccgtgtggctgggccccgggggctgccgccgccagccgcccagggggtcggggccctcggcgggccggcgcgacagcgccacggggcgcgggcgggcctgcgccgcggcggcccggggcgccgcgggctgggcgggggcgggctcgggccccgggggcgtggaggggggcgcgggcgcggggaggggggcgcgggcgtccgagccgggggcgtccgcgccgctcttcttcgtcttcgggggtcgcgggccgccgcctccgggcggccgggccgggccgggactcttgcgcttgcgcccctcccgcggcgcggcggaggcggcggccgcgacccccgaagacgaagaagagcggcgcggacccgccgccagcagggggcgcaggctctggttctcaaacagcaggtccgcggcggcggcggccgcggagctcggcaggcgcgggtcccgcggcagcgcgggacccagggccccggcgaccaggctcacggcgcgcacggcggccacggcggcctcgctgccgccggccacgcgcaggtccccgcgcaggcgcatgagcaccagcgcgtcgcgcacgaaccgcagctcgcgcagccacgcgcgcaggcggggcgcgtcggcgtgcggcggcggcggggaagcggggcccgcgggtccctccggccgcggggggctggcgggccgggccccggccagccccgggacggccgccaggtcgccgtcgaagccctcggccagcgcctccaggatcccgcggcaggcggccaggcactccacggccacgcggccggcctgggcgcggcgcccggcgtcgtcgtcggcgtcggcgtggcgggcggcgtcggggtcgtcgccccccgcgggggaggcgggcgcggcggacagccgccccagggcggcgaggatccccgcggcgccgtacccggcgggcaccgcgcgctcgcccggtgcggcggcggcggcgacgacggcggcggcgaccccctcgtcatctgcgccggcgccggggctccccgcggcccccgtcagcgccgcgttctcgcgcgccaacaggggcgcgtaggcgcggcgcaggctggtcagcaggaagcccttctgcgcgcggtcgtatcggcggctcatggccacggcggccgccgcgtgcgccaggccccagccgaagcggccggccgccatggcgtagcccaggtggggcacggcccgcgccacgctgccggtgatgaaggagctgctgttgcgcgcggcgcccgagatccggaagcaggcctggtccagcgccacgtccccggggaccacgcgcgggttctggagccaccccatggcctccgcgtccggggtgtacagcagccgcgtgatcagggcgtactgctgcgcggcgtcgcccagctcgggcgcccacacggccgccggggcgcccgaggcctcgaaccggcgtcgcgcctcctccgcctcgggcgccccccagaggcccgggcggctgtcgcccaggccgccgtacagcacccgccccgggggcgggggcccggcgccgggccacggctccccgctgacgtacccgtcgcgatagcgcgcgtagaaggcgccggaggccgcgtcggcgtccagctcgacccgccggggctgcccggccgtgaagcggcccgtggcgtcgcggccggccaccgccgcgcgggcccggcggcgctcgatgcggcccgcggaggccgcgggggtcctcgccgccgcccggggcttgggcgcggcctcggagagggggggtggcccgggcgggggcggcgtccgcccgggggcttccggcgccgcgctcgacggaccccgcccgacggcccgcgcctcgcgtgcgtggtcggccgcgtcgttgccgtcgtcgtcctcgtcctcgtcggacgacgaggacgaagaggatgcggacgacgaggacgaggacccggagtccgacgaggtcgatgacgccgatggccgccgccggccgtgacgacgtctctgcggcggctgggccggcgggcgcggcgacaggcggtccgtggggtccggatacgcgccgcgtagcggggcctcccgtgcgcggccccgggccggggcccggtcgccggcggcgtcggctgcgtcgtcgtactcgtccccgtcatcgtcgtcggctcgaaaggcgggggtccggggcggcgaggccgcggggtcgggcgtcgggatcgtccggacggcctcctctaccatggaggccagcagggccagctgtcgcggcgagacggcgtccccggcgtcctcgccggcgtcggtgcccgccgcgggggccctcccgtcccgccgggcgtcgtcgaggtcgtgggggtggtcggggtcgtggtcggggtcgtccccgccctcctccgtctccgcgccccacccgagggccccccgctcgtcgcggtctgggctcggggtgggcggcggcccgtcggtggggcccggggagccggggcgctgcttgttctccgacgccatcgccgatgcggggcgatcctccggggatacgactgcgacggcggacgtagcacggtaggtcacctacggactctcgatggggagggggcgagacccacggaccccgacgacccccgccgtcgacgcggaactagcgcggaccggtcgatgcttgggtgggaaaaaggacagggacggccgatccccctcccgcgcttcgtccgcgtatcggcgtcccggcgcggcgagcgtctgacggtctgtctctggcggtcccgcgtcgggtcgtggatccgtgtcggcagccgcgctccgtgtggacgatcggggcgtcctcgggctcatatagtcccaggggccggcgggaaggaggagcagcggaggccgccggccccccgcccccacggcgggcccgccccgaacggaattccattatgcacgaccccgccccgacgccggcacgccgggggcccgtggccgcggcccgttggtcgaacccccggccccgcccatccgcgccatctgccatgggcggggcgctagggcgggtgggcccgcgccccgccccgcatggcatctcattaccgcccgatccggcggtttccgcttccgttccgcatgctaacgaggaacgggcagggggcggggcccgggccccgacttcccggttcggcggtaatgagatacgagccccgcgcgcccgttggccgtccccgggcccccggtcccgcccgccggacgccgggaccaacgggacggcgggcggcccaagggccgcccgccttgccgcccccccattggccggcgggcgggaccgccccaagggggcggggccgccgggtaaaagaagtgagaacgcgaagcgttcgcacttcgtcccaatatatatatattattagggcgaagtgcgagcactggcgccgtgcccgactccgcgccggccccgggggcgggcccgggcggcggggggcgggtctctccggcgcacataaaggcccggcgcgaccgacgcccgcagacggcgccggccacgaacgacgggagctgctgcggagcacgcggaccgggagcgggactcgcagagggccgtcggagcggacggcgtcggcatcgcgacgccccggctcgggatcgggatcgcatcggaaagggacacgcggaaagacccacccaccccacccacgaaacacaggggacgcaccccgggggcctccgacgacagaaacccaccggtccgcctttttgcacgggtaagcaccttgggtgggcggaggagggcggaggaggggggacgcgggggcggaggaggggggacgcgggggcggaggaggggggacgcgggggcggaggaggggggacgcgggggcggaggagggggctcacccgcgttcgtgccttcccgcaggaggaacgtcctcgtcgaggcgaccggcggcgaccgttgcgtggaccgcttcctgctcgtcggggcgaccggcggcgaccgttgcgtggaccgcttcctgctcgtcggggcgaccggcggcgaccgttgcgtggaccgcttcctgctcgtcgggggggggggggggaagccactgtggtcctccgggacgttttctggatggccgacatttccccaggcgcttttgcgccttgtgtaaaagcgcggcgtcccgctctccgatccccgcccctgggcacgcgcaagcgcaagcgccctgcccgccccctctcatcggagtctgaggtcgaaaccgatacagccttggagtctgaggtcgaatccgagacagcatcggattcgaccgagtctggggaccaggaggaagccccccgcatcggtggccgtagggccccccggaggcttggggggcggttttttctggacatgtcggcggaatccaccacggggacggaaacggatacggcggtgtcggacgaccccgacgacacgtccgactggtcttatgacgacattcccccacgacccaagcgggcccgggtaaacctgcggctcacgagctctcccgatcggcgggatggggttatttttcctaagatggggcgggtccggtctacccgggaaacgcagccccgggccccaaccccgtcggccccaagcccaaatgcaatgctacggcgctcggtgcgccaggcccagaggcggagcagcgcacgatggacccccgacctgggctacatgcgccagtgtatcaatcagctgtttcgggtcctgcgggtcgcccgggacccccacggcagtgccaaccgcctgcgccacctgatacgcgactgttacctgatgggatactgccgagcccgtctggccccgcgcacgtggtgccgcttgctgcaggtgtccggcggaacctggggcatgcacctgcgcaacaccatacgggaggtggaggctcgattcgacgccaccgcggaacccgtgtgcaaacttccttgtttggaggccagacggtacggcccggagtgtgatcttagtaatctcgagattcatctcagcgcgacaagcgatgatgaaatctccgatgccaccgatctggaggccgccggttcggaccacacgctcgcgtcccagtccgacacggaggatgccccctcccccgttacgctggaaaccccagaaccccgcgggtccctcgctgtgcgtctggaggatgagtttggggagtttgactggaccccccaggagggctcccagccctggctgtctgcggtcgtggccgataccagctccgtggaacgcccgggcccatccgattctggggcgggtcgcgccgcagaagaccgcaagtgtctggacggctgccggaaaatgcgcttctccaccgcctgcccctatccgtgtagcgacacgtttctccggccgtgagtccggtcgccccgacccctttgtatgtcaccaaaataaaagaccaaaatcaaagcgtttgtcccagcgtcttaatggcgggaagggcggagagaaacagaccacgcggacatggggggtgtttgggggtttattggcaccgggggctaaagggtggtaaccggatagcagatgtgaggaagtcggggccgttcgccgcgaacggcgatcagagggtcagtttcttgcggaccacggcccggcgatgtgggttgctcgtctgggacctcgggcatgcccatacacgcacaacacggacgccgcaccggatgggacgtcgtaagggggcctggggtagctgggtggggtttgtgcagagcaatcagggaccgcagccagcgcatacaatcgcgctcccgtccgtttgtcccgggcagtaccacgccgtactggtattcgtaccggctgagcagggtctccagggggtggttgggggccgcggggaacggggtccacgccacggtccactcgggcaaaaaccgagtcggcacggcccacggttctcccacccacgcgtctggggtcttgatggcgataaatcttaccccgagccggattttttgggcgtattcgagaaacggcacacacagatccgccgcgcctaccacccacaagtggtagatgcgaggggggctgggttggtctcggtgcagcagtcggaagcacgccacggcgtccacgacctcggtgctctccaaggggctgtcctccgcaaacaggcccgtggtggtgtttggggggcagcgacaggacctagtgcgcacgatcgggcgggtgggtttgggtaagtccatcagcggctcggccaaccgtcgaaggttggccggacgaacgacgaccggggtacccaggggttctgatgccaaaatgcggcactgcctaagcaggaagctccacagggccgggcttgcgtcgacggaagtccggggcagggcgttgttctggtcaaggagggtcattacgttgacgacaacaacgcccatgttggtatattacaggcccgtgtccgatttggggcacttgcagatttgtaaggccacgcacggcggggagacaggccgacgcgggggctgctctaaaaatttaagggccctacggtccacagacccgccttcccggggggggggcccttggagcgaccggcagcgtaggcgtccgggggaggggagggtgatttacgggggggtaggtcagggggtgggtcgtcaaactgccgctccttaaaaccccggggcccgtcgttcggggtgctcgttggttggcactcacggtgcggcgaatggcctgtcgtaagttttgtcgcgtttacgggggacagggcaggaggaaggaggaggccgtcccgccggagacaaagccgtcccgggtgtttcctcatggccccttttataccccagccgaggacgcgtgcctggactccccgcccccggagacccccaaaccttcccacaccacaccacccagcgaggccgagcgcctgtttcatctgcaggagatccttgcccagatgtacggaaaccaggactaccccatagaggacgaccccagcgcggatgccgcggacgatgtcgacgaggacgccccggacgacgtggcctatccggaggaatacgcagaggagctttttctgcccggggacgcgaccggtccccttatcggggccaacgaccacatccctcccccgtgtggcgcatctccccccggtatacgacgacgcagccgggatgagattggggccacgggatttaccgcggaagagctggacgccatggacagggaggcggctcgagccatcagccgcggcggcaagcccccctcgaccatggccaagctggtgactggcatgggctttacgatccacggagcgctcaccccaggatcggaggggtgtgtctttgatagcagccacccagattacccccaacgggtaatcgtgaaggcggggtggtacacgagcacgagccacgaggcgcgactgctgaggcgactggaccaccccgcgatcctgcccctcctggacctgcatgtcgtctccggggtcacgtgtctggtcctccccaagtaccaggccgacctgtatacctatctgagtaggcgcctgaacccgctgggacgcccgcagatcgcagcggtctcccggcagctcctaagcgccgttgactacattcaccgccagggcattatccaccgcgacattaagaccgaaaatatttttattaacacccccgaggacatttgcctgggggactttggtgccgcgtgcttcgtgcagggttcccgatcaagccccttcccctacggaatcgccggaaccatcgacaccaacgcccccgaggtcctggccggggatccgtataccacgaccgtcgacatttggagcgccggtctggtgatcttcgagactgccgtccacaacgcgtccttgttctcggccccccgcggccccaaaaggggcccgtgtgacagtcagatcacccgcatcatccgacaggcccaggtccacgttgacgagttttccccgcatccagaatcgcgcctcacctcgcgctaccgctcccgcgcggccgggaacaatcgcccgccttacacccgaccggcctggacccgctactacaagatggacatagacgtcgaatatctggtttgcaaagccctcaccttcgacggcgcgcttcgccccagcgccgcagagctgctttgtttgccgctgtttcaacagaaatgaccgcccccggggggcggtgctgtttgcgggttggcacaaaaagaccccgacccgcgtctgtggtgtttttggcatcatgtcgccgggcgccatgcgtgccgttgttcccattatcccattccttttggttcttgtcggtgtatcgggggttcccaccaacgtctcctccaccacccaaccccaactccagaccaccggtcgtccctcgcatgaagcccccaacatgacccagaccggcaccaccgactctcccaccgccatcagccttaccacgcccgaccacacaccccccatgccaagtatcggactggaggaggaggaggaagaggaggagggggccggggatggcgaacatcttaaggggggagatgggacccgtgacaccctaccccagtccccgggtccagccgtcccgttggccggggatgacgagaaggacaaacccaaccgtcccgtagtcccaccccccggtcccaacaactcccccgcgcgccccgagaccagtcgaccgaagacaccccccaccagtatcgggccgctggcaactcgacccacgacccaactcccctcaaaggggcgacccttggttccgacgcctcaacataccccgctgttctcgttcctcactgcctcccccgccctggacaccctcttcgtcgtcagcaccgtcatccacaccttatcgtttttgtgtattggtgcgatggcgacacacctgtgtggcggttggtccagacgcgggcgacgcacacaccctagcgtgcgttacgtgtgcctgccgtccgaacgcgggtagggtatggggcgggggatggggagagcccacatgcggaaagcaagaacaataaaggcggtggtatctagttgatatgcatctctgggtgtttttggggtgtggcggacgcggggcggtcattggacggggtgcagttaaatacatgcccgggacccatgaagcatgcgcgacttccgggcctcggaacccacccgaaacggccaacggacgtctgagccaggcctggctatccggagaaacagcacacgacttggcgttctgtgtgtcgcgatgtctctgcgcgcagtctggcatctggggcttttgggaagcctcgtgggggctgttcttgccgccacccatcggggacctgcggccaacacaacggaccccttaacgcacgccccagtgtcccctcaccccagccccctggggggctttgccgtccccctcgtagtcggtgggctgtgcgccgtagtcctgggggcggcgtgtctgcttgagctcctgcgtcgtacgtgccgcgggtgggggcgttaccatccctacatggacccagttgtcgtataattcccccccccccttctccgcatgggtgatgtcgggtccaaactcccgacaccaccagctggcatggtataaatcaccggtgcgccccccaaaccatgtccggcagggggatgggggggcgaatgcggagggcacccaacaacaccgggctaaccaggaaatccgtggccccggcccccaataaagatcgcggtagcccggccgtgtgacactatcgtccataccgaccacaccgacgaatcccctaagggggaggggccattttacgaggaggaggggtataacaaagtctgtctttaaaaagcaggggttagggagttgttcggtcataagcttcagcgcgaacgaccaactaccccgatcatcagttatccttaaggtctcttttgtgtggtgcgttccggtatggggggggctgccgccaggttgggggccgtgattttgtttgtcgtcatagtgggcctccatggggtccgcggcaaatatgccttggcggatgcctctctcaagatggccgaccccaatcgctttcgcggcaaagaccttccggtcctggaccagctgaccgaccctccgggggtccggcgcgtgtaccacatccaggcgggcctaccggacccgttccagccccccagcctcccgatcacggtttactacgccgtgttggagcgcgcctgccgcagcgtgctcctaaacgcaccgtcggaggccccccagattgtccgcggggcctccgaagacgtccggaaacaaccctacaacctgaccatcgcttggtttcggatgggaggcaactgtgctatccccatcacggtcatggagtacaccgaatgctcctacaacaagtctctgggggcctgtcccatccgaacgcagccccgctggaactactatgacagcttcagcgccgtcagcgaggataacctggggttcctgatgcacgcccccgcgtttgagaccgccggcacgtacctgcggctcgtgaagataaacgactggacggagattacacagtttatcctggagcaccgagccaagggctcctgtaagtacgccctcccgctgcgcatccccccgtcagcctgcctgtccccccaggcctaccagcagggggtgacggtggacagcatcgggatgctgccccgcttcatccccgagaaccagcgcaccgtcgccgtatacagcttgaagatcgccgggtggcacgggcccaaggccccatacacgagcaccctgctgcccccggagctgtccgagacccccaacgccacgcagccagaactcgccccggaagaccccgaggattcggccctcttggaggaccccgtggggacggtggcgccgcaaatcccaccaaactggcacataccgtcgatccaggacgccgcgacgccttaccatcccccggccaccccgaacaacatgggcctgatcgccggcgcggtgggcggcagtctcctggcagccctggtcatttgcggaattgtgtactggatgcgccgccgcactcaaaaagccccaaagcgcatacgcctcccccacatccgggaagacgaccagccgtcctcgcaccagcccttgttttactagatacccccccttaatgggtgcgggggggtcaggtctgcggggttgggatgggaccttaactccatataaagcgagtctggaaggggggaaaggcggacagtcgataagtcggtagcgggggacgcgcacctgttccgcctgtcgcacccacagctttttttgcgaaccgtcccgttccgggatgccgtgccgcccgttgcagggcctggtgctcgtgggcctctgggtctgtgccaccagcctggttgtccgtggccccacggtcagtctggtatcaaactcatttgtggacgccggggccttggggcccgacggcgtagtggaggaagacctgcttattctcggggagcttcgctttgtgggggaccaggtcccccacaccacctactacgatggggtcgtagagctgtggcactaccccatgggacacaaatgcccacgggtcgtgcatgtcgtcacggtgaccgcgtgcccacgtcgccccgccgtggctttcgccctgtgtcgcgcgaccgacaacactcacagccccgcatatcccaccctggagctgaatctggcccaacagccgcttttgcgggtccggagggcgacgcgtgactatgccggggtgtacgtgttacgcgtatgggtcgtggacgcaccaaacgccagcctgtttgtcctggggatggccatagccgccgaagggactctggcgtacaacggctcggcccatggctcctgcgacccgaaactgcttccgtattcggccccgcgtctggccccggcgagcgtataccaacccgcccctaacccggcctccaccccctcgaccaccacctccaccccctcgaccaccacctccaccccctcgaccaccacctccaccccctcgaccaccacctccaccccctcgaccaccacctccaccccctcgaccaccacctccaccccctcgaccaccatccccgctccccaagcatcgaccacacccttccccacgggagacccaaaaccccaacctcacggggtcaaccacgaacccccatcgaatgccacgcgagcgacccgcgactcgcgatacgcgctaacggtgacccagataatccagatagccatccccgcgtccattatagccctggtgtttctggggagctgtatttgctttatacacagatgtcaacgccgctaccgacgctcccgccgcccgatttacaacccccagatacccacgggcatctcatgcgcggtgaacgaagcggccatggcccgcctcggagccgagctcaaatcgcatccgagcaccccccccaaatcccggcgccggtcgtcacgcacgccaatgccctccctgacggccatcgccgaagagtcggagcccgcgggggcggctgggcttccgacgccccccgtggaccccacgacatccaccccaacgcctcccctgttggtataggtccacggccactggccgggggcaccacataaccgaccgcagtcactgagttgggaataaaccggtattatttacctatatccgtgtatgtccatttctttcccccccccccccccccggaaacccaaagaaggaagcaaagaatggatgggaggagttcaggaagccggggagagggcccgcggcgcatttaaggcgttgttgtgttgactttggctcttctggcgggttggtgcggtgctgtttgttgggctcccattttacccgaagatcggctgctatccccgggacatggatcgcggggcggtggtggggtttcttctcggtgtttgtgttgtatcgtgcttggcgggaatgcccaaaacgtcctggagacgggtgagtgtcggcgaggacgtttcgttgcttccagctccggggcctacggggcgcggcccgacccagaaactactatgggccgtggaacccctggatgggtgcggccccttacacccgtcgtgggtctcgctgatgccccccaagcaggtgcccgagacggtcgtggatgcggcgtgcatgcgcgctccggtcccgctggcgatggcgtacgcccccccggccccatctgcgaccgggggtctacgaacggacttcgtgtggcaggagcgcgcggccgtggttaaccggagtctggttattcacggggtccgagagacggacagcggcctgtataccctgtccgtgggcgacataaaggacccggctcgccaagtggcctcggtggtcctggtggtgcaaccggccccagttccgaccccacccccgaccccagccgattacgacgaggatgacaatgacgagggcgagggcgaggacgaaagtctagccggcactcccgccagcgggaccccccggctcccgcctccccccgcccccccgaggtcttggcccagcgcccccgaagtctcacacgtgcgtggggtgaccgtgcgtatggagactccggaagctatcctgttttcccccggggaggcgtttagcacgaacgtctccatccatgccatcgcccacgacgaccagacctacaccatggacgtcgtctggttgaggttcgacgtgccgacctcgtgtgccgagatgcgaatatacgaatcgtgtctgtatcacccgcagctcccagagtgtctgtccccggccgacgctccgtgcgccgcgagtacgtggacgtctcgcctggccgtccgcagctacgcggggtgttccagaacaaaccccccgccgcgctgttcggccgaggctcacatggagcccttcccggggctggcgtggcaggcggcctccgtcaatctggagttccgggacgcgtccccacaacactccggcctgtatctgtgcgtggtgtacgtcaacgaccatattcacgcatggggccacattaccatcagcaccgcggcgcagtaccggaacgcggtggtggaacagcccctcccacagcgcggcgcggatttggccgagcccacccacccgcacgtcggggcccctccccacgcgcccccaacccacggcgccctgcggttaggggcggtgatgggggccgccctgctgctgtctgcgctggggttgtcggtgtgggcgtgtatgacctgttggcgcaggcgtgcctggcgggcggttaaaagcagggcctcgggtaaggggcccacgtacattcgcgtggccgacagcgagctgtacgcggactggagctcggacagcgagggagaacgcgaccaggtcccgtggctggcccccccggagagacccgactctccctccaccaatggatccggctttgagatcttatcaccaacggctccgtctgtatacccccgtagcgatgggcatcaatctcgccgccagctcacaacctttggatccggaaggcccgatcgccgttactcccaggcctccgattcgtccgtcttctggtaaggcgccccatcccgaggccccacgtcggtcgccgaactgggcgaccgccggcgaggtggacgtcggagacgagctaatcgcgatttccgacgaacgcggacccccccgacatgaccgcccgcccctcgccacgtcgaccgcgccctcgccacacccgcgacccccgggctacacggccgttgtctccccgatggccctccaggctgtcgacgccccctccctgtttgtcgcctggctggccgctcggtggctccggggggcttccggcctgggggccgtcttgtgtgggattgcgtggtatgtgacgtcaattgcccgaggcgcataaagggccggtggtccgcctagccgcagcaaattaaaaatcgtgagtcactgcgaccgcaacttcccacccggagctttcttccggcctcgatgacgtcccggctctccgatcccaactcctcagcgcgatccgacatgtccgtgccgctttatcccacggcctcgccagtttcggtcgaagcctactactcggaaagcgaagacgaggcggccaacgacttcctcgtacgcatgggccgccaacagtcggtattaaggcgtcgacgcagacgcacccgctgcgtcggcatggtgatcgcctgtctcctcgtggccgttctgtcgggcggatttggggcgctcctgatgtggctgctccgctaaaagaccgcatcgacacgcgcgtccttcttgtcgtctctcttccccccatcaccccgcaatttgcacccagcctttaactacattaaattgggttcgattggcaatgttgtctcccggttgatttttgggtgggtggggagtgggtgggtggggagtgggtgggtggggagtgggtgggtggggagtgggtgggtggggagtgggtgggtggggagtgggtgggtggggagtgggtgggtggggagtgggtgggtggggagtgggtgggtggggagtgggtgggtggggagtgggtgggtggggagtgggtgggtggggagtgggtgggtggggagtgggtgggtggggagtgggtgggtggggagtggcaaggaagaaacaagcccgaccaccagacagaaaatgtaaccatacccaaaccgactctgggggctgtttgtggggtcggaaccataggatgaacaaaccaccccgtacctcccgcacccttgggtgcgggtggctcatcggcatctgtccggtatgggttgttccccacccactcgcgttcggacgtcttagaatcatggcggtttctatgccgacatcggtttctcccccgcaataagacacgatgcgataaaatctgtttgtgaaatttattaagggtacaaattgccctagcacaggggtggggttagggccgggtccccacacccaaacgcaccaaacagatgcaggcagtgggtcgagtacagccccgcgtacgaacacgtcgatgcgtgtgtcagacagcaccagaaagcacaggccatcaacaggtcgtgcatgtgtcggtgggtttggacgcggggggccatggtgggtgataaagttaatggccgccgtccgccagggccacaggggcgacgtctcttggttggcccggagccactgggtgtggaccagccgcgcgtggcggcccaacatggcccctgtagccgggggcgggggatcgcgcacgtttgcagcgcacatgcgagacacctcgaccacggttcggaagaaggcccggtggtccgcgggcaacatcaccaggtgcgcaagcgcccgggcgtccagagggtagagccctgagtcatccgaggttggctcatcgcccgggtcatgccgcaagtgcgtgtgggttgggcttccggtgggcgggacgcgaaccgcggtgtggagcccgacgcgggcccgagcgtacgctccatcttgtggggagaaggggtctgggctcgccaggggggcatacttgcccgggctatacagacccgcgagccgtacgtggttcgcggggggtgcgtggggtccggggctcccggggaggccggggctcccggggttgtcgtggatccctggggtcacgcggtaccctggggtctctgggagctcgcggtactctgggttccctaggttctcggggtggtcgcggaacccggggctcccggggaacacgcggtgtcctggggattgttggcggtcggacggcttcagatggcttcgagatcgtagtgtccgcaccgactcgtagtagacccgaatctccacattgccctgccgcttgatcattatcaccccgttgcgggggtccggagatcatgcgcgggtgtcctcgaggtgcgtgaacacctctggggtgcatgccggcggacggcacgccttttaagtaaacatctgggtcgcccggcccaactggggccgggggttgggtctggctcatctcgagagccacggggggaaccaccctccgcccagaaacttgggcgatggtcgtacccgggactcaacgggttaccggattacggggactgtcggtcacggtcccgccggttcttcgatgtgccacacccaaggatgcgttgggggcgattttgggcagcagcccgggagagcgcagcagaggacgctccgggtcgtgcacggcggttctggccgcctcccggtcctcacgcccccttttattgatctcatcgcgtacgtcggcgtacgtcctgggcccaacccgcatgttgtccaggaaggtgtccgccatttccagggcccacgacatgctcccccccccccccccgacgagcaggaagcggtccacgcaacggtcgccgccggtcgccccgacgagcaggaagcggtccacgcaacggtcgccgccggtcgccccgacgagcaggaagcggtccacgcaacggtcgccgccggtcgcctcgacgaggacgttcctcctgcgggaaggcacgaacgcgggtgagccccctcctccgcccccgcgtcccccctcctccgcccccgcgtcccccctcctccgcccccgcgtcccccctcctccgcccccgcgtcccccctcctccgccctcctccgcccacccaaggtgcttacccgtgcaaaaaggcggaccggtgggtttctgtcgtcggaggcccccggggtgcgtcccctgtgtttcgtgggtggggtgggtgggtctttccgcgtgtccctttccgatgcgatcccgatcccgagccggggcgtcgcgatgccgacgccgtccgctccgacggccctctgcgagtcccgctcccggtccgcgtgctccgcagcagctcccgtcgttcgtggccggcgccgtctgcgggcgtcggtcgcgccgggcctttatgtgcgccggagagacccgccccccgccgcccgggcccgcccccggggccggcgcggagtcgggcacggcgccagtgctcgcacttcgccctaataatatatatatattgggacgaagtgcgaacgcttcgcgttctcacttcttttacccggcggccccgcccccttggggcggtcccgcccgccggccaatgggggggcggcaaggcgggcggcccttgggccgcccgccgtcccgttggtcccggcgtccggcgggcgggaccgggggcccggggacggccaacgggcgcgcggggctcgtatctcattaccgccgaaccgggaagtcggggcccgggccccgccccctgcccgttcctcgttagcatgcggaacggaagcggaaaccgccggatcgggcggtaatgagatgccatgcggggcggggcgcgggcccacccgccctagcgccccgcccatggcagatggcgcggatgggcggggccgggggttcgaccaacgggccgcggccacgggcccccggcgtgccggcgtcggggcggggtcgtgcataatggaattccgttcggggcgggcccgccgtgggggcggggggccggcggcctccgctgctcctccttcccgccggcccctgggactatatgagcccgaggacgccccgatcgtccacacggagcgcggctgccgacacggatccacgacccgacgcgggaccgccagagacagaccgtcagacgctcgccgcgccgggacgccgatacgcggacgaagcgcgggagggggatcggccgtccctgtcctttttcccacccaagcatcgaccggtccgcgctagttccgcgtcgacggcgggggtcgtcggggtccgtgggtctcgccccctccccatcgagagtccgtaggtgacctaccgtgctacgtccgccgtcgcagtcgtatccccggaggatcgccccgcatcggcgatggcgtcggagaacaagcagcgccccggctccccgggccccaccgacgggccgccgcccaccccgagcccagaccgcgacgagcggggggccctcgggtggggcgcggagacggaggagggcggggacgaccccgaccacgaccccgaccacccccacgacctcgacgacgcccggcgggacgggagggcccccgcggcgggcaccgacgccggcgaggacgccggggacgccgtctcgccgcgacagctggccctgctggcctccatggtagaggaggccgtccggacgatcccgacgcccgaccccgcggcctcgccgccccggacccccgcctttcgagccgacgacgatgacggggacgagtacgacgacgcagccgacgccgccggcgaccgggccccggcccggggccgcgcacgggaggccccgctacgcggcgcgtatccggaccccacggaccgcctgtcgccgcgcccgccggcccagccgccgcagagacgtcgtcacggccggcggcggccatcggcgtcatcgacctcgtcggactccgggtcctcgtcctcgtcgtccgcatcctcttcgtcctcgtcgtccgacgaggacgaggacgacgacggcaacgacgcggccgaccacgcacgcgaggcgcgggccgtcgggcggggtccgtcgagcgcggcgccggaagcccccgggcggacgccgcccccgcccgggccaccccccctctccgaggccgcgcccaagccccgggcggcggcgaggacccccgcggcctccgcgggccgcatcgagcgccgccgggcccgcgcggcggtggccggccgcgacgccacgggccgcttcacggccgggcagccccggcgggtcgagctggacgccgacgcggcctccggcgccttctacgcgcgctatcgcgacgggtacgtcagcggggagccgtggcccggcgccgggcccccgcccccggggcgggtgctgtacggcggcctgggcgacagccgcccgggcctctggggggcgcccgaggcggaggaggcgcgacgccggttcgaggcctcgggcgccccggcggccgtgtgggcgcccgagctgggcgacgccgcgcagcagtacgccctgatcacgcggctgctgtacaccccggacgcggaggccatggggtggctccagaacccgcgcgtggtccccggggacgtggcgctggaccaggcctgcttccggatctcgggcgccgcgcgcaacagcagctccttcatcaccggcagcgtggcgcgggccgtgccccacctgggctacgccatggcggccggccgcttcggctggggcctggcgcacgcggcggccgccgtggccatgagccgccgatacgaccgcgcgcagaagggcttcctgctgaccagcctgcgccgcgcctacgcgcccctgttggcgcgcgagaacgcggcgctgacgggggccgcggggagccccggcgccggcgcagatgacgagggggtcgccgccgccgtcgtcgccgccgccgccgcaccgggcgagcgcgcggtgcccgccgggtacggcgccgcggggatcctcgccgccctggggcggctgtccgccgcgcccgcctcccccgcggggggcgacgaccccgacgccgcccgccacgccgacgccgacgacgacgccgggcgccgcgcccaggccggccgcgtggccgtggagtgcctggccgcctgccgcgggatcctggaggcgctggccgagggcttcgacggcgacctggcggccgtcccggggctggccggggcccggcccgccagccccccgcggccggagggacccgcgggccccgcttccccgccgccgccgcacgccgacgcgccccgcctgcgcgcgtggctgcgcgagctgcggttcgtgcgcgacgcgctggtgctcatgcgcctgcgcggggacctgcgcgtggccggcggcagcgaggccgccgtggccgccgtgcgcgccgtgagcctggtcgccggggccctgggtcccgcgctgccgcgggacccgcgcctgccgagctccgcggccgccgccgccgcggacctgctgtttgagaaccagagcctgcgccccctgctggcggcgggtccgcgccgctcttcttcgtcttcgggggtcgcggccgccgcctccgccgcgccgcgggaggggcgcaagcgcaagagtcccggcccggcccggccgcccggaggcggcggcccgcgacccccgaagacgaagaagagcggcgcggacgcccccggctcggacgcccgcgcccccctccccgcgcccgcgcccccctccacgcccccggggcccgagcccgcccccgcccagcccgcggcgccccgggccgccgcggcgcaggcccgcccgcgccccgtggcgctgtcgcgccggcccgccgagggccccgaccccctgggcggctggcggcggcagcccccggggcccagccacacggcggcgcccgcggccgccgccctggaggcctactgctccccgcgcgccgtggccgagctcacggaccacccgctgttccccgtcccctggcgaccggccctcatgtttgacccgcgggccctggcctcgatcgccgcgcggtgcgccgggcccgcccccgccgcccaggccgcgtgcggcggcggcgacgacgacgagaacccccacccccacggggccgccgggggccgcctctttggccccctgcgcgcctcgggcccgctgcgccgcatggcggcctggatgcgccagatccccgaccccgaggacgtgcgcgtggtggtgctgtactcgccgctgccgggcgaggacctggccggcggcggggcctcgggggggccgccggagtggtccgccgagcgcggcgggctgtcctgcctgctggcggccctggccaaccggctgtgcgggccggacacggccgcctgggcgggcaactggaccggcgcccccgacgtgtcggcgctgggcgcgcagggcgtgctgctgctgtccacgcgggacctggccttcgccggggccgtggagtttctggggctgctcgccagcgccggcgaccggcggctcatcgtggtcaacaccgtgcgcgcctgcgactggcccgccgacgggcccgcggtgtcgcggcagcacgcctacctggcgtgcgacctgctgcccgccgtgcagtgcgccgtgcgctggccggcggcgcgcgacctgcgccgcacggtgctggcctcgggccgcgtgttcggcccgggggtcttcgcgcgcgtggaggccgcgcacgcgcgcctgtaccccgacgcgccgccgctgcgcctgtgccgcggcggcaacgtgcgctaccgcgtgcgcacgcgcttcggcccggacacgccggtgcccatgtccccgcgcgagtaccgccgggccgtgctgccggcgctggacggccgggcggcggcctcggggaccaccgacgccatggcgcccggcgcgccggacttctgcgaggaggaggcccactcgcaccgcgcctgcgcgcgctggggcctgggcgcgccgctgcggcccgtgtacgtggcgctggggcgcgaggcggtgcgcgccggcccggcccggtggcgcgggccgcggagggacttttgcgcccgcgccctgctggagcccgacgacgacgcccccccgctggtgctgcgcggcgacgacgacggcccgggggccctgccgccggcgccgcccgggattcgctgggcctcggccacgggccgcagcggcaccgtgctggcggcggcgggggccgtggaggtgctgggggcggaggcgggcttggccacgcccccgcgacgggacgttgtggactgggaaggcgcctgggacgaagacgacggcggcgcgttcgagggggacggggtgctgtaacgggccgggacggggcggggcgcttgtgaaacccgaagacgcaataaacggcaacgacctgattaagttttgcagtagcgttgtttattcgaggggcgggagggggcgaggggcgggagggggcgaggggcgggagggggcgaggggcgggagggggcgaggggcgggagggggcgaggggcgggagggggcgaggggcgggagggggcgaggggcgggagggggcgaggggcggtggtggtgcgcgggcgcccccggagggtttggatctctgacctgagattggcggcactgaggtagagatgcccgaacccccccgagggagcgcgggacgcggctggggagggctggggctggggagggctggggctggggagggctggggctggggagggctggggctggggagggctggggctggggagggctggggctggggagggctggggctggggagggctggggctggggagggctggggctggggagggctggggctggggagggctggggctggggagggctggggctgtggtgtgtgacaggagcggcgtgttgcgctgggggacgtctggaggagcggggggtgcgcggtgacgtgtggatgaggaacaggagttgttgcgcggtgagttgtcgctgtgagttgtgttgttgggcaggtgtgttggatgacgtgacgtgtggatgaggaaccggagtcgccggtgcgccgtgctgttggtgttctgttggtgttgttacacctgtggcagcccgggccccccgcgcgcggggcggcgcgcaaaaaaggcgggcggcggtccgggcggcgtgcgcgcgcgcggcgggcgtggggggcggggccgcgggagcgggggaggagccccacccacagacggggaggagcgggggaggagcgggggaggagcgggggaggagccccacccacagacggggaggagcgggggaggagcggccagaccccaaaaacgggcccccccgaaacacaccccccgggggtcgcgcgcggccctttaaagcgcggcggcgggcagcccgggccccccgcgg

SEQ ID NO: 2 - protein, 1300 aa, unidentified
  source 1..1300: note = human herpesvirus 1 strain McKrae ICP4
MASENKQRPGSPGPTDGPPPTPSPDRDERGALGWGAETEEGGDDPDHDPDHPHDLDDARRDGRAPAAGTDAGEDAGDAVSPRQLALLASMVEEAVRTIPTPDPAASPPRTPAFRADDDDGDEYDDAADAAGDRAPARGRAREAPLRGAYPDPTDRLSPRPPAQPPQRRRHGRRRPSASSTSSDSGSSSSSSASSSSSSSDEDEDDDGNDAADHAREARAVGRGPSSAAPEAPGRTPPPPGPPPLSEAAPKPRAAARTPAASAGRIERRRARAAVAGRDATGRFTAGQPRRVELDADAASGAFYARYRDGYVSGEPWPGAGPPPPGRVLYGGLGDSRPGLWGAPEAEEARRRFEASGAPAAVWAPELGDAAQQYALITRLLYTPDAEAMGWLQNPRVVPGDVALDQACFRISGAARNSSSFITGSVARAVPHLGYAMAAGRFGWGLAHAAAAVAMSRRYDRAQKGFLLTSLRRAYAPLLARENAALTGAAGSPGAGADDEGVAAAVVAAAAAPGERAVPAGYGAAGILAALGRLSAAPASPAGGDDPDAARHADADDDAGRRAQAGRVAVECLAACRGILEALAEGFDGDLAAVPGLAGARPASPPRPEGPAGPASPPPPHADAPRLRAWLRELRFVRDALVLMRLRGDLRVAGGSEAAVAAVRAVSLVAGALGPALPRDPRLPSSAAAAAADLLFENQSLRPLLAAGPRRSSSSSGVAAAASAAPREGRKRKSPGPARPPGGGGPRPPKTKKSGADAPGSDARAPLPAPAPPSTPPGPEPAPAQPAAPRAAAAQARPRPVALSRRPAEGPDPLGGWRRQPPGPSHTAAPAAAALEAYCSPRAVAELTDHPLFPVPWRPALMFDPRALASIAARCAGPAPAAQAACGGGDDDENPHPHGAAGGRLFGPLRASGPLRRMAAWMRQIPDPEDVRVVVLYSPLPGEDLAGGGASGGPPEWSAERGGLSCLLAALANRLCGPDTAAWAGNWTGAPDVSALGAQGVLLLSTRDLAFAGAVEFLGLLASAGDRRLIVVNTVRACDWPADGPAVSRQHAYLACDLLPAVQCAVRWPAARDLRRTVLASGRVFGPGVFARVEAAHARLYPDAPPLRLCRGGNVRYRVRTRFGPDTPVPMSPREYRRAVLPALDGRAAASGTTDAMAPGAPDFCEEEAHSHRACARWGLGAPLRPVYVALGREAVRAGPARWRGPRRDFCARALLEPDDDAPPLVLRGDDDGPGALPPAPPGIRWASATGRSGTVLAAAGAVEVLGAEAGLATPPRRDVVDWEGAWDEDDGGAFEGDGVL

SEQ ID NO: 3 - protein, 420 aa, unidentified
  source 1..420: note = human herpesvirus 1 strain McKrae ICP22
MADISPGAFAPCVKARRPALRSPPLGTRKRKRPARPLSSESEVETDTALESEVESETASDSTESGDQEEAPRIGGRRAPRRLGGRFFLDMSAESTTGTETDTAVSDDPDDTSDWSYDDIPPRPKRARVNLRLTSSPDRRDGVIFPKMGRVRSTRETQPRAPTPSAPSPNAMLRRSVRQAQRRSSARWTPDLGYMRQCINQLFRVLRVARDPHGSANRLRHLIRDCYLMGYCRARLAPRTWCRLLQVSGGTWGMHLRNTIREVEARFDATAEPVCKLPCLEARRYGPECDLSNLEIHLSATSDDEISDATDLEAAGSDHTLASQSDTEDAPSPVTLETPEPRGSLAVRLEDEFGEFDWTPQEGSQPWLSAVVADTSSVERPGPSDSGAGRAAEDRKCLDGCRKMRFSTACPYPCSDTFLRP

SEQ ID NO: 4 - protein, 88 aa, unidentified
  source 1..88: note = human herpesvirus 1 strain McKrae ICP47
MSWALEMADTFLDNMRVGPRTYADVRDEINKRGREDREAARTAVHDPERPLLRSPGLLPKIAPNASLGVAHRRTGGTVTDSPRNPVTR

SEQ ID NO: 5 - DNA, 4020 bp, unidentified
  source 1..4020: mol_type = genomic DNA; note = human herpesvirus 1 strain McKrae ICP4
tttattgcgtcttcgggtttcacaagcgccccgccccgtcccggcccgttacagcaccccgtccccctcgaacgcgccgccgtcgtcttcgtcccaggcgccttcccagtccacaacgtcccgtcgcgggggcgtggccaagcccgcctccgcccccagcacctccacggcccccgccgccgccagcacggtgccgctgcggcccgtggccgaggcccagcgaatcccgggcggcgccggcggcagggcccccgggccgtcgtcgtcgccgcgcagcaccagcgggggggcgtcgtcgtcgggctccagcagggcgcgggcgcaaaagtccctccgcggcccgcgccaccgggccgggccggcgcgcaccgcctcgcgccccagcgccacgtacacgggccgcagcggcgcgcccaggccccagcgcgcgcaggcgcggtgcgagtgggcctcctcctcgcagaagtccggcgcgccgggcgccatggcgtcggtggtccccgaggccgccgcccggccgtccagcgccggcagcacggcccggcggtactcgcgcggggacatgggcaccggcgtgtccgggccgaagcgcgtgcgcacgcggtagcgcacgttgccgccgcggcacaggcgcagcggcggcgcgtcggggtacaggcgcgcgtgcgcggcctccacgcgcgcgaagacccccgggccgaacacgcggcccgaggccagcaccgtgcggcgcaggtcgcgcgccgccggccagcgcacggcgcactgcacggcgggcagcaggtcgcacgccaggtaggcgtgctgccgcgacaccgcgggcccgtcggcgggccagtcgcaggcgcgcacggtgttgaccacgatgagccgccggtcgccggcgctggcgagcagccccagaaactccacggccccggcgaaggccaggtcccgcgtggacagcagcagcacgccctgcgcgcccagcgccgacacgtcgggggcgccggtccagttgcccgcccaggcggccgtgtccggcccgcacagccggttggccagggccgccagcaggcaggacagcccgccgcgctcggcggaccactccggcggcccccccgaggccccgccgccggccaggtcctcgcccggcagcggcgagtacagcaccaccacgcgcacgtcctcggggtcggggatctggcgcatccaggccgccatgcggcgcagcgggcccgaggcgcgcagggggccaaagaggcggcccccggcggccccgtgggggtgggggttctcgtcgtcgtcgccgccgccgcacgcggcctgggcggcgggggcgggcccggcgcaccgcgcggcgatcgaggccagggcccgcgggtcaaacatgagggccggtcgccaggggacggggaacagcgggtggtccgtgagctcggccacggcgcgcggggagcagtaggcctccagggcggcggccgcgggcgccgccgtgtggctgggccccgggggctgccgccgccagccgcccagggggtcggggccctcggcgggccggcgcgacagcgccacggggcgcgggcgggcctgcgccgcggcggcccggggcgccgcgggctgggcgggggcgggctcgggccccgggggcgtggaggggggcgcgggcgcggggaggggggcgcgggcgtccgagccgggggcgtccgcgccgctcttcttcgtcttcgggggtcgcgggccgccgcctccgggcggccgggccgggccgggactcttgcgcttgcgcccctcccgcggcgcggcggaggcggcggccgcgacccccgaagacgaagaagagcggcgcggacccgccgccagcagggggcgcaggctctggttctcaaacagcaggtccgcggcggcggcggccgcggagctcggcaggcgcgggtcccgcggcagcgcgggacccagggccccggcgaccaggctcacggcgcgcacggcggccacggcggcctcgctgccgccggccacgcgcaggtccccgcgcaggcgcatgagcaccagcgcgtcgcgcacgaaccgcagctcgcgcagccacgcgcgcaggcggggcgcgtcggcgtgcggcggcggcggggaagcggggcccgcgggtccctccggccgcggggggctggcgggccgggccccggccagccccgggacggccgccaggtcgccgtcgaagccctcggccagcgcctccaggatcccgcggcaggcggccaggcactccacggccacgcggccggcctgggcgcggcgcccggcgtcgtcgtcggcgtcggcgtggcgggcggcgtcggggtcgtcgccccccgcgggggaggcgggcgcggcggacagccgccccagggcggcgaggatccccgcggcgccgtacccggcgggcaccgcgcgctcgcccggtgcggcggcggcggcgacgacggcggcggcgaccccctcgtcatctgcgccggcgccggggctccccgcggcccccgtcagcgccgcgttctcgcgcgccaacaggggcgcgtaggcgcggcgcaggctggtcagcaggaagcccttctgcgcgcggtcgtatcggcggctcatggccacggcggccgccgcgtgcgccaggccccagccgaagcggccggccgccatggcgtagcccaggtggggcacggcccgcgccacgctgccggtgatgaaggagctgctgttgcgcgcggcgcccgagatccggaagcaggcctggtccagcgccacgtccccggggaccacgcgcgggttctggagccaccccatggcctccgcgtccggggtgtacagcagccgcgtgatcagggcgtactgctgcgcggcgtcgcccagctcgggcgcccacacggccgccggggcgcccgaggcctcgaaccggcgtcgcgcctcctccgcctcgggcgccccccagaggcccgggcggctgtcgcccaggccgccgtacagcacccgccccgggggcgggggcccggcgccgggccacggctccccgctgacgtacccgtcgcgatagcgcgcgtagaaggcgccggaggccgcgtcggcgtccagctcgacccgccggggctgcccggccgtgaagcggcccgtggcgtcgcggccggccaccgccgcgcgggcccggcggcgctcgatgcggcccgcggaggccgcgggggtcctcgccgccgcccggggcttgggcgcggcctcggagagggggggtggcccgggcgggggcggcgtccgcccgggggcttccggcgccgcgctcgacggaccccgcccgacggcccgcgcctcgcgtgcgtggtcggccgcgtcgttgccgtcgtcgtcctcgtcctcgtcggacgacgaggacgaagaggatgcggacgacgaggacgaggacccggagtccgacgaggtcgatgacgccgatggccgccgccggccgtgacgacgtctctgcggcggctgggccggcgggcgcggcgacaggcggtccgtggggtccggatacgcgccgcgtagcggggcctcccgtgcgcggccccgggccggggcccggtcgccggcggcgtcggctgcgtcgtcgtactcgtccccgtcatcgtcgtcggctcgaaaggcgggggtccggggcggcgaggccgcggggtcgggcgtcgggatcgtccggacggcctcctctaccatggaggccagcagggccagctgtcgcggcgagacggcgtccccggcgtcctcgccggcgtcggtgcccgccgcgggggccctcccgtcccgccgggcgtcgtcgaggtcgtgggggtggtcggggtcgtggtcggggtcgtccccgccctcctccgtctccgcgccccacccgagggccccccgctcgtcgcggtctgggctcggggtgggcggcggcccgtcggtggggcccggggagccggggcgctgcttgttctccgacgccatcgccgatgcggggcgatcctccggggatacgactgcgacggcggacgtagcacggtaggtcacctacgg

SEQ ID NO: 6 - DNA, 1320 bp, unidentified
  source 1..1320: mol_type = genomic DNA; note = human herpesvirus 1 strain McKrae ICP22
ggtcctccgggacgttttctggatggccgacatttccccaggcgcttttgtgccttgtgtaaaagcgcggcgtcccgctctccgatccccgcccctgggcacgcgcaagcgcaagcgccctgcccgccccctctcatcggagtctgaggtcgaatccgagacagccttggagtctgaggtcgaatccgagacagcatcggattcgaccgagtctggggaccaggaggaagccccccgcatcggtggccgtagggccccccggaggcttggggggcggttttttctggacatgtcggcggaatccaccacggggacggaaacggatgcgtcggtgtcggacgaccccgacgacacgtccgactggtcttgtgacgacattcccccacgacccaagcgggcccgggtaaacctgcggctcactagctctcccgatcggcgggatggggttatttttcctaagatggggcgggtccggtctacccgggaaacgcagccccgggcccccaccccgtcggccccaagcccaaatgcaatgctccggcgctcggtgcgccaggcccagaggcggagcagcgcacgatggacccccgacctgggctacatgcgccagtgtatcaatcagctgtttcgggtcctgcgggtcgcccgggacccccacggcagtgccaaccgcctgcgccacctgatacgcgactgttacctgatgggatactgccgagcccgtctggccccgcgcacgtggtgccgcttgctgcaggtgtccggcggaacctggggcatgcacctgcgcaacaccatacgggaggtggaggctcgattcgacgccaccgcagaacccgtgtgcaagcttccttgtttggaggccagacggtacggcccggagtgtgatcttagtaatctcgagattcatctcagcgcgacaagcgatgatgaaatctccgatgccaccgatctggaggccgccggttcggaccacacgctcgcgtcccagtccgacacggaggatgccccctcccccgttacgctggaaaccccagaaccccgcgggtccctcgctgtgcgtctggaggatgagtttggggagtttgactggaccccccaggagggctcccagccctggctgtctgcggtcgtggccgataccagctccgtggaacgcccgggcccatccgattctggggcgggtcgcgcagcagaagaccgcaagtgtctggacggctgccggaaaatgcgcttctccaccgcctgcccctatccgtgcagcgacacgtttctccggccgtgagtccggtcgccccgacccccttgtatgtccccaaa

SEQ ID NO: 7 - DNA, 360 bp, unidentified
  source 1..360: mol_type = genomic DNA; note = human herpesvirus 1 strain McKrae ICP47
tccgcccagagactcgggtgatggtcgtacccgggactcaacgggttaccggattacggggactgtcggtcacggtcccgccggttcttcgatgtgccacacccaaggatgcgttgggggcgatttcgggcagcagcccgggagagcgcagcaggggacgctccgggtcgtgcacggcggttctggccgcctcccggtcctcacgcccccttttattgatctcatcgcgtacgtcggcgtacgtcctgggcccaacccgcatgttgtccaggaaggtgtccgccatttccagggcccacgacatgcttttccccccgacgagcaggaagcggtccacgcaacggtcgccgccggtcgcct

SEQ ID NO: 8 - DNA, 523 bp, unidentified
  source 1..523: mol_type = genomic DNA; note = Human cytomegalovirus
gaagatctttggttatatagcataaatcaatattggctattggccattgcatacgttgtatccatatcataatatgtacatttatattggctcatgtccaacattaccgccatgttgacattgattattgactagttattaatagtaatcaattacggggtcattagttcatagcccatatatggagttccgcgttacataacttacggtaaatggcccgcctggctgaccgcccaacgacccccgcccattgacgtcaataatgacgtatgttcccatagtaacgccaatagggactttccattgacgtcaatgggtggagtatttacggtaaactgcccacttggcagtacatcaagtgtatcatatgccaagtacgccccctattgacgtcaatgacggtaaatggcccgcctggcattatgcccagtacatgaccttatgggactttcctacttggcagtacatctacgtattagtcatcgctattaccatggtgatgcggttttggcagtacatcaat

SEQ ID NO: 9 - DNA, 1199 bp, Homo sapiens
  source 1..1199: mol_type = genomic DNA
aatgggtttgggtgtgtgtaaatgagtgtgaccggaagcgagtgtgagcttgatctaggcagggaccacacagcactgtcacacctgcctgctctttagtagaggactgaagtgcgggggtgggggtacggggccggaatagaatgtctctgggacatcttggcaaacagcagccggaagcaaaggggcagctgtgcaaacggctcaggcaggtgatggatggcagggtaggaagggggaggtccagaggtctggatggaggcttccgcatctgtaccttgcaactcacccctcaggcccagcaggtcatcggccccctcctcacacatgtaatgacgtagaagagtaccccgggacagtccggggagatggagattcggaaagtatccatggagctcttacagaatcccctgtgcggaccaggaaactcttgtagatccctgcctatctgaggcccaggcgctgggctgtttctcacaatattccttcaagatgagattgtggtccccatttcaaagatgagtacactgagcctctgtgaagttacttgcccatgatcacacaaccaggaattgggccaactgtaattgaactcctgtctaacaaagttcttgctcccagctccgtctcttgtttcccacgagccctggccctctgtgggtaataccagctactggagtcagatttcttgggcccagaacccacccttaggggcattaacctttaaaatctcacttgggcaggggtctgggatcagagttggaagagtccctacaatcctggaccctttccgccaaatcgtgaaaccaggggtggagtggggcgagggttcaaaaccaggccggactgagaggtgaaattcaccatgacgtcaaactgccctcaaattcccgctcactttaagggcgttacttgttggtgcccccaccatcccccaccatttccatcaatgacctcaatgcaaatacaagtgggacggtcctgctgacgcctccaggttctggaagcatgagggtgacgcacccaggggcaaaggacccctccgcccattggttgctgtgcactggcggaactttcccgacccacagcggcgggaataagagcagtcgctggcgctgggaggcatcagagacactgcccagcccaagtgtcgccgccgcttccacagggctctggctggacgccgccgccgccgctgc

SEQ ID NO: 10 - DNA, 225 bp, synthetic construct
  misc_feature 1..225: note = bovine growth hormone polyadenylation signal
  source 1..225: mol_type = other DNA
ggatcccgactgtgccttctagttgccagccatctgttgtttgcccctcccccgtgccttccttgaccctggaaggtgccactcccactgtcctttcctaataaaatgaggaaattgcatcgcattgtctgagtaggtgtcattctattctggggggtggggtggggcaggacagcaagggggaggattgggaagacaatagcaggcatgctggggaagatcttc

SEQ ID NO: 11 - protein, 7 aa, unidentified
  source 1..7: note = human herpesvirus 1 strain McKrae
STPSTTT

SEQ ID NO: 12 - DNA, 16 bp, unidentified
  source 1..16: mol_type = genomic DNA; note = human herpesvirus 1 strain McKrae
gcacccccactcccac

SEQ ID NO: 13 - DNA, 16 bp, unidentified
  source 1..16: mol_type = genomic DNA; note = human herpesvirus 1 strain McKrae
ccccagccctccccag

SEQ ID NO: 14 - DNA, 17 bp, unidentified
  source 1..17: mol_type = genomic DNA; note = human herpesvirus 1 strain McKrae
cccctcgccccctcccg

SEQ ID NO: 15 - protein, 14 aa, unidentified
  source 1..14: note = human herpesvirus 1 strain KOS
AASAPDAADALAAA

SEQ ID NO: 16 - protein, 13 aa, unidentified
  source 1..13: note = human herpesvirus 1 strain McKrae
GPRRSSSSSGVAA

SEQ ID NO: 17-18 - skipped (2 entries)

SEQ ID NO: 19 - protein, 9 aa, unidentified
  source 1..9: note = human herpesvirus 1
TAATGARAT